European Patent Application EP 4 230 650 A1, published August 23, 2023. Title: ANTIBODIES. Applicant: Oxford University Innovation Limited. Application EP. The sequence listing filed with the application follows.

SEQUENCE LISTING (967 sequences)

SEQ ID NO: 1 - DNA, 379 bp, Homo sapiens
  source 1..379: mol_type = other DNA
gaggtgcagctggtgcagtctggggctgaggtgaagaagcctgggtcctcggtgaaggtctcctgcaaggcttctggaggcaccttcagcaactatgctatcagctgggtgcgacaggcccctggacaagggcttgagtggatgggagggatcatccctatctttggtacagcaaactacgcacagaacttccagggcagagtcacgattaccgcggacgaatccatgagcacagcctacatggagctgagcagcctgagatctgaggacacggccgtatattactgtgcgggaggtgggaggtattgtagtggtggtaggtgccactctgcctactctgcctactggggccagggaaccctggtcaccgtctcctcag

SEQ ID NO: 2 - protein, 126 aa, Homo sapiens
EVQLVQSGAEVKKPGSSVKVSCKASGGTFSNYAISWVRQAPGQGLEWMGGIIPIFGTANYAQNFQGRVTITADESMSTAYMELSSLRSEDTAVYYCAGGGRYCSGGRCHSAYSAYWGQGTLVTVSS

SEQ ID NO: 3 - DNA, 322 bp, Homo sapiens
  source 1..322: mol_type = other DNA
gccatccagttgacccagtctccaggcaccctgtctttgcctccaggggaaagagccaccctctcctgcagggccagtcagagtgttagcagcagctacttagcctggtaccagcagaaacctggccaggctcccaggctcctcatctatggtgcatccagcagggccactggcatcccagacaggttcagtggcagtgggtctgggacagacttcactctcaccatcagcagactggaccctgaagattttgcagtgtattactgtcagcaatatggtagctcactcactttcggcggagggaccaaagtggatatcaaac

SEQ ID NO: 4 - protein, 107 aa, Homo sapiens
AIQLTQSPGTLSLPPGERATLSCRASQSVSSSYLAWYQQKPGQAPRLLIYGASSRATGIPDRFSGSGSGTDFTLTISRLDPEDFAVYYCQQYGSSLTFGGGTKVDIK

SEQ ID NO: 5 - protein, 8 aa, Homo sapiens
GGTFSNYA

SEQ ID NO: 6 - protein, 8 aa, Homo sapiens
IIPIFGTA

SEQ ID NO: 7 - protein, 19 aa, Homo sapiens
AGGGRYCSGGRCHSAYSAY

SEQ ID NO: 8 - protein, 7 aa, Homo sapiens
QSVSSSY

SEQ ID NO: 9 - skipped

SEQ ID NO: 10 - protein, 8 aa, Homo sapiens
QQYGSSLT

SEQ ID NO: 11 - DNA, 364 bp, Homo sapiens
  source 1..364: mol_type = other DNA
caggtgcagctggtggagtctgggggaggcttggtccaccctggggggtccctgagactctcctgttcagcctctggattcaccttcagtaactatgctatgcactgggtccgccaggctccagggaagggactggaatatgtttcagctattagtagtagtggggatatcacatactacgcggactccgtaaagggcagattcaccatctccagagacaattccaagaactcactgtatcttcaaatgaacagtctgagagctgaggacacggctgtttattactgtgtgaaagatgtaacgaggacctactacgtagtctttgactactggggccagggaaccctggtcaccgtctcctcag

SEQ ID NO: 12 - protein, 121 aa, Homo sapiens
QVQLVESGGGLVHPGGSLRLSCSASGFTFSNYAMHWVRQAPGKGLEYVSAISSSGDITYYADSVKGRFTISRDNSKNSLYLQMNSLRAEDTAVYYCVKDVTRTYYVVFDYWGQGTLVTVSS

SEQ ID NO: 13 - DNA, 322 bp, Homo sapiens
  source 1..322: mol_type = other DNA
gccatccagttgacccagtctccatcctccctgtctgcatctgtgggagacagagtcaccatcacttgccgggcaagtcagagcattagcagttatttaaattggtatcagcaggaaccagggaaagcccctaaactcctgatctatgctgcatccagtttgcaaggtggggtcccatcaaggttcagtggcagtggatctgggacagatttcactctcaccatcagcagtctgcaacctgaagattttgcaacttactactgtcaacagagttacactaccccgtacacttttggccaggggaccaaagtggatatcaaac

SEQ ID NO: 14 - protein, 107 aa, Homo sapiens
AIQLTQSPSSLSASVGDRVTITCRASQSISSYLNWYQQEPGKAPKLLIYAASSLQGGVPSRFSGSGSGTDFTLTISSLQPEDFATYYCQQSYTTPYTFGQGTKVDIK

SEQ ID NO: 15 - protein, 8 aa, Homo sapiens
GFTFSNYA

SEQ ID NO: 16 - protein, 8 aa, Homo sapiens
ISSSGDIT

SEQ ID NO: 17 - protein, 14 aa, Homo sapiens
VKDVTRTYYVVFDY

SEQ ID NO: 18 - protein, 6 aa, Homo sapiens
QSISSY

SEQ ID NO: 19 - skipped

SEQ ID NO: 20 - protein, 9 aa, Homo sapiens
QQSYTTPYT

SEQ ID NO: 21 - DNA, 358 bp, Homo sapiens
  source 1..358: mol_type = other DNA
caggtgcagctggtggagtctgggggaggcttggtccagcctggggggtccctgagactctcctgtgcagtctctggattcaccgtcagtaggaactacatgagctgggtccgccaggctccagggaaggggctggagtgggtctcacttatttatagcggtggtagcacattctacgcagactccgtgaagggcagattcaccatctccagagacaattccaagaacacgctgtatcttcaaatgaacagcctgagagccgaggacacggctgtgtattactgtgcgagagatctgtttcataggagtggttatcacgactactggggccagggaaccctggtcaccgtctcctcag

SEQ ID NO: 22 - protein, 119 aa, Homo sapiens
QVQLVESGGGLVQPGGSLRLSCAVSGFTVSRNYMSWVRQAPGKGLEWVSLIYSGGSTFYADSVKGRFTISRDNSKNTLYLQMNSLRAEDTAVYYCARDLFHRSGYHDYWGQGTLVTVSS

SEQ ID NO: 23 - DNA, 319 bp, Homo sapiens
  source 1..319: mol_type = other DNA
gtcatctggatgacccagtctccatcctccctgtctgcatctgtaggagacagagtcaccatcacttgccaggcgagtcaggacattaacaactatttaaattggtatcagcagaaaccagggaaagcccctaagctcctgatcttcgatgcctccaatttggaaacaggggtcccatcaaggttcagtggcagtggatctgggacagattttactttcaccatcagcagcctacagcctgaagatattgcaacatattactgtcaacagtatgataatctccctgccttcggcggagggaccaaagtggatatcaaac

SEQ ID NO: 24 - protein, 106 aa, Homo sapiens
VIWMTQSPSSLSASVGDRVTITCQASQDINNYLNWYQQKPGKAPKLLIFDASNLETGVPSRFSGSGSGTDFTFTISSLQPEDIATYYCQQYDNLPAFGGGTKVDIK

SEQ ID NO: 25 - protein, 8 aa, Homo sapiens
GFTVSRNY

SEQ ID NO: 26 - protein, 7 aa, Homo sapiens
IYSGGST

SEQ ID NO: 27 - protein, 13 aa, Homo sapiens
ARDLFHRSGYHDY

SEQ ID NO: 28 - protein, 6 aa, Homo sapiens
QDINNY

SEQ ID NO: 29 - skipped

SEQ ID NO: 30 - protein, 8 aa, Homo sapiens
QQYDNLPA

SEQ ID NO: 31 - DNA, 361 bp, Homo sapiens
  source 1..361: mol_type = other DNA
gaagtgcagctggtggagtctgggggaggcgtggtccagcctgggaggtccctgagactctcctgtgcagcgtctggattcaccttcagtaactatggcatgcactgggtccgccaggctccaggcaaggggctggagtgggtggcggttgtatggtatgatggaagcaagaaatactatgcagactccgtgaagggccgattcaccatctccagagacaattccaagaacaccctgtatctgcaaatgaacagcctgagagtcgaggacacggctgtgtattactgcgcgagagattttgcggtgggggaggagatcgctgactcctggggccagggaaccctggtcaccgtctcctcag

SEQ ID NO: 32 - protein, 120 aa, Homo sapiens
EVQLVESGGGVVQPGRSLRLSCAASGFTFSNYGMHWVRQAPGKGLEWVAVVWYDGSKKYYADSVKGRFTISRDNSKNTLYLQMNSLRVEDTAVYYCARDFAVGEEIADSWGQGTLVTVSS

SEQ ID NO: 33 - DNA, 325 bp, Homo sapiens
  source 1..325: mol_type = other DNA
tcctatgagctgactcagccaccctcggtgtcagtgtccccaggacaaacggccaggatcacctgctctggagatgcattgccaaaaaaatatgcttattggtaccagcagaagtcaggccaggcccctgtactggtcatctatgaggacagcaaacgaccctccgggatccctgagagattctctgggtccagctcagggacaatggccaccttgactatcagtggggcccaggtggaggatgaaggtgactactactgttactcaagagacagcagtggtgatcattgggtgttcggcgcagggaccaagctgaccgtcctag

SEQ ID NO: 34 - protein, 108 aa, Homo sapiens
SYELTQPPSVSVSPGQTARITCSGDALPKKYAYWYQQKSGQAPVLVIYEDSKRPSGIPERFSGSSSGTMATLTISGAQVEDEGDYYCYSRDSSGDHWVFGAGTKLTVL

SEQ ID NO: 35 - protein, 8 aa, Homo sapiens
GFTFSNYG

SEQ ID NO: 36 - protein, 8 aa, Homo sapiens
VWYDGSKK

SEQ ID NO: 37 - protein, 13 aa, Homo sapiens
ARDFAVGEEIADS

SEQ ID NO: 38 - protein, 6 aa, Homo sapiens
ALPKKY

SEQ ID NO: 39 - skipped

SEQ ID NO: 40 - protein, 11 aa, Homo sapiens
YSRDSSGDHWV

SEQ ID NO: 41 - DNA, 363 bp, Homo sapiens
  source 1..363: mol_type = other DNA
caggtgcagctggtggagtctgggggaggcgtggtccagcctgggaggtccctgagactctcctgtgcagcctctggattcaccttcagtacctatgctatgcactgggtccgccaggctccaggcaaggggctggagtgggtggctgttctttcatatgatggaagcaataaatactacgcagactccgtgaagggccgattcaccatctccagagacaattccaagaacacgctgtatctgcaaatgaacagcctgagagctgaggacacggctgtgtattactgtgcgaaagggggctcgtacgcgtactactactacatggacgtctggggcaaagggaccacggtcaccgtctcctca

SEQ ID NO: 42 - protein, 121 aa, Homo sapiens
QVQLVESGGGVVQPGRSLRLSCAASGFTFSTYAMHWVRQAPGKGLEWVAVLSYDGSNKYYADSVKGRFTISRDNSKNTLYLQMNSLRAEDTAVYYCAKGGSYAYYYYMDVWGKGTTVTVSS

SEQ ID NO: 43 - DNA, 322 bp, Homo sapiens
  source 1..322: mol_type = other DNA
gacatccagttgacccagtctccatcctccctgtctgcatctgtaggagacagagtcaccatcacttgccaggcgagtcaggacattagcaactatttaaattggtatcagcagaaaccagggaaagcccctaagctcctgatctacgatgcatccaatttggaaacaggggtcccatcaaggttcagtggaggtggatctgggacagattttactttcaccatcaccagcctgcagcctgaagatattgcaacatattactgtcaacagtatgataatctcccgctcactttcggcggagggaccaaagtggatatcaaac

SEQ ID NO: 44 - protein, 107 aa, Homo sapiens
DIQLTQSPSSLSASVGDRVTITCQASQDISNYLNWYQQKPGKAPKLLIYDASNLETGVPSRFSGGGSGTDFTFTITSLQPEDIATYYCQQYDNLPLTFGGGTKVDIK

SEQ ID NO: 45 - protein, 8 aa, Homo sapiens
GFTFSTYA

SEQ ID NO: 46 - protein, 8 aa, Homo sapiens
LSYDGSNK

SEQ ID NO: 47 - protein, 14 aa, Homo sapiens
AKGGSYAYYYYMDV

SEQ ID NO: 48 - protein, 6 aa, Homo sapiens
QDISNY

SEQ ID NO: 49 - skipped

SEQ ID NO: 50 - protein, 9 aa, Homo sapiens
QQYDNLPLT

SEQ ID NO: 51 - DNA, 376 bp, Homo sapiens
  source 1..376: mol_type = other DNA
gttcagctggtgcaggagtcgggcccaggactggtgaagccttcggagaccctgtccctcacctgcactgtctctggtggctccgtcagtagtggtagttactactggagctggatccggcagcccccagggaagggactggagtggattgggtatatgtatttcagtgggagcaccaactataatccctccctcaagagtcgagtcaccatatcattagccacgtccaagaaccagttctccctgaagctgagctctgtgaccgctgcggacacggccgtctattactgtgcgagaggggattacgatttttggagtggtccccccggtcgggtggacgtctggggcaaagggaccacggtcaccgtctcctcag

SEQ ID NO: 52 - protein, 125 aa, Homo sapiens
VQLVQESGPGLVKPSETLSLTCTVSGGSVSSGSYYWSWIRQPPGKGLEWIGYMYFSGSTNYNPSLKSRVTISLATSKNQFSLKLSSVTAADTAVYYCARGDYDFWSGPPGRVDVWGKGTTVTVSS

SEQ ID NO: 53 - DNA, 325 bp, Homo sapiens
  source 1..325: mol_type = other DNA
gaaatagtgatgacgcagtctccaggcaccctgtctttgtctccaggggaaagagccaccctctcctgcagggccagtcagagtgttagcagcagctacttagcctggtaccagcagaaacctggccaggctcccaggctcctcatctatggtgcatccagcagggccactggcatcccagacaggttcagtggcagtgggtctgggacagacttcactctcaccatcagcagactggagcctgaagattttgcagtgtattactgtcagcactatggtagttcacccgtaacttttggccaggggaccaaagtggatatcaaac

SEQ ID NO: 54 - protein, 108 aa, Homo sapiens
EIVMTQSPGTLSLSPGERATLSCRASQSVSSSYLAWYQQKPGQAPRLLIYGASSRATGIPDRFSGSGSGTDFTLTISRLEPEDFAVYYCQHYGSSPVTFGQGTKVDIK

SEQ ID NO: 55 - protein, 10 aa, Homo sapiens
GGSVSSGSYY

SEQ ID NO: 56 - protein, 7 aa, Homo sapiens
MYFSGST

SEQ ID NO: 57 - protein, 17 aa, Homo sapiens
ARGDYDFWSGPPGRVDV

SEQ ID NO: 58 - protein, 7 aa, Homo sapiens
QSVSSSY

SEQ ID NO: 59 - skipped

SEQ ID NO: 60 - protein, 9 aa, Homo sapiens
QHYGSSPVT

SEQ ID NO: 61 - DNA, 367 bp, Homo sapiens
  source 1..367: mol_type = other DNA
caggtgcagctggtgcagtctgggcctgaggtgaagaagcctgggacctcagtgaaggtctcctgcaaggcttctggattcacctttactagctctgctgtgcagtgggtgcgacaggctcgtggacaacgccttgagtggataggatggatcgtcgttggcagtggtaacacaaactacgcacagaagttccaggaaagagtcaccattaccagggacatgtccacaagcacagcctacatggagatgagcagcctgagatccgaggacacggccgtgtattactgtgcggcaccggcctgtggtaccagctgctctgatgcctttgatatctggggccaagggacaatggtcaccgtctcttcag

SEQ ID NO: 62 - protein, 122 aa, Homo sapiens
QVQLVQSGPEVKKPGTSVKVSCKASGFTFTSSAVQWVRQARGQRLEWIGWIVVGSGNTNYAQKFQERVTITRDMSTSTAYMEMSSLRSEDTAVYYCAAPACGTSCSDAFDIWGQGTMVTVSS

SEQ ID NO: 63 - DNA, 325 bp, Homo sapiens
  source 1..325: mol_type = other DNA
gacatccagatgacccagtctccaggcaccctgtctttgtctccaggggaaagagccaccctctcctgcagggccagtcagagtgttagcagcagctacttagcctggtaccagcagaaacctggccaggctcccaggctcctcatctatggtgcatccagcagggccactggcatcccagacaggttcagtggcagtgggtctgggacagacttcactctcaccatcagcagactggagcctgaagattttggagtgtattactgtcagcagtatggtagctcaccgtggacgttcggccaagggaccaaggtggaaatcaaac

SEQ ID NO: 64 - protein, 108 aa, Homo sapiens
DIQMTQSPGTLSLSPGERATLSCRASQSVSSSYLAWYQQKPGQAPRLLIYGASSRATGIPDRFSGSGSGTDFTLTISRLEPEDFGVYYCQQYGSSPWTFGQGTKVEIK

SEQ ID NO: 65 - protein, 8 aa, Homo sapiens
GFTFTSSA

SEQ ID NO: 66 - protein, 8 aa, Homo sapiens
IVVGSGNT

SEQ ID NO: 67 - protein, 15 aa, Homo sapiens
AAPACGTSCSDAFDI

SEQ ID NO: 68 - protein, 7 aa, Homo sapiens
QSVSSSY

SEQ ID NO: 69 - skipped

SEQ ID NO: 70 - protein, 9 aa, Homo sapiens
QQYGSSPWT

SEQ ID NO: 71 - DNA, 382 bp, Homo sapiens
  source 1..382: mol_type = other DNA
caggtgcagctggtggagtctgggggaggcttggtacagcctggcaggtccctgagactctcctgtgcagcctctggattcacctttgatgattatgccatgcactgggtccggcaacctccagggaagggcctggagtgggtctcaggtgtcagttggaacagtggtaccataggctatgcggactctgtgaagggccgattcatcatctccagagacaacgccaagaactccctgtatctgcaaatgaacagtctgaaagctgaggacacggccttgtattactgtgcaagagaagtgggggggacttttggagtccttatttcacgcgaggggggacttgattactggggccagggaaccctggtcaccgtctcctcag

SEQ ID NO: 72 - protein, 127 aa, Homo sapiens
QVQLVESGGGLVQPGRSLRLSCAASGFTFDDYAMHWVRQPPGKGLEWVSGVSWNSGTIGYADSVKGRFIISRDNAKNSLYLQMNSLKAEDTALYYCAREVGGTFGVLISREGGLDYWGQGTLVTVSS

SEQ ID NO: 73 - DNA, 325 bp, Homo sapiens
  source 1..325: mol_type = other DNA
tcctatgagctgacacagccaccctcggtgtcagtggccccaggacagacggccagaattacctgtgggggaaacaccattggaagtaaaagtgtgcactggtaccagcagagaccaggccaggcccctgtgctggtcgtctatgatgatagcgaccggccctcagggatccctgagcgattctctggctccaactctgggaacacggccaccctgaccatcagcagggtcgaagccggggatgaggccgactattactgtcaggtgtgggatagtagtagtgatcgggtggtattcggcggagggaccaagctgaccgtcctag

SEQ ID NO: 74 - protein, 108 aa, Homo sapiens
SYELTQPPSVSVAPGQTARITCGGNTIGSKSVHWYQQRPGQAPVLVVYDDSDRPSGIPERFSGSNSGNTATLTISRVEAGDEADYYCQVWDSSSDRVVFGGGTKLTVL

SEQ ID NO: 75 - protein, 8 aa, Homo sapiens
GFTFDDYA

SEQ ID NO: 76 - protein, 8 aa, Homo sapiens
VSWNSGTI

SEQ ID NO: 77 - protein, 20 aa, Homo sapiens
AREVGGTFGVLISREGGLDY

SEQ ID NO: 78 - protein, 6 aa, Homo sapiens
TIGSKS

SEQ ID NO: 79 - skipped

SEQ ID NO: 80 - protein, 11 aa, Homo sapiens
QVWDSSSDRVV

SEQ ID NO: 81 - DNA, 385 bp, Homo sapiens
  source 1..385: mol_type = other DNA
caggtgcagctgcaggagtcgggcccaggactggtgaagccttcggagaccctgtccctcatctgcactgtctctggtggctccgtcagcagtggtaatttctactggagctggatccggcagcccccagggaagggactggagtggattggatctatctattacactgggagccccaactacaacccctccctcaagagtcgagtcaccatatccctagacacgtccaagaaccagttctccctgaagctgagctctgtgaccgctgcggacacggccgtgtattactgtgcgagagagatctattattatgatagaagtggttcttacaactctgatgcttttgatatctggggccaagggacaatggtcaccgtctcttcag

SEQ ID NO: 82 - protein, 128 aa, Homo sapiens
QVQLQESGPGLVKPSETLSLICTVSGGSVSSGNFYWSWIRQPPGKGLEWIGSIYYTGSPNYNPSLKSRVTISLDTSKNQFSLKLSSVTAADTAVYYCAREIYYYDRSGSYNSDAFDIWGQGTMVTVSS

SEQ ID NO: 83 - DNA, 325 bp, Homo sapiens
  source 1..325: mol_type = other DNA
gatatcgtgatgactcagtctccagccaccctgtctgtgtctccaggggaaagaggcaccctctcctgcagggccagtcagagtgttagcagcaacttagcctggtaccagcagaaaccgggccaggctcccaggctcctcatctatggtgcatccacgagggccactggtatcccagccaggttcagtggcagtgggtctgggacagagttcactctcaccatcagcagcctgcagtctgaagattttgcagtttattactgccagcagtataataactggcctccgctcactttcggcggagggaccaaagtggatatcaaac

SEQ ID NO: 84 - protein, 108 aa, Homo sapiens
DIVMTQSPATLSVSPGERGTLSCRASQSVSSNLAWYQQKPGQAPRLLIYGASTRATGIPARFSGSGSGTEFTLTISSLQSEDFAVYYCQQYNNWPPLTFGGGTKVDIK

SEQ ID NO: 85 - protein, 10 aa, Homo sapiens
GGSVSSGNFY

SEQ ID NO: 86 - protein, 7 aa, Homo sapiens
IYYTGSP

SEQ ID NO: 87 - protein, 20 aa, Homo sapiens
AREIYYYDRSGSYNSDAFDI

SEQ ID NO: 88 - protein, 6 aa, Homo sapiens
QSVSSN

SEQ ID NO: 89 - skipped

SEQ ID NO: 90 - protein, 10 aa, Homo sapiens
QQYNNWPPLT

SEQ ID NO: 91 - DNA, 381 bp, Homo sapiens
  source 1..381: mol_type = other DNA
caggtgcagctggtggagtctgggggaggcgtggttcagcctgggaggtccctgagactctcctgtgcagcctctggattcaccttcaataactatcctttgcactgggtccgccaggctccaggcaaggggccggagtgggtggcagttatttcacaggatggaggcaataaatactacgtagactccgtgaagggccgattcaccatctccagagacaattccaagaacaccctgtatctgcaaatgaacaacctgagagctgaggacacggctctgtattactgtgcgagagatgttgtagtggtggtagctgctaggaaccactactacaacggtatggacgtctggggccaagggaccacggtcaccgtctcctca

SEQ ID NO: 92 - protein, 127 aa, Homo sapiens
QVQLVESGGGVVQPGRSLRLSCAASGFTFNNYPLHWVRQAPGKGPEWVAVISQDGGNKYYVDSVKGRFTISRDNSKNTLYLQMNNLRAEDTALYYCARDVVVVVAARNHYYNGMDVWGQGTTVTVSS

SEQ ID NO: 93 - DNA, 322 bp, Homo sapiens
  source 1..322: mol_type = other DNA
gacatccagttgacccagtctccatcttccgtgtctgcatctgtaggagacagagtcaccatcacttgtcgggcgagtcagggtattagcagctggttagcctggtatcagcagaaaccagggaaagcccctaagctcctgatctatgctgtatccagtttgcaaagtggggtcccatcaaggttcagcggcagtggatctgggacagatttcactctcaccatcagcagcctgcagcctgaagattttgcaacttactattgtcaacaggctaagagtttccctttcactttcggccctgggaccaaggtggagattaaac

SEQ ID NO: 94 - protein, 107 aa, Homo sapiens
DIQLTQSPSSVSASVGDRVTITCRASQGISSWLAWYQQKPGKAPKLLIYAVSSLQSGVPSRFSGSGSGTDFTLTISSLQPEDFATYYCQQAKSFPFTFGPGTKVEIK

SEQ ID NO: 95 - protein, 8 aa, Homo sapiens
GFTFNNYP

SEQ ID NO: 96 - protein, 8 aa, Homo sapiens
ISQDGGNK

SEQ ID NO: 97 - protein, 20 aa, Homo sapiens
ARDVVVVVAARNHYYNGMDV

SEQ ID NO: 98 - protein, 6 aa, Homo sapiens
QGISSW

SEQ ID NO: 99 - skipped

SEQ ID NO: 100 - protein, 9 aa, Homo sapiens
QQAKSFPFT

SEQ ID NO: 101 - DNA, 381 bp, Homo sapiens
  source 1..381: mol_type = other DNA
cagctgcagctgcaggagtcgggcccaggactggtgaagccttcacagaccctgtccctcacctgcactgtctctggtggctccatcagtagtggtagttataattggacctggatccggcagcccgccgggaagggactggagtggattgggcgtatatataatagtgggagcaccaactacaacccctccctcaagagtcgagtcaccatatcagtagacacgtccaagaaccagttgtccctgaaggtgaggtctgtgaccgccgcagacacggccgtgtattactgtgcgagacattgcagtggtggtacctgctacccgaagtactactacggtatggacgtctggggccaagggaccacggtcaccgtctcctca

SEQ ID NO: 102 - protein, 127 aa, Homo sapiens
QLQLQESGPGLVKPSQTLSLTCTVSGGSISSGSYNWTWIRQPAGKGLEWIGRIYNSGSTNYNPSLKSRVTISVDTSKNQLSLKVRSVTAADTAVYYCARHCSGGTCYPKYYYGMDVWGQGTTVTVSS

SEQ ID NO: 103 - DNA, 331 bp, Homo sapiens
  source 1..331: mol_type = other DNA
caatctgccctgactcagccaccctcggtgtctgaagcccccaggcagagggtcaccatctcctgttctggaagcagctccaacatcggaaataatgctgtaaactggtaccagcagttcccaggaaaggctcccaaactcctcatctattatgatgatctgctgccctcaggggtctctgaccgattctctggctccaagtctggcacctcagcctccctggccatcagtggggtccagtctgaggatgaggctgattattactgtgcagcatgggatgacagcctgaatgtcgtggtattcggcggagggaccaagctgaccgtcctag

SEQ ID NO: 104 - protein, 110 aa, Homo sapiens
QSALTQPPSVSEAPRQRVTISCSGSSSNIGNNAVNWYQQFPGKAPKLLIYYDDLLPSGVSDRFSGSKSGTSASLAISGVQSEDEADYYCAAWDDSLNVVVFGGGTKLTVL

SEQ ID NO: 105 - protein, 10 aa, Homo sapiens
GGSISSGSYN

SEQ ID NO: 106 - protein, 7 aa, Homo sapiens
IYNSGST

SEQ ID NO: 107 - protein, 19 aa, Homo sapiens
ARHCSGGTCYPKYYYGMDV

SEQ ID NO: 108 - protein, 8 aa, Homo sapiens
SSNIGNNA

SEQ ID NO: 109 - skipped

SEQ ID NO: 110 - protein, 11 aa, Homo sapiens
AAWDDSLNVVV

SEQ ID NO: 111 - DNA, 370 bp, Homo sapiens
  source 1..370: mol_type = other DNA
caggtgcagctggtggagtcgggcccaggactggtgaagccttcggagaccctgtccctcacctgcactgtctctggtggctccatcagcagtaatagttacttctggggctggatccgccagcccccagggacggggctggagtggattgggaatatctattatactgggagcacctactacaacccgtcgttcgagagtcgagtcaccatgtccgtagacacgtcgaagaaccagttctccctgaggctgagctctgtgaccgccgcagacacggctgtgtattactgtgcgagacatgtcagggcctacgactatgatgccccttttgatatctggggccaagggacaatggtcaccgtctcttcag

SEQ ID NO: 112 - protein, 123 aa, Homo sapiens
QVQLVESGPGLVKPSETLSLTCTVSGGSISSNSYFWGWIRQPPGTGLEWIGNIYYTGSTYYNPSFESRVTMSVDTSKNQFSLRLSSVTAADTAVYYCARHVRAYDYDAPFDIWGQGTMVTVSS

SEQ ID NO: 113 - DNA, 322 bp, Homo sapiens
  source 1..322: mol_type = other DNA
gtcatctggatgacccagtctccatcctccctgtctgcatctgtaggagacagagtcaccatcacttgccgggcaagtcagggcattagaaatgatttaggctggtatcagcagaaaccagggaaagcccctaagcgcctgatctatgctgcatccagtttgcaaagtggggtcccatcaaggttcagcggcagtggatctgggacacaattcactctcacaatcagcagcctgcagcctgaagattttgcaacttattactgtctacagattaatagttatccgctcactttcggcggagggaccaaggtggaaatcaaac

SEQ ID NO: 114 - protein, 107 aa, Homo sapiens
VIWMTQSPSSLSASVGDRVTITCRASQGIRNDLGWYQQKPGKAPKRLIYAASSLQSGVPSRFSGSGSGTQFTLTISSLQPEDFATYYCLQINSYPLTFGGGTKVEIK

SEQ ID NO: 115 - protein, 10 aa, Homo sapiens
GGSISSNSYF

SEQ ID NO: 116 - protein, 7 aa, Homo sapiens
IYYTGST

SEQ ID NO: 117 - protein, 15 aa, Homo sapiens
ARHVRAYDYDAPFDI

SEQ ID NO: 118 - protein, 6 aa, Homo sapiens
QGIRND

SEQ ID NO: 119 - skipped

SEQ ID NO: 120 - protein, 9 aa, Homo sapiens
LQINSYPLT

SEQ ID NO: 121 - DNA, 349 bp, Homo sapiens
  source 1..349: mol_type = other DNA
caggtacagctgcagcagtggggcgcaggactgttgaagccttcggagaccctgtccctcacctgcgctgtctatggtgggtccttcagtggttactactggagctggatccgccagcccccagggaaggggctggagtggattggggaaatcaatcatagtggaagcaccaactacaacccgtccctcaagagtcgagtcaccatatcagtagacacgtccaagaaccagttctccctgaagctgagttctgtgaccgccgcggacacggctgtgtattactgtgcgagaactgattactatgatagtatagactggggccagggaaccctggtcaccgtctcctcag

SEQ ID NO: 122 - protein, 116 aa, Homo sapiens
QVQLQQWGAGLLKPSETLSLTCAVYGGSFSGYYWSWIRQPPGKGLEWIGEINHSGSTNYNPSLKSRVTISVDTSKNQFSLKLSSVTAADTAVYYCARTDYYDSIDWGQGTLVTVSS

SEQ ID NO: 123 - DNA, 328 bp, Homo sapiens
  source 1..328: mol_type = other DNA
cagtctgtgctgactcaggagccctcactgactgtgtccccaggagggacagtcactctcacctgtggctccagcactggagctgtcaccagtggtcattatccctactggttccagcagaagcctggccaagtccccaggacactgatttatgatacaaggaacaaacactcctggacccctgcccggttctcaggctccctccttgggggcaaagctgccctgaccctttcgggtgcgcagcctgaggatgaggctgaatattactgcttgctctcctctagtggtgctcgggtgttcggcggagggaccaagctgaccgtcctag

SEQ ID NO: 124 - protein, 109 aa, Homo sapiens
QSVLTQEPSLTVSPGGTVTLTCGSSTGAVTSGHYPYWFQQKPGQVPRTLIYDTRNKHSWTPARFSGSLLGGKAALTLSGAQPEDEAEYYCLLSSSGARVFGGGTKLTVL

SEQ ID NO: 125 - protein, 8 aa, Homo sapiens
GGSFSGYY

SEQ ID NO: 126 - protein, 7 aa, Homo sapiens
INHSGST

SEQ ID NO: 127 - protein, 10 aa, Homo sapiens
ARTDYYDSID

SEQ ID NO: 128 - protein, 9 aa, Homo sapiens
TGAVTSGHY

SEQ ID NO: 129 - skipped

SEQ ID NO: 130 - protein, 9 aa, Homo sapiens
LLSSSGARV

SEQ ID NO: 131 - DNA, 358 bp, Homo sapiens
  source 1..358: mol_type = other DNA
gaggtgcagctggtggagtctgggggaggcttggtacagcctggggggtccctgagactctcctgtgcagcctctggattcaccttcagtacctacgacatccactgggtccgccaagctacaggaaaaggtctggagtgggtctcagctattggtactgctggtgacacatactattcaggctccgtgaagggccgattcaccatctccagagaaaatgccaagaactccttgtatcttcaaatgaacagcctgagagccggggacacggctgtgtattactgtgcaaggggtagtgggacctacttctactactttgactactggggccagggaaccctggtcaccgtctcctcag

SEQ ID NO: 132 - protein, 119 aa, Homo sapiens
EVQLVESGGGLVQPGGSLRLSCAASGFTFSTYDIHWVRQATGKGLEWVSAIGTAGDTYYSGSVKGRFTISRENAKNSLYLQMNSLRAGDTAVYYCARGSGTYFYYFDYWGQGTLVTVSS

SEQ ID NO: 133 - DNA, 325 bp, Homo sapiens
  source 1..325: mol_type = other DNA
gacatcgtgatgactcagtctccatcctccctgtctgcatctgtaggagacagaatcaccatcacttgccgggcaagtcagagcattaacaactatttaaattggtatcagcagaaaccagggaaagcccctaagctcctgatctatgctgcatcccgtttgcaaactggggtcccatcaaggttcagtggcagtggatctgggacagattccactctcaccatcaacactctgcaacctgaagattttgcaacttactactgtcaacagagttacagtgcccctccgtggacgttcggccaagggaccaaagtggatatcaaac

SEQ ID NO: 134 - protein, 108 aa, Homo sapiens
DIVMTQSPSSLSASVGDRITITCRASQSINNYLNWYQQKPGKAPKLLIYAASRLQTGVPSRFSGSGSGTDSTLTINTLQPEDFATYYCQQSYSAPPWTFGQGTKVDIK

SEQ ID NO: 135 - protein, 8 aa, Homo sapiens
GFTFSTYD

SEQ ID NO: 136 - protein, 7 aa, Homo sapiens
IGTAGDT

SEQ ID NO: 137 - protein, 13 aa, Homo sapiens
ARGSGTYFYYFDY

SEQ ID NO: 138 - protein, 6 aa, Homo sapiens
QSINNY

SEQ ID NO: 139 - skipped

SEQ ID NO: 140 - protein, 10 aa, Homo sapiens
QQSYSAPPWT

SEQ ID NO: 141 - DNA, 366 bp, Homo sapiens
  source 1..366: mol_type = other DNA
caggtgcagctggtggagtcgggcccaggactggtgaagccttcggagaccctgtccctcacctgcactgtctctggtggctcgatcagcagttcttactactggggctggatccgccagcccccagggaaggggctggagtggattgggagtgtctattatagtgggagcacctactacaacccgtccctcaagagtcgagtcaccatatccgtggacacgtccaagaaccagttctccctgaggctgagctctgtgaccgccgcagacacggctgtgtattattgtgcgaggctgatgaccacggaagactactactccggtatggacgtctggggccaagggaccacggtcaccgtctcctca

SEQ ID NO: 142 - protein, 122 aa, Homo sapiens
QVQLVESGPGLVKPSETLSLTCTVSGGSISSSYYWGWIRQPPGKGLEWIGSVYYSGSTYYNPSLKSRVTISVDTSKNQFSLRLSSVTAADTAVYYCARLMTTEDYYSGMDVWGQGTTVTVSS

SEQ ID NO: 143 - DNA, 322 bp, Homo sapiens
  source 1..322: mol_type = other DNA
gccatccagatgacccagtctccatcctcactgtctgcatctgtaggagacagagtcaccatcacttgtcgggcgagtcagggcattagcgattatttagcctggtttcagcagaaaccagggaaagcccctaagtccctgatctatgctgcatccagtttgcaaagtggggtcccatcaaagttcagcggcggtggatctgggacagatttcactctcaccatcagcagcctgcagcctgaagattttgcaacttattactgccaacagtatcatagttacccgatcaccttcggccaagggacacgactggagattaaac

SEQ ID NO: 144 - protein, 107 aa, Homo sapiens
AIQMTQSPSSLSASVGDRVTITCRASQGISDYLAWFQQKPGKAPKSLIYAASSLQSGVPSKFSGGGSGTDFTLTISSLQPEDFATYYCQQYHSYPITFGQGTRLEIK

SEQ ID NO: 145 - protein, 9 aa, Homo sapiens
GGSISSSYY

SEQ ID NO: 146 - protein, 7 aa, Homo sapiens
VYYSGST

SEQ ID NO: 147 - protein, 15 aa, Homo sapiens
ARLMTTEDYYSGMDV

SEQ ID NO: 148 - protein, 6 aa, Homo sapiens
QGISDY

SEQ ID NO: 149 - skipped

SEQ ID NO: 150 - protein, 9 aa, Homo sapiens
QQYHSYPIT

SEQ ID NO: 151 - DNA, 351 bp, Homo sapiens
  source 1..351: mol_type = other DNA
caggtgcagctggtggagtctggaggaggcttgatccagcctggggggtccctgagactctcctgtgcagcctctggggtcaccgtcagtagcaactacatgagttgggtccgccaggctccagggaaggggctggagtgggtctcaattatttatagtggtggtaccacatactacgcagactccgtgaagggccgattcaccatctccagagactcttccatgaacacgctgtatcttcaaatgaacagcctgagagccgaggacacggccgtgtattactgtgcgagagatctgatggtgtacggtatagacgtctggggccaagggaccacggtcaccgtctcctca

SEQ ID NO: 152 - protein, 117 aa, Homo sapiens
QVQLVESGGGLIQPGGSLRLSCAASGVTVSSNYMSWVRQAPGKGLEWVSIIYSGGTTYYADSVKGRFTISRDSSMNTLYLQMNSLRAEDTAVYYCARDLMVYGIDVWGQGTTVTVSS

SEQ ID NO: 153 - DNA, 328 bp, Homo sapiens
  source 1..328: mol_type = other DNA
gaaatagtgatgacgcagtctccatcctccctgtctgcatctgtaggagacagagtcaccatcacttgccgggccagtcagggcattagcagttatttagcctggtatcagcaaaaaccagggaaagcccctaagctcctgatctatgctgcatccactttgcaaagtggggtcccatcaaggttcagcggcagtggatctgggacagatttcactctcaccatcagcagcctgcagcctgaagattttgcaacttattactgtcaacagcttgatagttacccccccgggtacacttttggccaggggaccaaagtggatatcaaac

SEQ ID NO: 154 - protein, 109 aa, Homo sapiens
EIVMTQSPSSLSASVGDRVTITCRASQGISSYLAWYQQKPGKAPKLLIYAASTLQSGVPSRFSGSGSGTDFTLTISSLQPEDFATYYCQQLDSYPPGYTFGQGTKVDIK

SEQ ID NO: 155 - protein, 8 aa, Homo sapiens
GVTVSSNY

SEQ ID NO: 156 - protein, 7 aa, Homo sapiens
IYSGGTT

SEQ ID NO: 157 - protein, 11 aa, Homo sapiens
ARDLMVYGIDV

SEQ ID NO: 158 - protein, 6 aa, Homo sapiens
QGISSY

SEQ ID NO: 159 - skipped

SEQ ID NO: 160 - protein, 11 aa, Homo sapiens
QQLDSYPPGYT

SEQ ID NO: 161 - DNA, 351 bp, Homo sapiens
  source 1..351: mol_type = other DNA
gaggtgcagctgttggagtctggaggagacttgatccagcctggggggtccctgagactctcctgtgcagcctctggggtcaccgtcagtagcaactacatgagctgggtccgccaggctccagggaaggggctggagtgggtctcaattatttatcccggtgggagcacattctacgcagactccgtgaagggccgattcaccatctccagagacaattccaagaacacgctgtatcttcaaatgcacagcctgagagccgaggacacggccgtgtattactgtgcgagagatcttggctcaggggacatggacgtctggggcaaagggaccacggtcaccgtctcctca

SEQ ID NO: 162 - protein, 117 aa, Homo sapiens
EVQLLESGGDLIQPGGSLRLSCAASGVTVSSNYMSWVRQAPGKGLEWVSIIYPGGSTFYADSVKGRFTISRDNSKNTLYLQMHSLRAEDTAVYYCARDLGSGDMDVWGKGTTVTVSS

SEQ ID NO: 163 - DNA, 322 bp, Homo sapiens
  source 1..322: mol_type = other DNA
gacatcgtgatgactcagtctccatccttcctgtctgcatctgtaggagacagagtcaccatcacttgccgggccagtcagggcattagcagttatttagcctggtatcagcaaaaaccggggaaagcccctaagctcctgatccaagctgcatccactttgcaaagtggggtcccatcaaggttcagcggcagtggatctgggacagaattcactctcacaatcagcagcctgcagcctgaagattttgcaacttattactgtcaacagcttaatagttaccggtacacttttggccaggggaccaaggtggagatcaaac

SEQ ID NO: 164 - protein, 107 aa, Homo sapiens
DIVMTQSPSFLSASVGDRVTITCRASQGISSYLAWYQQKPGKAPKLLIQAASTLQSGVPSRFSGSGSGTEFTLTISSLQPEDFATYYCQQLNSYRYTFGQGTKVEIK

SEQ ID NO: 165 - protein, 8 aa, Homo sapiens
GVTVSSNY

SEQ ID NO: 166 - protein, 7 aa, Homo sapiens
IYPGGST

SEQ ID NO: 167 - protein, 11 aa, Homo sapiens
ARDLGSGDMDV

SEQ ID NO: 168 - protein, 6 aa, Homo sapiens
QGISSY

SEQ ID NO: 169 - skipped

SEQ ID NO: 170 - protein, 9 aa, Homo sapiens
QQLNSYRYT

SEQ ID NO: 171 - DNA, 369 bp, Homo sapiens
  source 1..369: mol_type = other DNA
gaggtgcagctggtggagtctgggggaggcgtggtccagcctgggaggtccctgagactctcctgtgcagcctctggattcaccttcagtagctatggcatgcactgggtccgccaggctccaggcaaggggctggagtgggtggcacttatatcatatgatggaggtaatagatactatgcagactccgtgaagggccgattcaccatctccagagacaattccaagaacacgctgtatctgcaaatgaacagactgagagctgaagacacggctatgtattactgtgcgaaagatcgtgatgatgggtgggattggtactacttcatggacgtctggggcaaagggaccacggtcaccgtctcctca

SEQ ID NO: 172 - protein, 123 aa, Homo sapiens
EVQLVESGGGVVQPGRSLRLSCAASGFTFSSYGMHWVRQAPGKGLEWVALISYDGGNRYYADSVKGRFTISRDNSKNTLYLQMNRLRAEDTAMYYCAKDRDDGWDWYYFMDVWGKGTTVTVSS

SEQ ID NO: 173 - DNA, 322 bp, Homo sapiens
  source 1..322: mol_type = other DNA
gacatccagttgacccagtctccaggcaccctgtctttgtctccaggggaaagagccaccctctcctgcagggccagtcagagtattagcggcaactacttagcctggtaccagcataaacctggccaggctcccagactcctcatctatggtgcatccaccagggccactggcatcccagacaggttcagtggcagtgggtctgggacagacttcactctcaccatcagcagactggagcctgaagattttgcagtgtattactgtcagcagtatggtagctcgtacacttttggccaggggaccaaggtggagatcaaac

SEQ ID NO: 174 - protein, 107 aa, Homo sapiens
DIQLTQSPGTLSLSPGERATLSCRASQSISGNYLAWYQHKPGQAPRLLIYGASTRATGIPDRFSGSGSGTDFTLTISRLEPEDFAVYYCQQYGSSYTFGQGTKVEIK

SEQ ID NO: 175 - protein, 8 aa, Homo sapiens
GFTFSSYG

SEQ ID NO: 176 - protein, 8 aa, Homo sapiens
ISYDGGNR

SEQ ID NO: 177 - protein, 16 aa, Homo sapiens
AKDRDDGWDWYYFMDV

SEQ ID NO: 178 - protein, 7 aa, Homo sapiens
QSISGNY

SEQ ID NO: 179 - skipped

SEQ ID NO: 180 - protein, 8 aa, Homo sapiens
QQYGSSYT

SEQ ID NO: 181 - DNA, 370 bp, Homo sapiens
  source 1..370: mol_type = other DNA
caggttcagctggtgcagtctgggcctgaggtgaagaagcctgggacctcagtgaaggtctcctgcaaggcttctggattcacctttactagctctgctgtgcagtgggtgcgacaggctcgtggacagcgccttgagtggataggatggatcgtcgttggcagtggtaacacaaactacgcacagaagttccaggaaagcgtcaccattaccagggacatgtccacaagcacagcctacatggagctgagcagcctgagatccgaggacacggccgtgtattactgtgcggccccacattgtattggtggtagctgccatgatgcttttgatatctggggccaagggacaatggtcaccgtctcttcag

SEQ ID NO: 182 - protein, 123 aa, Homo sapiens
QVQLVQSGPEVKKPGTSVKVSCKASGFTFTSSAVQWVRQARGQRLEWIGWIVVGSGNTNYAQKFQESVTITRDMSTSTAYMELSSLRSEDTAVYYCAAPHCIGGSCHDAFDIWGQGTMVTVSS

SEQ ID NO: 183 - DNA, 325 bp, Homo sapiens
  source 1..325: mol_type = other DNA
gatatcgtgatgacccagtctccaggcaccctatctttgtctccaggggaaagagccaccctctcctgcagggccagtcagagtgttagaagcagctacttagcctggtaccagcagaaacctggccaggctcccaggctcctcatctatggtgcatccaggaggggcactggcatcccagacaggttcagtggcagtgggtctgggacagacttcactctcaccatcagcagactggagcctgaagattttgcagtgtattactgtcagcagtatggtagctcaccctggacgttcggccaagggaccaaggtggaaatcaaac

SEQ ID NO: 184 - protein, 108 aa, Homo sapiens
DIVMTQSPGTLSLSPGERATLSCRASQSVRSSYLAWYQQKPGQAPRLLIYGASRRGTGIPDRFSGSGSGTDFTLTISRLEPEDFAVYYCQQYGSSPWTFGQGTKVEIK

SEQ ID NO: 185 - protein, 8 aa, Homo sapiens
GFTFTSSA

SEQ ID NO: 186 - protein, 8 aa, Homo sapiens
IVVGSGNT

SEQ ID NO: 187 - protein, 16 aa, Homo sapiens
AAPHCIGGSCHDAFDI

SEQ ID NO: 188 - protein, 7 aa, Homo sapiens
QSVRSSY

SEQ ID NO: 189 - skipped

SEQ ID NO: 190 - protein, 9 aa, Homo sapiens
QQYGSSPWT

SEQ ID NO: 191 - DNA, 352 bp, Homo sapiens
  source 1..352: mol_type = other DNA
caggtgcagctggtggagtcaggagcagaggtgaaaaagcccggggagtctctgaagatctcctgtaagggttctggatacagctttaccagctactggatcgtctgggtgcgccagatgcccgggaaaggcctggagtggatggggatcatctatcctggtgactctgataccaaatacagtccgtccttccaaggccaggtcagcatctcagccgacaagcccatcagcaccgcctacctgcagtggagcaggctgaaggcctcggacaccgccatgtattactgtgcgagactagggaattggctggtggactactggggccagggaaccctggtcaccgtctcctcag

SEQ ID NO: 192 - protein, 117 aa, Homo sapiens
QVQLVESGAEVKKPGESLKISCKGSGYSFTSYWIVWVRQMPGKGLEWMGIIYPGDSDTKYSPSFQGQVSISADKPISTAYLQWSRLKASDTAMYYCARLGNWLVDYWGQGTLVTVSS

SEQ ID NO: 193 - DNA, 343 bp, Homo sapiens
  source 1..343: mol_type = other DNA
gatattgtgatgactcagtctcctctctctctgtccgtcacccctggacagccggcctccatctcctgcaagtctagtcagagcctcctgcatagtgatggaaagacctatttgtattggtacctgcagaagccaggccagcctccacagctcctgatgtatgaagtttccaaccggttctctggagtgccagataggttcagtggcagcgggtcagggacagacttcacacttaaaatcagccgggtggagtctgaggatgttggggtttattactgcatgcaaagtatacagcttcctcgcgggatcaccttcggccaagggacacgactggagattaaac

SEQ ID NO: 194 - protein, 114 aa, Homo sapiens
DIVMTQSPLSLSVTPGQPASISCKSSQSLLHSDGKTYLYWYLQKPGQPPQLLMYEVSNRFSGVPDRFSGSGSGTDFTLKISRVESEDVGVYYCMQSIQLPRGITFGQGTRLEIK

SEQ ID NO: 195 - protein, 8 aa, Homo sapiens
GYSFTSYW

SEQ ID NO: 196 - protein, 8 aa, Homo sapiens
IYPGDSDT

SEQ ID NO: 197 - protein, 10 aa, Homo sapiens
ARLGNWLVDY

SEQ ID NO: 198 - protein, 11 aa, Homo sapiens
QSLLHSDGKTY

SEQ ID NO: 199 - skipped

SEQ ID NO: 200 - protein, 11 aa, Homo sapiens
MQSIQLPRGIT

SEQ ID NO: 201 - DNA, 343 bp, Homo sapiens
  source 1..343: mol_type = other DNA
gaggtgcagctggtggagtctggaggaggcttgatccagcctggggggtccctgagactctcctgtgcagcctctgggctcaccgtcagtcgcaattacatgagctgggtccgccaggctccagggaaggggctggagtgggtctcacttatttatagcggtggtagcacatactacgcagactccgtgaagggccgattcaccatctccagagacaattccaagaacacgctgtatcttcaaatgaacagcctgagagccgaggacacggccgtgtattactgtgcgagagatctacgcggagaagtctggggccaagggacaatggtcaccgtctcttcag

SEQ ID NO: 202 - protein, 114 aa, Homo sapiens
EVQLVESGGGLIQPGGSLRLSCAASGLTVSRNYMSWVRQAPGKGLEWVSLIYSGGSTYYADSVKGRFTISRDNSKNTLYLQMNSLRAEDTAVYYCARDLRGEVWGQGTMVTVSS

SEQ ID NO: 203 - DNA, 322 bp, Homo sapiens
  source 1..322: mol_type = other DNA
gccatccagatgacccagtctccatcctccctgtctgcatctgtaggagacagagtcaccatcacttgccaggcgagtcaggacattagcaactttttaaattggtatcagcagaaaccagggaaagcccctaagctcctgatctacgatgcatccaatttggaaacaggggtcccatcaaggttcagtggaagtggatctgggacagattttactttcaccatcagtagcctgcagcctgaagatattgcaacatattactgtcaccagtatgataatctccctcgaacgttcggccaagggaccaaagtggatatcaaac

SEQ ID NO: 204 - protein, 107 aa, Homo sapiens
AIQMTQSPSSLSASVGDRVTITCQASQDISNFLNWYQQKPGKAPKLLIYDASNLETGVPSRFSGSGSGTDFTFTISSLQPEDIATYYCHQYDNLPRTFGQGTKVDIK

SEQ ID NO: 205 - protein, 8 aa, Homo sapiens
GLTVSRNY

SEQ ID NO: 206 - protein, 7 aa, Homo sapiens
IYSGGST

SEQ ID NO: 207 - protein, 8 aa, Homo sapiens
ARDLRGEV

SEQ ID NO: 208 - protein, 6 aa, Homo sapiens
QDISNF

SEQ ID NO: 209 - skipped

SEQ ID NO: 210 - protein, 9 aa, Homo sapiens
HQYDNLPRT

SEQ ID NO: 211 - DNA, 372 bp, Homo sapiens
  source 1..372: mol_type = other DNA
gaggtgcagctggtggagtctgggggaggcttggtacagcctggggggtccctgagactctcctgtgcagcctctggattcaccttcagtaactacgacatgcactgggtccgccaagctacaggaaaaggtctggagtgggtctcacttattggtactgctggtgacacatactatccagactccgtgaagggccgattcaccatctccagagaaaatgccaagaactccttgtatcttcaaatgaacagcctgagagccggggacacggctgtgtattactgtgcaagagggcaacacactcaaatcggtcactactactactactacatggacgtctggggcaaagggaccacggtcaccgtctcctca

SEQ ID NO: 212 - protein, 124 aa, Homo sapiens
EVQLVESGGGLVQPGGSLRLSCAASGFTFSNYDMHWVRQATGKGLEWVSLIGTAGDTYYPDSVKGRFTISRENAKNSLYLQMNSLRAGDTAVYYCARGQHTQIGHYYYYYMDVWGKGTTVTVSS

SEQ ID NO: 213 - DNA, 328 bp, Homo sapiens
  source 1..328: mol_type = other DNA
gccatccggatgacccagtctccatcgtccctgtctgcatctgtaggagacagagtcaccatcacttgccgggcaagtcagagcattagcagctatttaaattggtatcagcagaaaccagggaaagcccctaagctcctgatctttgctgcatccagtttgcaaagtggggtcccatcaaggttcagtggcagtggatctgggacagattccactctaaccatcagcagtctgcaacctgaagattttgcaacttactactgtcaacagagttacagtaaccctccggagggcagttttggccaggggaccaaagtggagattaaac

SEQ ID NO: 214 - protein, 109 aa, Homo sapiens
AIRMTQSPSSLSASVGDRVTITCRASQSISSYLNWYQQKPGKAPKLLIFAASSLQSGVPSRFSGSGSGTDSTLTISSLQPEDFATYYCQQSYSNPPEGSFGQGTKVEIK

SEQ ID NO: 215 - protein, 8 aa, Homo sapiens
GFTFSNYD

SEQ ID NO: 216 - protein, 7 aa, Homo sapiens
IGTAGDT

SEQ ID NO: 217 - protein, 18 aa, Homo sapiens
ARGQHTQIGHYYYYYMDV

SEQ ID NO: 218 - protein, 6 aa, Homo sapiens
QSISSY

SEQ ID NO: 219 - skipped

SEQ ID NO: 220 - protein, 11 aa, Homo sapiens
QQSYSNPPEGS

SEQ ID NO: 221 - DNA, 361 bp, Homo sapiens
  source 1..361: mol_type = other DNA
gaagtgcagctggtggagactggaggaggcttgatccagcctggggggtccctgagactctcctgtgcagcctctgggttcaccgtcagtagcaactacatgagctgggtccgccaggctccagggaaggggctggagtgggtctcagttgtttatggcggtggtaccacatactacgcagactccgtgaagggccgattcaccatctccagagacaattccaagaacacgctgtatcttcaaatgaacagcctgagagccgaggacacggccgtatattactgtgcgactgacaatggatacagctatggtttttcatttgactactggggccagggaaccctggtcatcgtctcctcag

SEQ ID NO: 222 - protein, 120 aa, Homo sapiens
EVQLVETGGGLIQPGGSLRLSCAASGFTVSSNYMSWVRQAPGKGLEWVSVVYGGGTTYYADSVKGRFTISRDNSKNTLYLQMNSLRAEDTAVYYCATDNGYSYGFSFDYWGQGTLVIVSS

SEQ ID NO: 223 - DNA, 331 bp, Homo sapiens
  source 1..331: mol_type = other DNA
cagtctgtgctgactcagcctgcctccatgtctgggtctcctggacagtcgatcaccatctcctgcactggaaccagcagtgatgttgggggttataaccttgtctcctggtaccaacagcacccaggcaaagcccccaaactcatgatttatgagggcagtaagcggccctcaggggtttctaatcgcttctctggctccaagtctggcaacacggcctccctgacaatctctgggctccaggctgaggacgaggctgattattactgctgctcatatgcaggtagtagtaattgggtgttcggcggagggaccaagctgaccgtcctag

SEQ ID NO: 224 - protein, 110 aa, Homo sapiens
QSVLTQPASMSGSPGQSITISCTGTSSDVGGYNLVSWYQQHPGKAPKLMIYEGSKRPSGVSNRFSGSKSGNTASLTISGLQAEDEADYYCCSYAGSSNWVFGGGTKLTVL

SEQ ID NO: 225 - protein, 8 aa, Homo sapiens
GFTVSSNY

SEQ ID NO: 226 - protein, 7 aa, Homo sapiens
VYGGGTT

SEQ ID NO: 227 - protein, 14 aa, Homo sapiens
ATDNGYSYGFSFDY

SEQ ID NO: 228 - protein, 9 aa, Homo sapiens
SSDVGGYNL

SEQ ID NO: 229 - skipped

SEQ ID NO: 230 - protein, 10 aa, Homo sapiens
CSYAGSSNWV

SEQ ID NO: 231 - DNA, 373 bp, Homo sapiens
  source 1..373: mol_type = other DNA
caggtgcagctggtggagtctggggctgaggtggagaagcctggggcctcagtgaaggtctcctgcaaggcttctggatacaccttcaccggctactatatgcactgggtgcgacaggcccctggacaagggcttgagtggatgggatggatcaaccctatcagtggtggcacaaactatgcacagaagtttcagggcagggtcaccatgaccagggacacgtccatcagcacagcctacatggacctgagcaggctgagatctgacgacacggccgtgtattactgtgcgagaggaacgtattactatgatagtagtggttacatcccatttgactactggggccagggaaccctggtcaccgtctcctcag

SEQ ID NO: 232 - protein, 124 aa, Homo sapiens
QVQLVESGAEVEKPGASVKVSCKASGYTFTGYYMHWVRQAPGQGLEWMGWINPISGGTNYAQKFQGRVTMTRDTSISTAYMDLSRLRSDDTAVYYCARGTYYYDSSGYIPFDYWGQGTLVTVSS

SEQ ID NO: 233 - DNA, 331 bp, Homo sapiens
  source 1..331: mol_type = other DNA
cagtctgtgctgactcagcctgcctccgtatctgggtctcctggacagtcgatcaccatctcctgcactggaaccagcagtgatgttgggagttataaccttgtctcctggtaccaacagcacccaggcaaagcccccaaactcatgatttatgagggcagtaagcggccctcaggggtttctaatcgcttctctggctccaagtctggcaacacggcctccctgacaatctctgggctccaggctgaggacgaggctgattattactgctgctcatatgcaggtagtagcactttggtattcggcggagggaccaagctgaccgtcctag

SEQ ID NO: 234 - protein, 110 aa, Homo sapiens
QSVLTQPASVSGSPGQSITISCTGTSSDVGSYNLVSWYQQHPGKAPKLMIYEGSKRPSGVSNRFSGSKSGNTASLTISGLQAEDEADYYCCSYAGSSTLVFGGGTKLTVL

SEQ ID NO: 235 - protein, 8 aa, Homo sapiens
GYTFTGYY

SEQ ID NO: 236 - protein, 8 aa, Homo sapiens
INPISGGT

SEQ ID NO: 237 - protein, 17 aa, Homo sapiens
ARGTYYYDSSGYIPFDY

SEQ ID NO: 238 - protein, 9 aa, Homo sapiens
SSDVGSYNL

SEQ ID NO: 239 - skipped

SEQ ID NO: 240 - protein, 10 aa, Homo sapiens
CSYAGSSTLV

SEQ ID NO: 241 - DNA, 385 bp, Homo sapiens
  source 1..385: mol_type = other DNA
caggttcagctggtgcagtctgggtctgagttgaagaagcctggggcctcagtgaaggtttcctgcaaggcttctggatacaccttcagtagctatgctatgacttgggtgcgacaggcccctggacaagggcttgagtggatgggatggatcaacaccaacactgggaacccaacgtatgcccagggcttcacaggacggtttgtcttctccttggacacctctgtcagcacggcatatctgcagatcagcagcctaaaggctgaggacactgccgtgtattactgtgcgagagctctgggatattgtagtagtaccagctgctatcccgcttgggctgcttttgatatctggggccaagggacaatggtcaccgtctcttcag

SEQ ID NO: 242 - protein, 128 aa, Homo sapiens
QVQLVQSGSELKKPGASVKVSCKASGYTFSSYAMTWVRQAPGQGLEWMGWINTNTGNPTYAQGFTGRFVFSLDTSVSTAYLQISSLKAEDTAVYYCARALGYCSSTSCYPAWAAFDIWGQGTMVTVSS

SEQ ID NO: 243 - DNA, 316 bp, Homo sapiens
  source 1..316: mol_type = other DNA
tcctatgagctgactcagccactctcagtgtcagtggccctgggacagacggccagtattacctgtgggggaaacaacattggaagtaaaaatgtgcactggtaccagcagaagccaggccaggcccctgtgctggtcatctatagggatagcaaccggccctctgggatccctgagcgattctctggctccaactcggggaacacggccaccctgaccatcagcagagcccaagccggggatgaggctgactataactgtcaggtgtgggacagcagcgtggtattcggcggagggaccaagctgaccgtcctag

SEQ ID NO: 244 - protein, 105 aa, Homo sapiens
SYELTQPLSVSVALGQTASITCGGNNIGSKNVHWYQQKPGQAPVLVIYRDSNRPSGIPERFSGSNSGNTATLTISRAQAGDEADYNCQVWDSSVVFGGGTKLTVL

SEQ ID NO: 245 - protein, 8 aa, Homo sapiens
GYTFSSYA

SEQ ID NO: 246 - protein, 8 aa, Homo sapiens
INTNTGNP

SEQ ID NO: 247 - protein, 21 aa, Homo sapiens
ARALGYCSSTSCYPAWAAFDI

SEQ ID NO: 248 - protein, 6 aa, Homo sapiens
NIGSKN

SEQ ID NO: 249 - skipped

SEQ ID NO: 250 - protein, 8 aa, Homo sapiens
QVWDSSVV

SEQ ID NO: 251 - DNA, 358 bp, Homo sapiens
  source 1..358: mol_type = other DNA
gaggtgcagctggtggagtctggaggaggcttgatccagccgggggggtccctgagactctcctgtgcagcctctgggctcaccgtcagtagcaactacatgagttgggtccgccaggctccagggaaggggctggagtgggtctcagttatttatagtggtggtagcacgttctacgcagactccgtgaagggccgattcaccatctccagagacaattccaagaacacgctgtatcttcaaatgaacagcctgggagccgaggacacggccgtgtattactgtgcgagaggagaaggtagtcctggaaactggttcgacccctggggccagggaaccctggtcaccgtctcctcag

SEQ ID NO: 252 - protein, 119 aa, Homo sapiens
EVQLVESGGGLIQPGGSLRLSCAASGLTVSSNYMSWVRQAPGKGLEWVSVIYSGGSTFYADSVKGRFTISRDNSKNTLYLQMNSLGAEDTAVYYCARGEGSPGNWFDPWGQGTLVTVSS

SEQ ID NO: 253 - DNA, 322 bp, Homo sapiens
  source 1..322: mol_type = other DNA
gatgttgtgatgactcagtctccaggcaccctgtctttgtctccaggggaaagagccaccctctcctgcagggccagtcagagtgttcccagcagctacttagcctggtaccagcagaaacctggccaggctcccaggctcctcatctatggtgcatccaccagggccactggcatcccagacaggttcagtggcagtgggtctgggacagacttcactctcaccatcagcagactggagcctgaggattttgcagtgtattactgtcagcactatgatacctcaccccgtttcggcggagggaccaaagtggatatcaaac

SEQ ID NO: 254 - protein, 107 aa, Homo sapiens
DVVMTQSPGTLSLSPGERATLSCRASQSVPSSYLAWYQQKPGQAPRLLIYGASTRATGIPDRFSGSGSGTDFTLTISRLEPEDFAVYYCQHYDTSPRFGGGTKVDIK

SEQ ID NO: 255 - protein, 8 aa, Homo sapiens
GLTVSSNY

SEQ ID NO: 256 - protein, 7 aa, Homo sapiens
IYSGGST

SEQ ID NO: 257 - protein, 13 aa, Homo sapiens
ARGEGSPGNWFDP

SEQ ID NO: 258 - protein, 7 aa, Homo sapiens
QSVPSSY

SEQ ID NO: 259 - skipped

SEQ ID NO: 260 - protein, 8 aa, Homo sapiens
QHYDTSPR

SEQ ID NO: 261 - DNA, 370 bp, Homo sapiens
  source 1..370: mol_type = other DNA
caggtccagctggtacagtctgggcctgaggtgaagaagcctgggacctcagtgaaggtctcctgcaaggcttctggattcacctttactacctctgctgtgcagtgggtgcgacaggctcgtggacaacgccttgagtggataggatggatcgtcgttggcagtggtaacacaaactacgcacagaagttccaggaaagagtcaccattaccagggacatgtccacaaccacagcctacatggagctgagcagcctgagatccgaggacacggccgtgtatttctgtgcggcgcctcattgtaatagtaccagctgctatgacgcttttgatatctggggccaagggacaatggtcaccgtctcttcag

SEQ ID NO: 262 - protein, 123 aa, Homo sapiens
QVQLVQSGPEVKKPGTSVKVSCKASGFTFTTSAVQWVRQARGQRLEWIGWIVVGSGNTNYAQKFQERVTITRDMSTTTAYMELSSLRSEDTAVYFCAAPHCNSTSCYDAFDIWGQGTMVTVSS

SEQ ID NO: 263 - DNA, 325 bp, Homo sapiens
  source 1..325: mol_type = other DNA
gacatccagatgacccagtctccaggcaccctgtctttgtctccaggggaaggagccaccctctcctgcagggccagtcagagtgttagcagcagctacttagcctggtaccagcagaaacctggccaggctcccaggctcctcatctatggtgcatctagtggggccactggcatcccagacagattcagtggcagtgggtctgggacagacttcactctcaccatcagcagactggagcctgaagattttgcagtgtattactgtcagcagtatggtagctcaccttacacttttggccaggggaccaaggtggaaatcaaac

SEQ ID NO: 264 - protein, 108 aa, Homo sapiens
DIQMTQSPGTLSLSPGEGATLSCRASQSVSSSYLAWYQQKPGQAPRLLIYGASSGATGIPDRFSGSGSGTDFTLTISRLEPEDFAVYYCQQYGSSPYTFGQGTKVEIK

SEQ ID NO: 265 - protein, 8 aa, Homo sapiens
GFTFTTSA

SEQ ID NO: 266 - protein, 8 aa, Homo sapiens
IVVGSGNT

SEQ ID NO: 267 - protein, 16 aa, Homo sapiens
AAPHCNSTSCYDAFDI

SEQ ID NO: 268 - protein, 7 aa, Homo sapiens
QSVSSSY

SEQ ID NO: 269 - skipped

SEQ ID NO: 270 - protein, 9 aa, Homo sapiens
QQYGSSPYT

SEQ ID NO: 271 - DNA, 352 bp, Homo sapiens
  source 1..352: mol_type = other DNA
caggtgcagctggtggagtctggaggaggcttgatccagcctggggggtccctgagactctcctgtgcagcctctgggctcaccgtcaataggaactacatgagctggatccgccaggctccagggaaggggctggagtgggtctcagttatttatagcggtggtagtacattttacgcagactccgtgaagggccgattcaccatctccagagacaattccaagaacacactgtctcttcaaatgaacagcctgagagccgaggacacggccatttattactgtgcgagagacttctacgagggttcttttgatatctggggccaagggacaatggtcaccgtctcttcag

SEQ ID NO: 272 - protein, 117 aa, Homo sapiens
QVQLVESGGGLIQPGGSLRLSCAASGLTVNRNYMSWIRQAPGKGLEWVSVIYSGGSTFYADSVKGRFTISRDNSKNTLSLQMNSLRAEDTAIYYCARDFYEGSFDIWGQGTMVTVSS

SEQ ID NO: 273 - DNA, 325 bp, Homo sapiens
  source 1..325: mol_type = other DNA
gccatccagttgacccagtctccttccttcctgtctgcatctataggagacagagtcaccatcacttgccgggccagtcagggcattagcagttatttagcctggtatcagcaaaaaccagggaaagcccctaagctcctgatctatgctgcatccactttgcaaagtggggtcccatcaaggttcagcggcagtggatctgggacagaattcactctcacaatcagcagcctgcagcctgaagattttgcatcttattactgtcaacagcttaatagttaccccgctccggttttcggccctgggaccaaagtggatatcaaac

SEQ ID NO: 274 - protein, 108 aa, Homo sapiens
AIQLTQSPSFLSASIGDRVTITCRASQGISSYLAWYQQKPGKAPKLLIYAASTLQSGVPSRFSGSGSGTEFTLTISSLQPEDFASYYCQQLNSYPAPVFGPGTKVDIK

SEQ ID NO: 275 - protein, 8 aa, Homo sapiens
GLTVNRNY

SEQ ID NO: 276 - protein, 7 aa, Homo sapiens
IYSGGST

SEQ ID NO: 277 - protein, 11 aa, Homo sapiens
ARDFYEGSFDI

SEQ ID NO: 278 - protein, 6 aa, Homo sapiens
QGISSY

SEQ ID NO: 279 - skipped

SEQ ID NO: 280 - protein, 10 aa, Homo sapiens
QQLNSYPAPV

SEQ ID NO: 281 - DNA, 370 bp, Homo sapiens
  source 1..370: mol_type = other DNA
caggtacagctggtgcagtctggggctgaggtgaagaagcctggggcctcagtgaaggtctcctgcaaggcttctggttacatctttatcagatatggtattagctgggtgcgacaggcccctggacaagggcttgagtggatgggatggatcagcgctaacaatggttacacaaactatgcacagaagctccagggcagagtcaccatgaccacagacacatccacgagcacagcctacatggagctgaggagcctgagatctgacgacacggccgtgtattactgtgcgagagatgggggtattttgactggttatctcgactactttgaccactggggccagggaaccctggtcaccgtctcctcag

SEQ ID NO: 282 - protein, 123 aa, Homo sapiens
QVQLVQSGAEVKKPGASVKVSCKASGYIFIRYGISWVRQAPGQGLEWMGWISANNGYTNYAQKLQGRVTMTTDTSTSTAYMELRSLRSDDTAVYYCARDGGILTGYLDYFDHWGQGTLVTVSS

SEQ ID NO: 283 - DNA, 325 bp, Homo sapiens
  source 1..325: mol_type = other DNA
gacatccagatgacccagtctccatcctccctgtctgcatctgtaggagacagactcaccatcacttgccgggcaagtcagagcattgccagctatttaaattggtatcagcagaaaccagggaaagcccctaagctcctgatctatgctgcatccagtttgcaaagtggggtcccatcaaggttcagtggcagtggatctgggacagatttcactctcaccatcagcagtctgcaacctgaagattttgcaacttaccactgtcaacagagttacagtaccctcggaatcactttcggccctgggaccaaagtggatatcaaac

SEQ ID NO: 284 - protein, 108 aa, Homo sapiens
DIQMTQSPSSLSASVGDRLTITCRASQSIASYLNWYQQKPGKAPKLLIYAASSLQSGVPSRFSGSGSGTDFTLTISSLQPEDFATYHCQQSYSTLGITFGPGTKVDIK

SEQ ID NO: 285 - protein, 8 aa, Homo sapiens
GYIFIRYG

SEQ ID NO: 286 - protein, 8 aa, Homo sapiens
ISANNGYT

SEQ ID NO: 287 - protein, 16 aa, Homo sapiens
ARDGGILTGYLDYFDH

SEQ ID NO: 288 - protein, 6 aa, Homo sapiens
QSIASY

SEQ ID NO: 289 - skipped

SEQ ID NO: 290 - protein, 10 aa, Homo sapiens
QQSYSTLGIT

SEQ ID NO: 291 - DNA, 367 bp, Homo sapiens
  source 1..367: mol_type = other DNA
caggtgcagctggtggagtctgggggaggcttggtccagcctggggggtccctgagactctcctgtgcagcctctggattcccctttagtatctattggatgagctgggtccgccaggctccagggaaggggctggagtgggtggccaacataaagcaagatggaagtgagaaatactatgtggactctgtgaagggccgattcaccatctccagagacaacgccaagaactcactgtatctgcacatgaacagcctgagaggcgaggacacggctgtgtattactgtgcgagccgatattacgattttcgaccggaggcttggtttgactactggggccagggaaccctggtcaccgtctcctcag

SEQ ID NO: 292 - protein, 122 aa, Homo sapiens
QVQLVESGGGLVQPGGSLRLSCAASGFPFSIYWMSWVRQAPGKGLEWVANIKQDGSEKYYVDSVKGRFTISRDNAKNSLYLHMNSLRGEDTAVYYCASRYYDFRPEAWFDYWGQGTLVTVSS

SEQ ID NO: 293 - DNA, 343 bp, Homo sapiens
  source 1..343: mol_type = other DNA
gatattgtgatgacccagactccactctcctcacctgtcacccttggacagccggcctccatctcctgcaggtctagtcaaagcctcgtacacagggatggaaacacctacttgagctggcttcagcagaggccaggccagcctccaagactcctaatttataagatttctaaccggttctctggggtcccagacagattcagtggcagtggggcagggacagatttcacactgaaaatcagcagggtggaagctgaggatgtcggggtttattactgcatgcaagctacacaatttcctcatgggtacacttttggccaggggaccaaggtggagatcaaac

SEQ ID NO: 294 - protein, 114 aa, Homo sapiens
DIVMTQTPLSSPVTLGQPASISCRSSQSLVHRDGNTYLSWLQQRPGQPPRLLIYKISNRFSGVPDRFSGSGAGTDFTLKISRVEAEDVGVYYCMQATQFPHGYTFGQGTKVEIK

SEQ ID NO: 295 - protein, 8 aa, Homo sapiens
GFPFSIYW

SEQ ID NO: 296 - protein, 8 aa, Homo sapiens
IKQDGSEK

SEQ ID NO: 297 - protein, 15 aa, Homo sapiens
ASRYYDFRPEAWFDY

SEQ ID NO: 298 - protein, 11 aa, Homo sapiens
QSLVHRDGNTY

SEQ ID NO: 299 - skipped

SEQ ID NO: 300 - protein, 11 aa, Homo sapiens
MQATQFPHGYT

SEQ ID NO: 301 - DNA, 355 bp, Homo sapiens
  source 1..355: mol_type = other DNA
caggtgcagctgcaggagtctgggggaggcttggtccagcctggggggtccctgagactctcctgttcagcctctggattcaccgtcagtagcaactacatgacctgggtccgccaggctccagggaaggggctggagtgggtctcagttatttatagcggtggtagcacattctacgcagactccgtgaagggcagattcaccatctccagagacaattccaagaacacgctgtatcttcaaatgaacagcctgagagccgaggacaccgctgtgtattactgtgcgagagatctggaagaggccgggggatttgactactggggccagggaaccctggtcaccgtctcctcag

SEQ ID NO: 302 - protein, 118 aa, Homo sapiens
QVQLQESGGGLVQPGGSLRLSCSASGFTVSSNYMTWVRQAPGKGLEWVSVIYSGGSTFYADSVKGRFTISRDNSKNTLYLQMNSLRAEDTAVYYCARDLEEAGGFDYWGQGTLVTVSS

SEQ ID NO: 303 - DNA, 325 bp, Homo sapiens
  source 1..325: mol_type = other DNA
gaaattgtgttgacgcagtctccaggcaccctgtctttgtctccaggggaaaaagtcaccctctcctgcagggccagtcagagtgttagcagcacctacttagcctggtaccagcagaaacctggccaggctcccaggctcctcatctatggtgcatccagcagggccactggcgtcccagacaggttccgtggcagtgggtctgggacagacttcactctcaccatcagcagactggagcctgaagattttgcagtgtattactgtcagcagtatggtagctcgctgtacacttttggccaggggaccaaagtggatatcaaac

SEQ ID NO: 304 - protein, 108 aa, Homo sapiens
EIVLTQSPGTLSLSPGEKVTLSCRASQSVSSTYLAWYQQKPGQAPRLLIYGASSRATGVPDRFRGSGSGTDFTLTISRLEPEDFAVYYCQQYGSSLYTFGQGTKVDIK

SEQ ID NO: 305 - protein, 8 aa, Homo sapiens
GFTVSSNY

SEQ ID NO: 306 - protein, 7 aa, Homo sapiens
IYSGGST

SEQ ID NO: 307 - protein, 12 aa, Homo sapiens
ARDLEEAGGFDY

SEQ ID NO: 308 - protein, 7 aa, Homo sapiens
QSVSSTY

SEQ ID NO: 309 - skipped

SEQ ID NO: 310 - protein, 9 aa, Homo sapiens
QQYGSSLYT

SEQ ID NO: 311 - DNA, 385 bp, Homo sapiens
  source 1..385: mol_type = other DNA
cagctgcagctgcaggagtcgggcccaggactggtgaagccttcggagaccctgtccctcacctgcactgtctccggtgactccgtcagtaattactactggagctggatccggcagcccgccgggaagggactggagtggattgggcgtatctataccagtgggagcaccaactacaacccctccctcaagagtcgagtcaccatgtcagtagacacgtccaagaaccagttctccctgaagctgagctctgtgaccgccgcggacacggccgtgtattactgtgcgagagatcaccgggcttcccggtatagcagtggctggtacgaatggtggaactgcttcgacccctggggccagggaaccctggtcaccgtctcctcag

SEQ ID NO: 312 - protein, 128 aa, Homo sapiens
QLQLQESGPGLVKPSETLSLTCTVSGDSVSNYYWSWIRQPAGKGLEWIGRIYTSGSTNYNPSLKSRVTMSVDTSKNQFSLKLSSVTAADTAVYYCARDHRASRYSSGWYEWWNCFDPWGQGTLVTVSS

SEQ ID NO: 313 - DNA, 325 bp, Homo sapiens
  source 1..325: mol_type = other DNA
gacatccagatgacccagtctccatcctccctgtctgcatctgtaggagacagagtcaccatcacttgccgggcaagtcagagcattagcagctatttaaattggtatcagcagaaaccagggaaagcccctaagctcctgatctatgctgcatccagtttgcaaagtggggtcccgtcaaggttcagtggcagtggatctgggacagatttcactctcaccatcaacagtctgcaacctgaagattttgcaacttactactgtcaacagagttacagtacccccgcgctcactttcggcggagggaccaaagtggatatcaaac

SEQ ID NO: 314 - protein, 108 aa, Homo sapiens
DIQMTQSPSSLSASVGDRVTITCRASQSISSYLNWYQQKPGKAPKLLIYAASSLQSGVPSRFSGSGSGTDFTLTINSLQPEDFATYYCQQSYSTPALTFGGGTKVDIK

SEQ ID NO: 315 - protein, 8 aa, Homo sapiens
GDSVSNYY

SEQ ID NO: 316 - protein, 7 aa, Homo sapiens
IYTSGST

SEQ ID NO: 317 - protein, 22 aa, Homo sapiens
ARDHRASRYSSGWYEWWNCFDP

SEQ ID NO: 318 - protein, 6 aa, Homo sapiens
QSISSY

SEQ ID NO: 319 - skipped

SEQ ID NO: 320 - protein, 10 aa, Homo sapiens
QQSYSTPALT

SEQ ID NO: 321 - DNA, 367 bp, Homo sapiens
  source 1..367: mol_type = other DNA
caggttcagctggtgcagtctggggctgaggtgaagaagcctggggcctcagtgaaggtctcctgcaaggcttctggatacaccttcaccggctactatatgcactgggtgcgacaggcccctggacaagggcttgagtggatgggatggatcaaccctaacagtggtggcacaaactatacacagaagtttcagggcagggtcaccatgaccagggacacgtccatcagcacagcctacatggagctgagcaggctgagatctgacgacacggccgtgtattcctgtgcgagagatatggcgtttagtatggttcggggttcctttgactactggggccagggaaccctggtcaccgtctcctcag

SEQ ID NO: 322 - protein, 122 aa, Homo sapiens
QVQLVQSGAEVKKPGASVKVSCKASGYTFTGYYMHWVRQAPGQGLEWMGWINPNSGGTNYTQKFQGRVTMTRDTSISTAYMELSRLRSDDTAVYSCARDMAFSMVRGSFDYWGQGTLVTVSS

SEQ ID NO: 323 - DNA, 331 bp, Homo sapiens
  source 1..331: mol_type = other DNA
caggctgtgctgactcagcctccctccgcgtccgggtctcctggacagtcagtcaccatctcctgcactggaaccagcagtgacgttggtggttataactatgtctcctggtaccaacagcacccaggcaaagcccccaaactcatgatttatgaggtcagtaagcggccctcaggggtccctgatcgcttctctggctccaagtctggcaacacggcctccctgaccgtctctgggctccaggctgaggatgaggctgattattactgcagctcatatgcaggcagcaaccattgggtgttcggcggagggaccaagctgaccgtcctag

SEQ ID NO: 324 - protein, 110 aa, Homo sapiens
QAVLTQPPSASGSPGQSVTISCTGTSSDVGGYNYVSWYQQHPGKAPKLMIYEVSKRPSGVPDRFSGSKSGNTASLTVSGLQAEDEADYYCSSYAGSNHWVFGGGTKLTVL

SEQ ID NO: 325 - protein, 8 aa, Homo sapiens
GYTFTGYY

SEQ ID NO: 326 - protein, 8 aa, Homo sapiens
INPNSGGT

SEQ ID NO: 327 - protein, 15 aa, Homo sapiens
ARDMAFSMVRGSFDY

SEQ ID NO: 328 - protein, 9 aa, Homo sapiens
SSDVGGYNY

SEQ ID NO: 329 - skipped

SEQ ID NO: 330 - protein, 10 aa, Homo sapiens
SSYAGSNHWV

SEQ ID NO: 331 - DNA, 358 bp, Homo sapiens
  source 1..358: mol_type = other DNA
caggtgcagctggtgcagtctgggcctgaggtgaagaagcctgggacctcagtgaaggtctcctgcaaggcgtctggattcacccttactagctctgctatgcagtgggtgcgacaggctcgtggacaacgccttgagtggataggatggatcgtcgttggcagtggcaacacaaactacgcacagaagttccaggaaagagtcaccattaccagggacatgtccacaagcacagcctacatggagctgagcagcctgagatccgaggacacggccgtgtattattgtgcggccggccgtggctacaattcggactttgactactggggccagggaaccctggtcaccgtctcctcag

SEQ ID NO: 332 - protein, 119 aa, Homo sapiens
QVQLVQSGPEVKKPGTSVKVSCKASGFTLTSSAMQWVRQARGQRLEWIGWIVVGSGNTNYAQKFQERVTITRDMSTSTAYMELSSLRSEDTAVYYCAAGRGYNSDFDYWGQGTLVTVSS

SEQ ID NO: 333 - DNA, 325 bp, Homo sapiens
  source 1..325: mol_type = other DNA
gccatccggatgacccagtctccaggcaccctgtctttgtctccaggggaaagagccaccctctcctgcagggccagtcagagtgttagcagcagctacttagcctggtaccagcagagacctggccaggctcccaggctcctcatctatggtacatccagcagggccactggcatcccagacaggttcagtggcagtgggtctgggacagacttcactctcaccatcagcagactggagcctgaagattttgcagtgtattactgtcagcagtatggttactcagtgtacacttttggccaggggaccaaagtggatatcaaac

SEQ ID NO: 334 - protein, 108 aa, Homo sapiens
AIRMTQSPGTLSLSPGERATLSCRASQSVSSSYLAWYQQRPGQAPRLLIYGTSSRATGIPDRFSGSGSGTDFTLTISRLEPEDFAVYYCQQYGYSVYTFGQGTKVDIK

SEQ ID NO: 335 - protein, 8 aa, Homo sapiens
GFTLTSSA

SEQ ID NO: 336 - protein, 8 aa, Homo sapiens
IVVGSGNT

SEQ ID NO: 337 - protein, 12 aa, Homo sapiens
AAGRGYNSDFDY

SEQ ID NO: 338 - protein, 7 aa, Homo sapiens
QSVSSSY

SEQ ID NO: 339 - skipped

SEQ ID NO: 340 - protein, 9 aa, Homo sapiens
QQYGYSVYT

SEQ ID NO: 341 - DNA, 367 bp, Homo sapiens
  source 1..367: mol_type = other DNA
caggtgcagctggtggagtctgaggctgaggtgaagaagcctggggcctcagtgaaggtttcctgcaaggcatctggatacaccttcaccagctactatatgcactgggtgcgacaggcccctggacaagggcttcagtggatgggaataatcaaccctagtgctggtagcacaagctacgcacagaagttccagggcagagtcaccatgaccacggacacgtccacgaccacagtctacatggagctgagcagcctgagatctgaggacacggccgtgtattactgtgcgagagattctgtactagtaccagctgctaatgcttttgatatctggggccaagggacaatggtcaccgtctcttcag

SEQ ID NO: 342 - protein, 122 aa, Homo sapiens
QVQLVESEAEVKKPGASVKVSCKASGYTFTSYYMHWVRQAPGQGLQWMGIINPSAGSTSYAQKFQGRVTMTTDTSTTTVYMELSSLRSEDTAVYYCARDSVLVPAANAFDIWGQGTMVTVSS

SEQ ID NO: 343 - DNA, 322 bp, Homo sapiens
  source 1..322: mol_type = other DNA
gaaatagtgatgacgcagtctccagccaccctgtctttgtctccaggggaaagagccaccctctcctgcagggccagtcagagtgttagtagctacttagcctggtaccaacagaaacctggccaggctcccaggctcctcatctatgatgcatccaacagggccactggcatcccagccaggttcagtggcagtgggtctgggacagacttcactctcaccatcagcagcctagagcctgaagattttgcagtttattactgtcagcagcgtcgcaactggctattcactttcggccctgggaccaaagtggatatcaaac

SEQ ID NO: 344 - protein, 107 aa, Homo sapiens
EIVMTQSPATLSLSPGERATLSCRASQSVSSYLAWYQQKPGQAPRLLIYDASNRATGIPARFSGSGSGTDFTLTISSLEPEDFAVYYCQQRRNWLFTFGPGTKVDIK

SEQ ID NO: 345 - protein, 8 aa, Homo sapiens
GYTFTSYY

SEQ ID NO: 346 - protein, 8 aa, Homo sapiens
INPSAGST

SEQ ID NO: 347 - protein, 15 aa, Homo sapiens
ARDSVLVPAANAFDI

SEQ ID NO: 348 - protein, 6 aa, Homo sapiens
QSVSSY

SEQ ID NO: 349 - skipped

SEQ ID NO: 350 - protein, 9 aa, Homo sapiens
QQRRNWLFT

SEQ ID NO: 351 - DNA, 358 bp, Homo sapiens
  source 1..358: mol_type = other DNA
caggtgcagctggtgcagtctggggctgaggtgaagaagcctggggcctcagtgaaggtttcctgcaaggcttctggagacaccttcactagctatactctgcattgggtgcgccaggcccccggacaaaggcttgagtggatgggatggatcaacgctggcaatggttacacaaaatattcacagaagttccagggcagagtcaccattaccagggacacatccgcgagcacagcctacatggagctgagcagcctgagatctgaagacacggctgtgtattactgtgcgaaatgtactatgatagtagactactttgactactggggccagggaaccctggtcaccgtctcctcag

SEQ ID NO: 352 - protein, 119 aa, Homo sapiens
QVQLVQSGAEVKKPGASVKVSCKASGDTFTSYTLHWVRQAPGQRLEWMGWINAGNGYTKYSQKFQGRVTITRDTSASTAYMELSSLRSEDTAVYYCAKCTMIVDYFDYWGQGTLVTVSS

SEQ ID NO: 353 - DNA, 322 bp, Homo sapiens
  source 1..322: mol_type = other DNA
gccatccggatgacccagtctccttccaccctgtctgcatctgtaggagacagagtcaccatcacttgccgggccagtcagagtattagtggctggttggcctggtatcagcagaaaccagagaaagcccctaagctcctgatctatgatgcctccaatttggaaagtggggtcccatcaaggttcagcggcagtggatctgggacagaattcactctcaccatcaacagcctgcagcctgatgattttgcaacttattactgccaacagtataatagttacccgtggacgttcggccaagggaccaaagtggatatcaaac

SEQ ID NO: 354 - protein, 107 aa, Homo sapiens
AIRMTQSPSTLSASVGDRVTITCRASQSISGWLAWYQQKPEKAPKLLIYDASNLESGVPSRFSGSGSGTEFTLTINSLQPDDFATYYCQQYNSYPWTFGQGTKVDIK

SEQ ID NO: 355 - protein, 8 aa, Homo sapiens
GDTFTSYT

SEQ ID NO: 356 - protein, 8 aa, Homo sapiens
INAGNGYT

SEQ ID NO: 357 - protein, 12 aa, Homo sapiens
AKCTMIVDYFDY

SEQ ID NO: 358 - protein, 6 aa, Homo sapiens
QSISGW

SEQ ID NO: 359 - skipped

SEQ ID NO: 360 - protein, 9 aa, Homo sapiens
QQYNSYPWT

SEQ ID NO: 361 - DNA, 357 bp, Homo sapiens
  source 1..357: mol_type = other DNA
gaggtgcagctggtgcagtctggggctgaggtgaagaagcctggggcctcagtgaaggtctcctgcaaggcttctgggtacaccttcaccagttatgatatcaactgggtgcgacaggccactggacaagggcttgagtggatgggatggatgaaccctcacagtgataccacaggctatgcacagaagttccagggcagagtcaccatgaccaggaacacctccataaccacagcctacatggagctgagcagcctgagatctgaggacacggccgtgtattactgtgctcagggacccatagcagtgaactacatggacgtctggggcaaagggaccacggtcaccgtctcctca

SEQ ID NO: 362 - protein, 119 aa, Homo sapiens
EVQLVQSGAEVKKPGASVKVSCKASGYTFTSYDINWVRQATGQGLEWMGWMNPHSDTTGYAQKFQGRVTMTRNTSITTAYMELSSLRSEDTAVYYCAQGPIAVNYMDVWGKGTTVTVSS

SEQ ID NO: 363 - DNA, 325 bp, Homo sapiens
  source 1..325: mol_type = other DNA
cagcctgtgctgactcagccaccctcagtgtcagtggccccaggaaagacggccaggattacctgtgggggaagcaacattggaagtaaaagtgtgcactggtaccagcagaagccaggccaggcccctgtgctgatcatctattatgatagcgaccggccctcagggatccctgagcgattctctggctccaactctgggaacacggccaccctgaccatcagcagggtcgaagccggggatgaggccgacttttactgtcaggtgtgggatagtagtactgatcatgtggtattcggcggggggaccaagctgaccgtcctag

SEQ ID NO: 364 - protein, 108 aa, Homo sapiens
QPVLTQPPSVSVAPGKTARITCGGSNIGSKSVHWYQQKPGQAPVLIIYYDSDRPSGIPERFSGSNSGNTATLTISRVEAGDEADFYCQVWDSSTDHVVFGGGTKLTVL

SEQ ID NO: 365 - protein, 8 aa, Homo sapiens
GYTFTSYD

SEQ ID NO: 366 - protein, 8 aa, Homo sapiens
MNPHSDTT

SEQ ID NO: 367 - protein, 12 aa, Homo sapiens
AQGPIAVNYMDV

SEQ ID NO: 368 - protein, 6 aa, Homo sapiens
NIGSKS

SEQ ID NO: 369 - skipped

SEQ ID NO: 370 - protein, 11 aa, Homo sapiens
QVWDSSTDHVV

SEQ ID NO: 371 - DNA, 376 bp, Homo sapiens
  source 1..376: mol_type = other DNA
gaggtgcagctggtggagtctgggggaggcttggtcaagcctggagagtccctgagactctcctgtgcagcctctggattcaccttcagtgactactacatgacctggatccgccaggctccagggaaggggctggagtgggtttcatacattaggagtagtggtcatactatatactacgcagactctgtgaagggccgattcaccatctccagggacaacgccaagaactcactgtatctacaaatgaacagcctgagagtcgaggacacggccgtgtattactgtgcgagaggaggggttttacgatttttggagtggcctctcaatgcttttgatatctggggccaagggacaatggtcaccgtctcttcag

SEQ ID NO: 372 - protein, 125 aa, Homo sapiens
EVQLVESGGGLVKPGESLRLSCAASGFTFSDYYMTWIRQAPGKGLEWVSYIRSSGHTIYYADSVKGRFTISRDNAKNSLYLQMNSLRVEDTAVYYCARGGVLRFLEWPLNAFDIWGQGTMVTVSS

SEQ ID NO: 373 - DNA, 322 bp, Homo sapiens
  source 1..322: mol_type = other DNA
gacatccagttgacccagtctccatcctccctgtctgcatctgtaggagacagagtcaccatcacttgccgggcgagtcagggcattagcaattatttagcctggtatcagcagaaaccagggaaagttcctaagctcctgatctatgctgcatccactttgcaatcaggggtcccatctcggttcagtggcagtggatctgggacagatttcactctcaccatcagcagcctgcagcctgaagatgttgcaacttattactgtcaaaagtataacaatgccctcgggacgttcggccaagggaccaaggtggagatcaaac

SEQ ID NO: 374 - protein, 107 aa, Homo sapiens
DIQLTQSPSSLSASVGDRVTITCRASQGISNYLAWYQQKPGKVPKLLIYAASTLQSGVPSRFSGSGSGTDFTLTISSLQPEDVATYYCQKYNNALGTFGQGTKVEIK

SEQ ID NO: 375 - protein, 8 aa, Homo sapiens
GFTFSDYY

SEQ ID NO: 376 - protein, 8 aa, Homo sapiens
IRSSGHTI

SEQ ID NO: 377 - protein, 18 aa, Homo sapiens
ARGGVLRFLEWPLNAFDI

SEQ ID NO: 378 - protein, 6 aa, Homo sapiens
QGISNY

SEQ ID NO: 379 - skipped

SEQ ID NO: 380 - protein, 9 aa, Homo sapiens
QKYNNALGT

SEQ ID NO: 381 - DNA, 364 bp, Homo sapiens
  source 1..364: mol_type = other DNA
gaggtgcagctggtgcagtctggggctgaggtgaagaagcctggggcctcagtgaaggtctcctgcaaggcttctggatacaccttcaccggctactatatgcactgggtgcgacaggcccctggacaagggcttgagtggatgggatggatcagccctaacagtggtggcacaaactatgcacagaagtttcagggcagggtcaccatgaccagggacacgtccatcaccacagcctacatggacctgagcaggctgagatctgacgacacggccgtgtattactgtgcgagaggttattactatgaagccctcgatgcttttgatatctggggccaagggacaatggtcaccgtctcttcag

SEQ ID NO: 382 - protein, 121 aa, Homo sapiens
EVQLVQSGAEVKKPGASVKVSCKASGYTFTGYYMHWVRQAPGQGLEWMGWISPNSGGTNYAQKFQGRVTMTRDTSITTAYMDLSRLRSDDTAVYYCARGYYYEALDAFDIWGQGTMVTVSS

SEQ ID NO: 383 - DNA, 331 bp, Homo sapiens
  source 1..331: mol_type = other DNA
cagtctgtcgtgacgcagcctgcctccgtgtctgggtctcctggacagtcgatcaccatctcctgcactggaaccagcagtgacgttggtggttataactttgtctcctggtaccaacagcacccaggcaaagcccccaaactcatgatttatgaggtcagtaatcggccctcaggggtttctaatcgcttctctggctccaagtctggcatcacggcctccctgaccatctctgggctccaggctgaggacgaggctgattattactgcaactcatatacaagcaacagtactcgggtattcggcggagggaccaagctgaccgtcctag

SEQ ID NO: 384 - protein, 110 aa, Homo sapiens
QSVVTQPASVSGSPGQSITISCTGTSSDVGGYNFVSWYQQHPGKAPKLMIYEVSNRPSGVSNRFSGSKSGITASLTISGLQAEDEADYYCNSYTSNSTRVFGGGTKLTVL

SEQ ID NO: 385 - protein, 8 aa, Homo sapiens
GYTFTGYY

SEQ ID NO: 386 - protein, 8 aa, Homo sapiens
ISPNSGGT

SEQ ID NO: 387 - protein, 14 aa, Homo sapiens
ARGYYYEALDAFDI

SEQ ID NO: 388 - protein, 9 aa, Homo sapiens
SSDVGGYNF

SEQ ID NO: 389 - skipped

SEQ ID NO: 390 - protein, 10 aa, Homo sapiens
NSYTSNSTRV

SEQ ID NO: 391 - DNA, 382 bp, Homo sapiens
  source 1..382: mol_type = other DNA
caggtgcagctggtggagtctgggggaggcttggtccagcctggggggtccctgagactctcctgtgcagcctctggattcaccgtcagtagcaactacatgacctgggtccgccaggctccagggaaggggctggagtgggtctcagttatttatagcggtggtagcacatactacgcagactccgtgaagggcagattcaccatctccagagacaattccaagaacacgctatatcttcaaatgaacagcctgagagccgacgacacggctgtatattactgtgcgagagactctacagccgattacgatttttggagtggttattatgtaggtgcttttcatatctggggccaagggacaatggtcaccgtctcttcag

SEQ ID NO: 392 - protein, 127 aa, Homo sapiens
QVQLVESGGGLVQPGGSLRLSCAASGFTVSSNYMTWVRQAPGKGLEWVSVIYSGGSTYYADSVKGRFTISRDNSKNTLYLQMNSLRADDTAVYYCARDSTADYDFWSGYYVGAFHIWGQGTMVTVSS

SEQ ID NO: 393 - DNA, 331 bp, Homo sapiens
  source 1..331: mol_type = other DNA
cagactgtgctgactcagcctgcctccgtgtctgggtctcctggacagtcgatcaccatctcctgcactggaaccagcagtgacgttggtggttacaactatgtctcctggtaccaacagcacccaggcaaagcccccaaactcatgatttatgaggtcactaagcggccctcaggggtccctgatcgcttctctggctccaagtctggcaacacggcctccctgaccgtctctgggctccaggctgaggatgaggctgattattactgcagctcatatgcaggcagcaacaattgggtgttcggcggagggaccaagctgaccgtcctag

SEQ ID NO: 394 - protein, 110 aa, Homo sapiens
QTVLTQPASVSGSPGQSITISCTGTSSDVGGYNYVSWYQQHPGKAPKLMIYEVTKRPSGVPDRFSGSKSGNTASLTVSGLQAEDEADYYCSSYAGSNNWVFGGGTKLTVL

SEQ ID NO: 395 - protein, 8 aa, Homo sapiens
GFTVSSNY

SEQ ID NO: 396 - protein, 7 aa, Homo sapiens
IYSGGST

SEQ ID NO: 397 - protein, 21 aa, Homo sapiens
ARDSTADYDFWSGYYVGAFHI

SEQ ID NO: 398 - protein, 9 aa, Homo sapiens
SSDVGGYNY

SEQ ID NO: 399 - skipped

SEQ ID NO: 400 - protein, 10 aa, Homo sapiens
SSYAGSNNWV

SEQ ID NO: 401 - DNA, 370 bp, Homo sapiens
  source 1..370: mol_type = other DNA
gaggtgcagctggtggagtcgggcccaggactggtgaagccttcggagaccctgtccctcacctgcactgtctctggtgggtccatcagcagtagtagtcactactggggctggatccgccagcccccagggaaggggctggagtggattgggagtatttattatagtgagagtgcctactacaacccgtccctcaagagtcgagtcaccatgtcaatagacacgtccaagaaccagttctccctgaagctgaactctgtgaccgccgcggacacggccgtgtattactgtgcgagagtcactgagcctcggtggacttcttgttactttgactactggggccagggaaccctggtcaccgtctcctcag

SEQ ID NO: 402 - protein, 123 aa, Homo sapiens
EVQLVESGPGLVKPSETLSLTCTVSGGSISSSSHYWGWIRQPPGKGLEWIGSIYYSESAYYNPSLKSRVTMSIDTSKNQFSLKLNSVTAADTAVYYCARVTEPRWTSCYFDYWGQGTLVTVSS

SEQ ID NO: 403 - DNA, 325 bp, Homo sapiens
  source 1..325: mol_type = other DNA
gaaatagtgatgacgcagtctccagccaccctgtctttgtctccaggggaaagagccaccctctcctgcaggaccagtcagagtgttaccagctacttagcctggtaccaacagagacctggccaggctcccaggctcctcatctatgatgcatccgacagggccactggcatcccagccaggttcagtggcagtgggtctgggacagacttcactctcaccatcagcaacctagagcctgaagattttgcagtttattactgtcagctgcgtagcaactggcctccgatcaccttcggccaagggacacgactggagactaaac

SEQ ID NO: 404 - protein, 108 aa, Homo sapiens
EIVMTQSPATLSLSPGERATLSCRTSQSVTSYLAWYQQRPGQAPRLLIYDASDRATGIPARFSGSGSGTDFTLTISNLEPEDFAVYYCQLRSNWPPITFGQGTRLETK

SEQ ID NO: 405 - protein, 10 aa, Homo sapiens
GGSISSSSHY

SEQ ID NO: 406 - protein, 7 aa, Homo sapiens
IYYSESA

SEQ ID NO: 407 - protein, 15 aa, Homo sapiens
ARVTEPRWTSCYFDY

SEQ ID NO: 408 - protein, 6 aa, Homo sapiens
QSVTSY

SEQ ID NO: 409 - skipped

SEQ ID NO: 410 - protein, 10 aa, Homo sapiens
QLRSNWPPIT

SEQ ID NO: 411 - DNA, 370 bp, Homo sapiens
  source 1..370: mol_type = other DNA
gaagtgcagctggtggagtcgggcccaggactggtgaagccttcggagaccctgtccctcacctgcactgtctctgggggctccatcagcagtagtagttactactggggctggatccgccagcccccagggaaggggctggagtggattgggagtatctattatagtgggagcacctactacaacccgtccctcaagagtcgagtcaccatatcagtagacacgtccaagaaccagttctccctgaagctgagctctgtgaccgccgcggacacggccgtgtttttctgtgcgagagagaggagcgctcctctcgcgggcaactggttcgacccctggggccagggaaccctggtcaccgtctcttcag

SEQ ID NO: 412 - protein, 123 aa, Homo sapiens
EVQLVESGPGLVKPSETLSLTCTVSGGSISSSSYYWGWIRQPPGKGLEWIGSIYYSGSTYYNPSLKSRVTISVDTSKNQFSLKLSSVTAADTAVFFCARERSAPLAGNWFDPWGQGTLVTVSS

SEQ ID NO: 413 - DNA, 325 bp, Homo sapiens
  source 1..325: mol_type = other DNA
gacatccagatgacccagtctccatccttcctgtctgcatctgtaggagacagagtcaccatcacttgccgggccagtcagggcattagcagttatttagcctggtatcagcaaaaaccagggaaagcccctaagctcctgatctatgctgcatccactttgcaaagtggggtcccatcaaggttcagcggcagtggatctgggacagaattcactctcacaatcagcagcctgcagcctgaagattttgcaacttattactgtcaacagcttaatacttacccttcgatcaccttcggccaagggacacgactggagattaaac

SEQ ID NO: 414 - protein, 108 aa, Homo sapiens
DIQMTQSPSFLSASVGDRVTITCRASQGISSYLAWYQQKPGKAPKLLIYAASTLQSGVPSRFSGSGSGTEFTLTISSLQPEDFATYYCQQLNTYPSITFGQGTRLEIK

SEQ ID NO: 415 - protein, 10 aa, Homo sapiens
GGSISSSSYY

SEQ ID NO: 416 - protein, 7 aa, Homo sapiens
IYYSGST

SEQ ID NO: 417 - protein, 15 aa, Homo sapiens
ARERSAPLAGNWFDP

SEQ ID NO: 418 - protein, 6 aa, Homo sapiens
QGISSY

SEQ ID NO: 419 - skipped

SEQ ID NO: 420 - protein, 10 aa, Homo sapiens
QQLNTYPSIT

SEQ ID NO: 421 - DNA, 369 bp, Homo sapiens
  source 1..369: mol_type = other DNA
gaagtgcagctggtggagtctgggggaggcgtggtccagcctgggaggcccctgagactctcctgtgcagcctctggattccccttcagtaactatggcatgcactgggtccgccaggctccaggcaaggggctggaatgggtggcagttatatggtatgatggaagtaataaatactatgcagactccgtgaagggccgattcaccatctccagagacaattccaagaacacgctgtatctgcaaatgaacaacctgagagctgaggacacggctatatattactgtgcgaaagatgggtacacggcccactactactactactacatggacgtctggggcaaagggaccacggtcaccgtctcctca

SEQ ID NO: 422 - protein, 123 aa, Homo sapiens
EVQLVESGGGVVQPGRPLRLSCAASGFPFSNYGMHWVRQAPGKGLEWVAVIWYDGSNKYYADSVKGRFTISRDNSKNTLYLQMNNLRAEDTAIYYCAKDGYTAHYYYYYMDVWGKGTTVTVSS

SEQ ID NO: 423 - DNA, 328 bp, Homo sapiens
  source 1..328: mol_type = other DNA
gccatccagttgacccagtctccaggcaccctgtctttgtctccaggggaaagagccaccctctcctgcagggccagtcagagtgttagcagcagctacttagcctggtaccagcagaaacctggccaggctcccaggctcctaatctatggtgcatccagcagggccactggcatcccaggcaggttcagtggcagtgggtctgggacagacttcactctcaccatcagcagactggagcctgaagattttgcagtgtattactgtcagcagtatggtagctcacctgggatcactttcggcggagggaccaaagtggatatcaaac

SEQ ID NO: 424 - protein, 109 aa, Homo sapiens
AIQLTQSPGTLSLSPGERATLSCRASQSVSSSYLAWYQQKPGQAPRLLIYGASSRATGIPGRFSGSGSGTDFTLTISRLEPEDFAVYYCQQYGSSPGITFGGGTKVDIK

SEQ ID NO: 425 - protein, 8 aa, Homo sapiens
GFPFSNYG

SEQ ID NO: 426 - protein, 8 aa, Homo sapiens
IWYDGSNK

SEQ ID NO: 427 - protein, 16 aa, Homo sapiens
AKDGYTAHYYYYYMDV

SEQ ID NO: 428 - protein, 7 aa, Homo sapiens
QSVSSSY

SEQ ID NO: 429 - skipped

SEQ ID NO: 430 - protein, 10 aa, Homo sapiens
QQYGSSPGIT

SEQ ID NO: 431 - DNA, 372 bp, Homo sapiens
  source 1..372: mol_type = other DNA
gaagtgcagctggtggagtctgggggaggcgtggtccagcctgggaggtccctgagactctcctgtgcagcctctggattcaccttcagtaactatggcatacactgggtccgccaggctccaggcaaggggctggagtgggtggcagttatttcatatgatggaagtcataaatattatgcagactctgtgaagggccgattcaccatctccagagacaattccaagaacacgctatatctgcaaatgaacagcctgaaaactgaggacacggctgtgtattactgtgcgaaagatagttcagctgctattccctactactactacggtatggacgtctggggccaagggaccacggtcaccgtctcttca

SEQ ID NO: 432 - protein, 124 aa, Homo sapiens
EVQLVESGGGVVQPGRSLRLSCAASGFTFSNYGIHWVRQAPGKGLEWVAVISYDGSHKYYADSVKGRFTISRDNSKNTLYLQMNSLKTEDTAVYYCAKDSSAAIPYYYYGMDVWGQGTTVTVSS

SEQ ID NO: 433 - DNA, 340 bp, Homo sapiens
  source 1..340: mol_type = other DNA
gccatccagatgacccagtctccagactccctggctgtgtctctgggcgagagggccaccatcaactgcaagtccagccagagtattttatacaactccaacaataagacctacttagcttggtaccagcagaaaccaggacagcctcctaagctgctcattttctgggcatctacccgggaatccggggtccctgaccgattcagtggcagcgggtctgggacagatttcactctcaccatcagcagcctgcaggctgaagatgtggcagtttattactgtcagcaatattatagtattccccttattttcggccctgggaccaaagtggatatcaaac

SEQ ID NO: 434 - protein, 113 aa, Homo sapiens
AIQMTQSPDSLAVSLGERATINCKSSQSILYNSNNKTYLAWYQQKPGQPPKLLIFWASTRESGVPDRFSGSGSGTDFTLTISSLQAEDVAVYYCQQYYSIPLIFGPGTKVDIK

SEQ ID NO: 435 - protein, 8 aa, Homo sapiens
GFTFSNYG

SEQ ID NO: 436 - protein, 8 aa, Homo sapiens
ISYDGSHK

SEQ ID NO: 437 - protein, 17 aa, Homo sapiens
AKDSSAAIPYYYYGMDV

SEQ ID NO: 438 - protein, 12 aa, Homo sapiens
QSILYNSNNKTY

SEQ ID NO: 439 - skipped

SEQ ID NO: 440 - protein, 9 aa, Homo sapiens
QQYYSIPLI

SEQ ID NO: 441 - DNA, 370 bp, Homo sapiens
  source 1..370: mol_type = other DNA
cagctgcagctgcaggagtcgggcccaggactggtgaagccttcggagaccctgtccctcacctgcactgtctctggtggctccatcagcagtagtagttactactggggctggatccgccagcccccagggaaggggctggagtggattgggaatgtctactatagtgggggcacctactgcaacccgtccctcaagagtcgagtcaccatatcagtagacacgtccaagaatcagttctccctgaacctgagctccgtgaccgccgcggacacggccgtgtattactgtgcgagaatatggttcggggagcctgcgggtgggtactttgactactggggccagggaaccctggtcaccgtctcctcag

SEQ ID NO: 442 - protein, 123 aa, Homo sapiens
QLQLQESGPGLVKPSETLSLTCTVSGGSISSSSYYWGWIRQPPGKGLEWIGNVYYSGGTYCNPSLKSRVTISVDTSKNQFSLNLSSVTAADTAVYYCARIWFGEPAGGYFDYWGQGTLVTVSS

SEQ ID NO: 443 - DNA, 319 bp, Homo sapiens
  source 1..319: mol_type = other DNA
tcctatgagctgactcagccaccctcagtgtccgtgtccccaggacagacagccagcatcacctgctctggacataagttgggggataaaaatgcttgctggtatcagcagaagccaggccagtcccctgtgctggtcatctatgaatataacaagcggccctcagggatccctgagcgattctctggctccaactctgggaacacagccactctgaccatcagcgggacccaggctatggatgaggctgactattactgtcaggcgtgggacaccggcactcatgtcttcggaactgggaccaaggtcaccgtcctag

SEQ ID NO: 444 - protein, 106 aa, Homo sapiens
SYELTQPPSVSVSPGQTASITCSGHKLGDKNACWYQQKPGQSPVLVIYEYNKRPSGIPERFSGSNSGNTATLTISGTQAMDEADYYCQAWDTGTHVFGTGTKVTVL

SEQ ID NO: 445 - protein, 10 aa, Homo sapiens
GGSISSSSYY

SEQ ID NO: 446 - protein, 7 aa, Homo sapiens
VYYSGGT

SEQ ID NO: 447 - protein, 15 aa, Homo sapiens
ARIWFGEPAGGYFDY

SEQ ID NO: 448 - protein, 6 aa, Homo sapiens
KLGDKN

SEQ ID NO: 449 - skipped

SEQ ID NO: 450 - protein, 9 aa, Homo sapiens
QAWDTGTHV

SEQ ID NO: 451 - DNA, 370 bp, Homo sapiens
  source 1..370: mol_type = other DNA
caggtccagctggtacagtcgggcccaggactggtgaagccttcacagaccctgtccctcacctgctctgtctctgatggctccatcagcagtagtgattactactggagctggatccgccagccccccgggaagggcctggagtggattgggtacatctattacactgggagcacctactacaacccgtccctcaagagtcgagtttccatatcagtagacaggtccaagaaccaattctccctgaagctgagttctgtgactgccgcagacacggccgtttactattgtgccagactcgtagtaccatctccgaagggctcctggttcgacccctggggccagggaaccctggtcaccgtctcctcaa

SEQ ID NO: 452 - protein, 123 aa, Homo sapiens
QVQLVQSGPGLVKPSQTLSLTCSVSDGSISSSDYYWSWIRQPPGKGLEWIGYIYYTGSTYYNPSLKSRVSISVDRSKNQFSLKLSSVTAADTAVYYCARLVVPSPKGSWFDPWGQGTLVTVSS

SEQ ID NO: 453 - DNA, 331 bp, Homo sapiens
  source 1..331: mol_type = other DNA
tcctatgagctgactcagcctgcctccgtgtctgggtctcctggacagtcgatcaccatctcctgcactgggaccagcattgatgttgggaattataaccttgcctcctggtaccaacagcacccaggcaaagcccccaaactcatcatttatgagggcagtaggcggccctcaggggtttctaatcgcttctctggcgccaagtctggcaacacggcctccctgacaatctctgggctccaggctgaggacgaggctgattattactgctgctcatatgtaggtagtagcacttatgtcttcggatctgggaccaaggtcaccgtcctag

SEQ ID NO: 454 - protein, 110 aa, Homo sapiens
SYELTQPASVSGSPGQSITISCTGTSIDVGNYNLASWYQQHPGKAPKLIIYEGSRRPSGVSNRFSGAKSGNTASLTISGLQAEDEADYYCCSYVGSSTYVFGSGTKVTVL

SEQ ID NO: 455 - protein, 10 aa, Homo sapiens
DGSISSSDYY

SEQ ID NO: 456 - protein, 7 aa, Homo sapiens
IYYTGST

SEQ ID NO: 457 - protein, 15 aa, Homo sapiens
ARLVVPSPKGSWFDP

SEQ ID NO: 458 - protein, 9 aa, Homo sapiens
SIDVGNYNL

SEQ ID NO: 459 - skipped

SEQ ID NO: 460 - protein, 10 aa, Homo sapiens
CSYVGSSTYV

SEQ ID NO: 461 - DNA, 370 bp, Homo sapiens
  source 1..370: mol_type = other DNA
caggtccagctggtacagtctgggcctgaggtgaagaagcctgggacctcagtgaaggtctcctgcaaggcttctggattcacctttactagctctgctatgcagtgggtgcgacaggctcgtggacaacgccttgagtggataggatggatcgtcgttggcagtggtaacacaaactacgcacagaagttccaggaaagagtcaccattaccagggacatgtccacaagcacagcctacatggagctgagcagcctgagatccgaggacacggccgtgtattactgtgcggcagtttattgtagtggtggtagctgtaatgatgcttttgatatctggggccaagggacaatggtcaccgtctcttcag

SEQ ID NO: 462 - protein, 123 aa, Homo sapiens
QVQLVQSGPEVKKPGTSVKVSCKASGFTFTSSAMQWVRQARGQRLEWIGWIVVGSGNTNYAQKFQERVTITRDMSTSTAYMELSSLRSEDTAVYYCAAVYCSGGSCNDAFDIWGQGTMVTVSS

SEQ ID NO: 463 - DNA, 325 bp, Homo sapiens
  source 1..325: mol_type = other DNA
gaaatagtgatgacgcagtctccaggcaccctgtctttgtctccaggggaaagagccaccctctcctgcagggccagtcagagtgttagcagcagctacttagcctggtaccagcagaaacctggccaggctcccaggctcctcatctatggtgcatccagcagggccactggcatcccagacaggttcagtggcagtgggtctgggacagacttcactctcaccatcagcagactggagcctgaagattttgcagtgtattactgtcagcagtatggtagctcacccttcactttcggcggagggaccaaggtggaaatcaaac

SEQ ID NO: 464 - protein, 108 aa, Homo sapiens
EIVMTQSPGTLSLSPGERATLSCRASQSVSSSYLAWYQQKPGQAPRLLIYGASSRATGIPDRFSGSGSGTDFTLTISRLEPEDFAVYYCQQYGSSPFTFGGGTKVEIK

SEQ ID NO: 465 - protein, 8 aa, Homo sapiens
GFTFTSSA

SEQ ID NO: 466 - protein, 8 aa, Homo sapiens
IVVGSGNT

SEQ ID NO: 467 - protein, 16 aa, Homo sapiens
AAVYCSGGSCNDAFDI

SEQ ID NO: 468 - protein, 7 aa, Homo sapiens
QSVSSSY

SEQ ID NO: 469 - skipped

SEQ ID NO: 470 - protein, 9 aa, Homo sapiens
QQYGSSPFT

SEQ ID NO: 471 - DNA, 367 bp, Homo sapiens
  source 1..367: mol_type = other DNA
caggtacagctgcagcagtcgggcccaggactggtgaagccttcggagaccctgtccctcacctgcactgtctctggtgcctccattagtaattattactggagttggatccggcagcccccagggaagggactggagtgggttggatatatctattacactgggagcaccaaccacaacccctccctcaagagtcgagtcaccatatcactagacacgtccaagaatcagttctccctgaggctgagctctgtgaccgctgcggacacggccgtctattactgtgcgcgagcctattgtagtggtggtagctgcttcgatacttttgatatctggggccaagggacaatggtcaccgtctcttcag

SEQ ID NO: 472 - protein, 122 aa, Homo sapiens
QVQLQQSGPGLVKPSETLSLTCTVSGASISNYYWSWIRQPPGKGLEWVGYIYYTGSTNHNPSLKSRVTISLDTSKNQFSLRLSSVTAADTAVYYCARAYCSGGSCFDTFDIWGQGTMVTVSS

SEQ ID NO: 473 - DNA, 325 bp, Homo sapiens
  source 1..325: mol_type = other DNA
tcctatgagctgacacagccaccctcggtgtcagtggccccaggacagacggccagaattacctgtgggggaaacaacattggaagtaaaagtgtgcactggttccagcagaagccaggccaggcccctgtgctggtcgtctatgatgatagcgaccggccctcagggatccctgagcgattctctggctccaactctgggaacacggcctccctgaccatcagcagggtcgaagccggggatgaggccgactattactgtcaggtgtgggatagtgctagtgattcaggtgtcttcggaactgggaccaagctcaccgtcccag

SEQ ID NO: 474 - protein, 108 aa, Homo sapiens
SYELTQPPSVSVAPGQTARITCGGNNIGSKSVHWFQQKPGQAPVLVVYDDSDRPSGIPERFSGSNSGNTASLTISRVEAGDEADYYCQVWDSASDSGVFGTGTKLTVP

SEQ ID NO: 475 - protein, 8 aa, Homo sapiens
GASISNYY

SEQ ID NO: 476 - protein, 7 aa, Homo sapiens
IYYTGST

SEQ ID NO: 477 - protein, 16 aa, Homo sapiens
ARAYCSGGSCFDTFDI

SEQ ID NO: 478 - protein, 6 aa, Homo sapiens
NIGSKS

SEQ ID NO: 479 - skipped

SEQ ID NO: 480 - protein, 11 aa, Homo sapiens
QVWDSASDSGV

SEQ ID NO: 481 - DNA, 351 bp, Homo sapiens
  source 1..351: mol_type = other DNA
gaagtgcagctgttggagtctggaggaggcttggtccagcctggggggtccctgagactctcctgtgcagcctctgggttaaccgtcagaagcaactacatgaactgggtccgccaggctccagggaaggggctggagtgggtctcacttatttatagcggtggtagtacattctacgcagactccgtgaagggccgattcaccatctccagacacgattccaagaacacactgtatcttcaaatgaacagcctgagagctgaggacacggccgtgtattactgtgcgcgagatttggtagtctacggaatggacgtctggggccaagggaccacggtcaccgtctcctca

SEQ ID NO: 482 - protein, 117 aa, Homo sapiens
EVQLLESGGGLVQPGGSLRLSCAASGLTVRSNYMNWVRQAPGKGLEWVSLIYSGGSTFYADSVKGRFTISRHDSKNTLYLQMNSLRAEDTAVYYCARDLVVYGMDVWGQGTTVTVSS

SEQ ID NO: 483 - DNA, 322 bp, Homo sapiens
  source 1..322: mol_type = other DNA
gacatccagatgacccagtctccaggcaccctgtctttgtctccaggggaaagagccaccctctcctgcagggccagtcagagtgttagcagcagctccttagcctggtaccagcagaaacatggccaggctcccaggctcctcatctatggtacatccagcagggccactggcatcccagacaggttcagtggcagtgggtctgggacagacttcactctcaccatcagtggactggagcctgaagattttgcagtgtattactgtcagcagtatggtagctcaccccttttcggcggggggaccaaggtggaaatcaaac

SEQ ID NO: 484 - protein, 107 aa, Homo sapiens
DIQMTQSPGTLSLSPGERATLSCRASQSVSSSSLAWYQQKHGQAPRLLIYGTSSRATGIPDRFSGSGSGTDFTLTISGLEPEDFAVYYCQQYGSSPLFGGGTKVEIK

SEQ ID NO: 485 - protein, 8 aa, Homo sapiens
GLTVRSNY

SEQ ID NO: 486 - protein, 7 aa, Homo sapiens
IYSGGST

SEQ ID NO: 487 - protein, 11 aa, Homo sapiens
ARDLVVYGMDV

SEQ ID NO: 488 - protein, 7 aa, Homo sapiens
QSVSSSS

SEQ ID NO: 489 - skipped

SEQ ID NO: 490 - protein, 8 aa, Homo sapiens
QQYGSSPL

SEQ ID NO: 491 - DNA, 382 bp, Homo sapiens
  source 1..382: mol_type = other DNA
gaggtgcagctggtggagtctgggggaggcgtggtccagcctgggaggtccctgagactctcctgtgcagcctctggattcaccttcagtaattatggcatgcaccgggtccgccaggctccaggcaaggggctggagtgggtggcacttatttcatatgaagaaagtaatagatattatggagactccgtgaggggccgattcaccatctccagagacaattccaagaacactctgtatctgcaaatgaacagcctgagacctgaggacacggctgtgtattactgtgcgaaagatcaaggcccggctactgtgatggtgactgctattcggggcgctatggacgtctggggccaagggaccacggtcaccgtctcctcag

SEQ ID NO: 492 - protein, 127 aa, Homo sapiens
EVQLVESGGGVVQPGRSLRLSCAASGFTFSNYGMHRVRQAPGKGLEWVALISYEESNRYYGDSVRGRFTISRDNSKNTLYLQMNSLRPEDTAVYYCAKDQGPATVMVTAIRGAMDVWGQGTTVTVSS

SEQ ID NO: 493 - DNA, 343 bp, Homo sapiens
  source 1..343: mol_type = other DNA
gacatccagttgacccagtctccagattccctggctgtgtctctgggcgagagggccaccatcaactgcaagtccagccagagtgttttatacagctccaacaataagaactacttagcttggtaccagcagaaaccaggccagcctcctaaactcctcatttactgggcgtctacccgggaatccggggtccctgaccgattcagtggcagcgggtctgggacagatttcactctcaccatcagcagcctgcaggctgaagatgtggcagtatattactgtcagcaatattttggttctccttcgatcaccttcggccaagggacacgactggagattaaac

SEQ ID NO: 494 - protein, 114 aa, Homo sapiens
DIQLTQSPDSLAVSLGERATINCKSSQSVLYSSNNKNYLAWYQQKPGQPPKLLIYWASTRESGVPDRFSGSGSGTDFTLTISSLQAEDVAVYYCQQYFGSPSITFGQGTRLEIK

SEQ ID NO: 495 - protein, 8 aa, Homo sapiens
GFTFSNYG

SEQ ID NO: 496 - protein, 8 aa, Homo sapiens
ISYEESNR

SEQ ID NO: 497 - protein, 20 aa, Homo sapiens
AKDQGPATVMVTAIRGAMDV

SEQ ID NO: 498 - protein, 12 aa, Homo sapiens
QSVLYSSNNKNY

SEQ ID NO: 499 - skipped

SEQ ID NO: 500 - protein, 10 aa, Homo sapiens
QQYFGSPSIT

SEQ ID NO: 501 - DNA, 373 bp, Homo sapiens
  source 1..373: mol_type = other DNA
caggtgcagctggtgcagtctggggctgaggtgaagaagcctggggcctcagtgaaggtctcctgcaaggcttctggatacaccttcaccgactactatatgcactgggtgcgacaggcccctggacaagggcttgagtggatgggatggatcaactctaaagatggtggcgcgaactatgcacagaagtttcagggcagggtcaccctgaccagggacacgtcaatcgacacagcctacatagaactgagcaggctcagatctgacgacacggccgtgtattactgtgcgagatccgcctctacagtaaccgaaccaccgacaaactggttcgacccctggggccagggaaccctggtcaccgtctcctcag

SEQ ID NO: 502 - protein, 124 aa, Homo sapiens
QVQLVQSGAEVKKPGASVKVSCKASGYTFTDYYMHWVRQAPGQGLEWMGWINSKDGGANYAQKFQGRVTLTRDTSIDTAYIELSRLRSDDTAVYYCARSASTVTEPPTNWFDPWGQGTLVTVSS

SEQ ID NO: 503 - DNA, 325 bp, Homo sapiens
  source 1..325: mol_type = other DNA
gatgttgtgatgactcagtctccatcctccctgtctgcatctgtaggcgacagagtcaccgtcacttgccgggcaagtcagggcattagaaatgatttaggctggtatcagcagaaaccagggaaagctcctaagcgcctgatctatgctgcatccagtttgcaaagtggtgtcccatcaaggttcagcggcagtggatctgggacagacttcactctcacaatcagcagcctgcagcctgaagattttgcaacttattactgtctacagcataatagttacctccgtttcactttcggccctgggaccaaagtggatatcaaac

SEQ ID NO: 504 - protein, 108 aa, Homo sapiens
DVVMTQSPSSLSASVGDRVTVTCRASQGIRNDLGWYQQKPGKAPKRLIYAASSLQSGVPSRFSGSGSGTDFTLTISSLQPEDFATYYCLQHNSYLRFTFGPGTKVDIK

SEQ ID NO: 505 - protein, 8 aa, Homo sapiens
GYTFTDYY

SEQ ID NO: 506 - protein, 8 aa, Homo sapiens
INSKDGGA

SEQ ID NO: 507 - protein, 17 aa, Homo sapiens
ARSASTVTEPPTNWFDP

SEQ ID NO: 508 - protein, 6 aa, Homo sapiens
QGIRND

SEQ ID NO: 509 - skipped

SEQ ID NO: 510 - protein, 10 aa, Homo sapiens
LQHNSYLRFT

SEQ ID NO: 511 - DNA, 376 bp, Homo sapiens
  source 1..376: mol_type = other DNA
gaagtgcagctggtgcagtctggggctgaggtgaagaagcctggggcctcagtgaaggtctcctgcaaggcttctggatacaccttcaccggctactatatgcactgggtgcgacaggcccctggacaagggcttgagtggatgggatggatcaaccctaacagtggtggcacaaactatgcacagaagtttcagggcagggtcaccatgaccagggacacgtccatcaccacaggctacatggagctgagcagcctgagatctgacgacacggccctgtattactgtgcgagagttggggctcacgattactatgatagtagtgacaactggttcgacccctggggccagggaaccctggtcaccgtcttctcag

SEQ ID NO: 512 - protein, 125 aa, Homo sapiens
EVQLVQSGAEVKKPGASVKVSCKASGYTFTGYYMHWVRQAPGQGLEWMGWINPNSGGTNYAQKFQGRVTMTRDTSITTGYMELSSLRSDDTALYYCARVGAHDYYDSSDNWFDPWGQGTLVTVFS

SEQ ID NO: 513 - DNA, 322 bp, Homo sapiens
  source 1..322: mol_type = other DNA
gacatccagatgacccagtctccatcttccgtgtctgcatctgtaggagacagactcaccatcacttgtcgggcgagtcagggtattagcagctggttagcctggtatcagcagaaaccagggaaagcccctaagctcctgatctatgctgcatccagtttgcaaagtggggtcccatcaaggttcagcggcagtggatctgggacagatttcactctcaccatcagcagcctgcagcctgaagattttgcaacttactattgtcaacaggctaacagtttcccgtggacgttcggccaagggaccaaggtggagatcaaac

SEQ ID NO: 514 - protein, 107 aa, Homo sapiens
DIQMTQSPSSVSASVGDRLTITCRASQGISSWLAWYQQKPGKAPKLLIYAASSLQSGVPSRFSGSGSGTDFTLTISSLQPEDFATYYCQQANSFPWTFGQGTKVEIK

SEQ ID NO: 515 - protein, 8 aa, Homo sapiens
GYTFTGYY

SEQ ID NO: 516 - protein, 8 aa, Homo sapiens
INPNSGGT

SEQ ID NO: 517 - protein, 18 aa, Homo sapiens
ARVGAHDYYDSSDNWFDP

SEQ ID NO: 518 - protein, 6 aa, Homo sapiens
QGISSW

SEQ ID NO: 519 - skipped

SEQ ID NO: 520 - protein, 9 aa, Homo sapiens
QQANSFPWT

SEQ ID NO: 521 - DNA, 375 bp, Homo sapiens
  source 1..375: mol_type = other DNA
caggtgcagctggtgcagtctggggctgaggtgaagaagcctggggcctcagtgaaggtctcctgcaaggcttctggataccccctcaccggctactatatacactgggtgcgacaggcccctggacaaggacttgagtggatgggatggctcaaccctaacagtggtggcacaaagtatgcacagaagtttcagggcagggtcaccatgaccagggacacgtccatcagcacaggctacatggagctgagcaggctgagatctgacgacacggccgtgtactactgtgcgagagatggggggggaatagatgattacgttcaggaggacggtatggacgtctggggccaagggcccatggtcaccgtctcttca

SEQ ID NO: 522 - protein, 125 aa, Homo sapiens
QVQLVQSGAEVKKPGASVKVSCKASGYPLTGYYIHWVRQAPGQGLEWMGWLNPNSGGTKYAQKFQGRVTMTRDTSISTGYMELSRLRSDDTAVYYCARDGGGIDDYVQEDGMDVWGQGPMVTVSS

SEQ ID NO: 523 - DNA, 325 bp, Homo sapiens
  source 1..325: mol_type = other DNA
caatctgccctgactcagccaccctcggtgtcagtgtccccaggacagacggccaggatcacctgctctggagatgcattgtcaaagcaacatgcttattggtaccagcagaagccaggccaggcccctgtattggtgatatataaagacagtgagaggccctcagggatccctgagcgattctctggctccagctcagggacaatagtcacgttgaccatcagtggagtccaggcagaagacgaggctgactattactgtcaatcagcagacaacagtggtagtagatatgtcttcggaactgggaccaaggtcaccgtcctag

SEQ ID NO: 524 - protein, 108 aa, Homo sapiens
QSALTQPPSVSVSPGQTARITCSGDALSKQHAYWYQQKPGQAPVLVIYKDSERPSGIPERFSGSSSGTIVTLTISGVQAEDEADYYCQSADNSGSRYVFGTGTKVTVL

SEQ ID NO: 525 - protein, 8 aa, Homo sapiens
GYPLTGYY

SEQ ID NO: 526 - protein, 8 aa, Homo sapiens
LNPNSGGT

SEQ ID NO: 527 - protein, 18 aa, Homo sapiens
ARDGGGIDDYVQEDGMDV

SEQ ID NO: 528 - protein, 6 aa, Homo sapiens
ALSKQH

SEQ ID NO: 529 - skipped

SEQ ID NO: 530 - protein, 11 aa, Homo sapiens
QSADNSGSRYV

SEQ ID NO: 531 - DNA, 355 bp, Homo sapiens
  source 1..355: mol_type = other DNA
gaagtgcagctggtggagtctgggggaggcttggtacagcctggggggtccctgagactctcctgtgcagcctctggattcaccttcagtagctatagcatgaactgggtccgccaggctccagggaaggggctggagtgggtctcatacattagtggcattaatagtgccatatattacgcagactctgtgaagggccgcttcaccatctccagagacaacgccaagaactcactgtatctgcaaatgaacagcctgagagtcgaggacacggctgtgtattactgtgcgagagataaatacttaggtataaaagatatgtggggccaagggacaatggtcaccgtctcttcag

SEQ ID NO: 532 - protein, 118 aa, Homo sapiens
EVQLVESGGGLVQPGGSLRLSCAASGFTFSSYSMNWVRQAPGKGLEWVSYISGINSAIYYADSVKGRFTISRDNAKNSLYLQMNSLRVEDTAVYYCARDKYLGIKDMWGQGTMVTVSS

SEQ ID NO: 533 - DNA, 322 bp, Homo sapiens
  source 1..322: mol_type = other DNA
gacatccagatgacccagtctccagccaccctgtctttgtctccaggggaaagagccaccctctcctgcagggccagtcagagtgttagcacctacttagcctggtaccaacagaaacctggccaggctcccaggctcgtcatctatgatgcatccaacagggccactggcatcccagccaggttcagtggcggtgggtctgggacagacttcactctcaccatcagcagcctagagcctgaagattttgcagtttattactgtcaacagcgtctcaactggcctctcactttcggcggagggaccaaagtggatatcaaac

SEQ ID NO: 534 - protein, 107 aa, Homo sapiens
DIQMTQSPATLSLSPGERATLSCRASQSVSTYLAWYQQKPGQAPRLVIYDASNRATGIPARFSGGGSGTDFTLTISSLEPEDFAVYYCQQRLNWPLTFGGGTKVDIK

SEQ ID NO: 535 - protein, 8 aa, Homo sapiens
GFTFSSYS

SEQ ID NO: 536 - protein, 8 aa, Homo sapiens
ISGINSAI

SEQ ID NO: 537 - protein, 11 aa, Homo sapiens
ARDKYLGIKDM

SEQ ID NO: 538 - protein, 6 aa, Homo sapiens
QSVSTY

SEQ ID NO: 539 - skipped

SEQ ID NO: 540 - protein, 9 aa, Homo sapiens
QQRLNWPLT

SEQ ID NO: 541 - DNA, 375 bp, Homo sapiens
  source 1..375: mol_type = other DNA
gaggtgcagctggtacagtctggagcagaggtgaaaaagccgggggagtctctgaagatctcctgtaagggctctggatacagctttaccaactactggatcggctgggtgcgccagatgcccgggaaaggcctggagtggatggggatcatctatcctggtgactctggtaccagatacagcccgtccttccaaggccaggtcaccatctcagccgacaagtccatcagaaccgcctacctgcagtggagcagcctgaaggcctcggacagcgccatgtattactgtgcgaggtctagagtgggagctactgggggctattatgactactatatggacgtctggggccaagggaccacggtcaccgtctcctca

SEQ ID NO: 542 - protein, 125 aa, Homo sapiens
EVQLVQSGAEVKKPGESLKISCKGSGYSFTNYWIGWVRQMPGKGLEWMGIIYPGDSGTRYSPSFQGQVTISADKSIRTAYLQWSSLKASDSAMYYCARSRVGATGGYYDYYMDVWGQGTTVTVSS

SEQ ID NO: 543 - DNA, 331 bp, Homo sapiens
  source 1..331: mol_type = other DNA
cagtctgtgttgacgcagccaccctcagcgtctgggacccccgggcagagggtcaccatctcttgttctggaagcagctccaacctcggaggtaatactgtaaactggtaccagcagctcccaggaacggcccccaaactcctcatctatagtaataatcagcggccctcaggggtccctgaccgattctctggctccaagtctggcacctcagcctccctggccatcagtgggctccagtctgaggatgaggctgattattactgtgcagcatgggatgacagcctgaatggtcccgtcttcggaactgggaccaaggtcaccgtcctag

SEQ ID NO: 544 - protein, 110 aa, Homo sapiens
QSVLTQPPSASGTPGQRVTISCSGSSSNLGGNTVNWYQQLPGTAPKLLIYSNNQRPSGVPDRFSGSKSGTSASLAISGLQSEDEADYYCAAWDDSLNGPVFGTGTKVTVL

SEQ ID NO: 545 - protein, 8 aa, Homo sapiens
GYSFTNYW

SEQ ID NO: 546 - protein, 8 aa, Homo sapiens
IYPGDSGT

SEQ ID NO: 547 - protein, 18 aa, Homo sapiens
ARSRVGATGGYYDYYMDV

SEQ ID NO: 548 - protein, 8 aa, Homo sapiens
SSNLGGNT

SEQ ID NO: 549 - skipped

SEQ ID NO: 550 - protein, 11 aa, Homo sapiens
AAWDDSLNGPV

SEQ ID NO: 551 - DNA, 370 bp, Homo sapiens
  source 1..370: mol_type = other DNA
caggtgcagctggtggagtcgggcccaggacaggtgaagccttcggagaccctgtccctcacctgcactgtctctggtggctccatcagcagtagtagttactactggggctggatccgccagcccccagggaagggactggagtggattgggagtatctattatagtgggagcgcctactataacccgtccctcaagagtcgagtcaccatatccgtagacacgtccaagaaccagttctccctgaagctgaactctgtgaccgccgcagacacggctgtcttttactgtgcgagacacgcagctcccagtccgggggacaactggttcgacccctggggccagggaaccctggtcaccgtctcctcag

SEQ ID NO: 552 - protein, 123 aa, Homo sapiens
QVQLVESGPGQVKPSETLSLTCTVSGGSISSSSYYWGWIRQPPGKGLEWIGSIYYSGSAYYNPSLKSRVTISVDTSKNQFSLKLNSVTAADTAVFYCARHAAPSPGDNWFDPWGQGTLVTVSS

SEQ ID NO: 553 - DNA, 322 bp, Homo sapiens
  source 1..322: mol_type = other DNA
cagtctgtgttgactcagccaccctcggtgtcagtgtccccaggacagacggcccggatcacctgctctggagatgcattgtcaacgcaaaatggtaattggtaccagcagaagccaggccaggcccctgtgatggtgatatgtaaagacagtgagaggccctcagggatccctgagcgattctctggctccaggtcagggacaacagtcacgttgaccatcagtggagtccaggcagaagacgaagctgactatcactgtcaatcagcagacaacagggcacatgtagtattcggcggagggaccaagctgaccgtcctag

SEQ ID NO: 554 - protein, 107 aa, Homo sapiens
QSVLTQPPSVSVSPGQTARITCSGDALSTQNGNWYQQKPGQAPVMVICKDSERPSGIPERFSGSRSGTTVTLTISGVQAEDEADYHCQSADNRAHVVFGGGTKLTVL

SEQ ID NO: 555 - protein, 10 aa, Homo sapiens
GGSISSSSYY

SEQ ID NO: 556 - protein, 7 aa, Homo sapiens
IYYSGSA

SEQ ID NO: 557 - protein, 15 aa, Homo sapiens
ARHAAPSPGDNWFDP

SEQ ID NO: 558 - protein, 6 aa, Homo sapiens
ALSTQN

SEQ ID NO: 559 - skipped

SEQ ID NO: 560 - protein, 10 aa, Homo sapiens
QSADNRAHVV

SEQ ID NO: 561 - DNA, 378 bp, Homo sapiens
  source 1..378: mol_type = other DNA
gaggtgcagctggtggagtctgggggaggcgtggtccagcctgggaggtccctgagactctcctgtgcagcgtctggattcacctttagtagttatggcatgcactgggtccgccaggctccaggcaaggggctggagtgggtggcagttatatggtatgatggaagtaataacttctatgcagactccgtgaagggccgattcaccatctccagagacaatttcaagaacacgctgtatttgcaaatgaacagcctgagagccgaggacacggctgtgtattactgtgcgagatcatattgtagtggtggtttctgcttcggctactactatggtttggacgtgtggggccaagggaccacggtcaccgtctcctca

SEQ ID NO: 562 - protein, 126 aa, Homo sapiens
EVQLVESGGGVVQPGRSLRLSCAASGFTFSSYGMHWVRQAPGKGLEWVAVIWYDGSNNFYADSVKGRFTISRDNFKNTLYLQMNSLRAEDTAVYYCARSYCSGGFCFGYYYGLDVWGQGTTVTVSS

SEQ ID NO: 563 - DNA, 325 bp, Homo sapiens
  source 1..325: mol_type = other DNA
tcctatgagctgactcagccaccctcagtgtcagtggccccaggaaagacggccacgattacctgtgggggaaacaacattggaactaaaagtgtgcactggtaccagcagaagccaggccaggcccctgtgttggtcatctattataatagcgaccggccctccgggatccctgagcgattctctggctccaactctgggaacacggtcaccctgaccatcagcagggtcgaagccggggatgaggccgactattactgtcaggtgtgggatagtggtagtgatcattatgtcttcggaactgggaccaaggtcaccgtcgtag

SEQ ID NO: 564 - protein, 108 aa, Homo sapiens
SYELTQPPSVSVAPGKTATITCGGNNIGTKSVHWYQQKPGQAPVLVIYYNSDRPSGIPERFSGSNSGNTVTLTISRVEAGDEADYYCQVWDSGSDHYVFGTGTKVTVV

SEQ ID NO: 565 - protein, 8 aa, Homo sapiens
GFTFSSYG

SEQ ID NO: 566 - protein, 8 aa, Homo sapiens
IWYDGSNN

SEQ ID NO: 567 - protein, 19 aa, Homo sapiens
ARSYCSGGFCFGYYYGLDV

SEQ ID NO: 568 - protein, 6 aa, Homo sapiens
NIGTKS

SEQ ID NO: 569 - skipped

SEQ ID NO: 570 - protein, 11 aa, Homo sapiens
QVWDSGSDHYV

SEQ ID NO: 571 - DNA, 358 bp, Homo sapiens
  source 1..358: mol_type = other DNA
caggtgcagctggtgcagtctggagctgaggtgaagaagcctggggcctcagtgaaggtctcctgcaaggcttctggttacacctttaccagctatggtatcagctgggtgcgacaggcccctggacaagggcttgagtggatgggatggatcagcccttacaatggtaacacacactatgcacagaagctccagggcagagtcaccatgaccacagacacatccacgagcacagcctacatggagctgaggagcctgagatctgacgacacggccgtatattactgtgcgagagatggggagttattgggctggttcgacccctggggccagggaaccctggtcaccgtctcctcag

SEQ ID NO: 572 - protein, 119 aa, Homo sapiens
QVQLVQSGAEVKKPGASVKVSCKASGYTFTSYGISWVRQAPGQGLEWMGWISPYNGNTHYAQKLQGRVTMTTDTSTSTAYMELRSLRSDDTAVYYCARDGELLGWFDPWGQGTLVTVSS

SEQ ID NO: 573 - DNA, 331 bp, Homo sapiens
  source 1..331: mol_type = other DNA
cagtctgtcgtgacgcagcctgcctccgtgtctgggtctcctggacagtcgatcaccatctcctgcactggaaccagcagtgatgttgggagttataaccttgtctcctggtaccaacagcacccaggcaaagcccccaaactcatgatttatgcgggcagtaagcggccctcaggggtttctaatcgcttctctggctccaagtctggcaacacggcctccctgacaatctctgggctccaggctgaggacgaggctgattattactgctgctcatatgcaggtagtagcacttgggtgttcggcggagggaccaagctgaccgtcctag

SEQ ID NO: 574 - protein, 110 aa, Homo sapiens
QSVVTQPASVSGSPGQSITISCTGTSSDVGSYNLVSWYQQHPGKAPKLMIYAGSKRPSGVSNRFSGSKSGNTASLTISGLQAEDEADYYCCSYAGSSTWVFGGGTKLTVL

SEQ ID NO: 575 - protein, 8 aa, Homo sapiens
GYTFTSYG

SEQ ID NO: 576 - protein, 8 aa, Homo sapiens
ISPYNGNT

SEQ ID NO: 577 - protein, 12 aa, Homo sapiens
ARDGELLGWFDP

SEQ ID NO: 578 - protein, 9 aa, Homo sapiens
SSDVGSYNL

SEQ ID NO: 579 - skipped

SEQ ID NO: 580 - protein, 10 aa, Homo sapiens
CSYAGSSTWV

SEQ ID NO: 581 - DNA, 378 bp, Homo sapiens
  source 1..378: mol_type = other DNA
ccaggtcagctggtggaatctgggggaagcttggtacagcctgggggggccctgagactctcctgtgaagcctctggattcacctttagcgactatgccatgagctgggtccgccaggctccagggaaggggctggagtgggtctcagttattaatagtagtggtggtatcacaaactacgcagactccgtgaagggccggttcaccatctccagaaacaattccaagaacacgctctatctgcaaatgaacagcctgagaggcgacgacacggccatatattactgtgcgaagggacccccgagaattaacaccttctacaggcactactacggtatggacgtctggggccaagggatcacggtcaccgtctcctca

SEQ ID NO: 582 - protein, 126 aa, Homo sapiens
PGQLVESGGSLVQPGGALRLSCEASGFTFSDYAMSWVRQAPGKGLEWVSVINSSGGITNYADSVKGRFTISRNNSKNTLYLQMNSLRGDDTAIYYCAKGPPRINTFYRHYYGMDVWGQGITVTVSS

SEQ ID NO: 583 - DNA, 322 bp, Homo sapiens
  source 1..322: mol_type = other DNA
gccatccagttgacccagtctccatcctccctgtctgcatctgtaggagacagagtcaccatcacttgccaggcgagtcaggacattaggaactatttaaattggtatcagcagaaaccagggaaagcccctaagctcctgatctacgatgcatccaatttggaaacaggggtcccatcaaggttcagtggaagtggatctgggacagattttactttcaccatcggcagcctgcagcctgaagatattgcaacatattactgtcaacaatatgataatctccgggccactttcggcggagggaccaaggtggagatcaaac

SEQ ID NO: 584 - protein, 107 aa, Homo sapiens
AIQLTQSPSSLSASVGDRVTITCQASQDIRNYLNWYQQKPGKAPKLLIYDASNLETGVPSRFSGSGSGTDFTFTIGSLQPEDIATYYCQQYDNLRATFGGGTKVEIK

SEQ ID NO: 585 - protein, 8 aa, Homo sapiens
GFTFSDYA

SEQ ID NO: 586 - protein, 8 aa, Homo sapiens
INSSGGIT

SEQ ID NO: 587 - protein, 19 aa, Homo sapiens
AKGPPRINTFYRHYYGMDV

SEQ ID NO: 588 - protein, 6 aa, Homo sapiens
QDIRNY

SEQ ID NO: 589 - skipped

SEQ ID NO: 590 - protein, 9 aa, Homo sapiens
QQYDNLRAT

SEQ ID NO: 591 - DNA, 370 bp, Homo sapiens
  source 1..370: mol_type = other DNA
caggtgcagctggtggagtctgggcctgaaatgaagaagcctgggacctcagtgaaggtctcctgcaaggcttctggattcacctttattacgtctgctgttcagtgggtgcgacaggctcgtggacaacgccttgagtggatgggatggatcgccgttggcagtggtaacacaaactacgcacagaaattccaggacagagtcaccattaacagggacatgtccacaagcacagcctacatggagctgagcagcctgagatccgaggacacggccgtgtattactgtgcggccccgcattgtaatcgtaccagctgccatgatggttttgatatctggggccaagggacaatggtcaccgtctcttcag

SEQ ID NO: 592 - protein, 123 aa, Homo sapiens
QVQLVESGPEMKKPGTSVKVSCKASGFTFITSAVQWVRQARGQRLEWMGWIAVGSGNTNYAQKFQDRVTINRDMSTSTAYMELSSLRSEDTAVYYCAAPHCNRTSCHDGFDIWGQGTMVTVSS

SEQ ID NO: 593 - DNA, 325 bp, Homo sapiens
  source 1..325: mol_type = other DNA
gaaattgtgttgacgcagtctccaggcaccctgtctttgtctccaggggaaagagccaccctctcctgcagggccagtcagagtgttagcagaaactacttagcctggtaccagcagaaacctggccaggttcccaggctcctcatctatggtgcatccagcagggccactggcatcccagacaggttcagaggtagtgggtctgggacagacttcactctcaccatcaacagactggagtctgaagattttgcagtgtattactgtcagcagtatggtagctccctattcactttcggccctgggaccaaagtggatatcaaac

SEQ ID NO: 594 - protein, 108 aa, Homo sapiens
EIVLTQSPGTLSLSPGERATLSCRASQSVSRNYLAWYQQKPGQVPRLLIYGASSRATGIPDRFRGSGSGTDFTLTINRLESEDFAVYYCQQYGSSLFTFGPGTKVDIK

SEQ ID NO: 595 - protein, 8 aa, Homo sapiens
GFTFITSA

SEQ ID NO: 596 - protein, 8 aa, Homo sapiens
IAVGSGNT

SEQ ID NO: 597 - protein, 16 aa, Homo sapiens
AAPHCNRTSCHDGFDI

SEQ ID NO: 598 - protein, 7 aa, Homo sapiens
QSVSRNY

SEQ ID NO: 599 - skipped

SEQ ID NO: 600 - protein, 9 aa, Homo sapiens
QQYGSSLFT

SEQ ID NO: 601 - DNA, 361 bp, Homo sapiens
  source 1..361: mol_type = other DNA
gaagtgcagctggtggagtcggggggaggcctggtcaagcctggggagtccctgagactctcctgtgcagcctctggattcaccttcagtagctatgccatgaactgggtccgccaggctccagggaaggggctggagtgggtctcatccattagtactggtagttatttcatatactactcagactcagtgaagggccgattcaccatttccagagacaacgccaagaactcactgtatctgcaaatgaacagcctgagagccgcggacacggctatctattactgtgcgagaggaaaggaagatacaagcgctgcttttgatatctggggccaagggacaatggtcaccgtctcttcag

SEQ ID NO: 602 - protein, 120 aa, Homo sapiens
EVQLVESGGGLVKPGESLRLSCAASGFTFSSYAMNWVRQAPGKGLEWVSSISTGSYFIYYSDSVKGRFTISRDNAKNSLYLQMNSLRAADTAIYYCARGKEDTSAAFDIWGQGTMVTVSS

SEQ ID NO: 603 - DNA, 325 bp, Homo sapiens
  source 1..325: mol_type = other DNA
gccatccagatgacccagtctcttcctcctgcgactctggctccaggggaaagagccaccctctcctgcagggccagtcagagtgttagcaacaacttagcctggtaccagcagaaacctggccaggctcccaggctcctcatctatggtgcatccaccagggccactggtatcccagccaggttcagtggcagtgggtctgggacagagttcactctcaccatcagcagcctgcagtctgaagattttgcagtttattactgtcagcagtataataactggcctccgtggacgttcggccaagggaccaaagtggatatcaaac

SEQ ID NO: 604 - protein, 108 aa, Homo sapiens
AIQMTQSLPPATLAPGERATLSCRASQSVSNNLAWYQQKPGQAPRLLIYGASTRATGIPARFSGSGSGTEFTLTISSLQSEDFAVYYCQQYNNWPPWTFGQGTKVDIK

SEQ ID NO: 605 - protein, 8 aa, Homo sapiens
GFTFSSYA

SEQ ID NO: 606 - protein, 8 aa, Homo sapiens
ISTGSYFI

SEQ ID NO: 607 - protein, 13 aa, Homo sapiens
ARGKEDTSAAFDI

SEQ ID NO: 608 - protein, 6 aa, Homo sapiens
QSVSNN

SEQ ID NO: 609 - skipped

SEQ ID NO: 610 - protein, 10 aa, Homo sapiens [sequence omitted]

SEQ ID NO: 611 - DNA, 355 bp, Homo sapiens
  source 1..355: mol_type = other DNA
gaggtgcagctggtgcagtctggggctgaggtgaagaagcctgggtcctcggtgaaggtctcctgcaaggcttctggaggcaccttcagcagctctgttatcagctgggtgcgacaggcccctggacaaggccttgagtggatgggagggatcatccctctctttggttcagcaaactacgcacagaagttccagggcagagtcacgattaccgcggacgaatccacgagcacagcctacatggagatgactagcctgagatctgaagacacggccgtgtattactgtgcgaaagtttcccagtgggcgttaatactcttctggggccagggaaccctggtcaccgtctcctcag

SEQ ID NO: 612 - protein, 118 aa, Homo sapiens
EVQLVQSGAEVKKPGSSVKVSCKASGGTFSSSVISWVRQAPGQGLEWMGGIIPLFGSANYAQKFQGRVTITADESTSTAYMEMTSLRSEDTAVYYCAKVSQWALILFWGQGTLVTVSS

SEQ ID NO: 613 - DNA, 328 bp, Homo sapiens
  source 1..328: mol_type = other DNA
gccatccggatgacccagtctccaggcaccctgtctttgtctccaggggaaagagccaccctctcctgcagggccagtcagagtgttagcagcagctacttagcctggtaccagcagaaacctggccaggctcccaggctcctcatctatggtgcatccagcagggccactggcatcccagacaggttcagtggcagtgggtctgggacagacttcactctcaccatcagcagactggagcctgaagattttgcagtgtattactgtcagcagtatggtacctcaccttcgtggacgttcggccaagggaccaaggtggagatcaaac

SEQ ID NO: 614 - protein, 109 aa, Homo sapiens
AIRMTQSPGTLSLSPGERATLSCRASQSVSSSYLAWYQQKPGQAPRLLIYGASSRATGIPDRFSGSGSGTDFTLTISRLEPEDFAVYYCQQYGTSPSWTFGQGTKVEIK

SEQ ID NO: 615 - protein, 8 aa, Homo sapiens
GGTFSSSV

SEQ ID NO: 616 - protein, 8 aa, Homo sapiens
IIPLFGSA

SEQ ID NO: 617 - protein, 11 aa, Homo sapiens
AKVSQWALILF

SEQ ID NO: 618 - protein, 7 aa, Homo sapiens
QSVSSSY

SEQ ID NO: 619 - skipped

SEQ ID NO: 620 - protein, 10 aa, Homo sapiens
QQYGTSPSWT

SEQ ID NO: 621 - DNA, 355 bp, Homo sapiens
  source 1..355: mol_type = other DNA
gaggtgcagctggtgcagtctggggctgaggtgaagaagcctgggtcctcggtgaaggtctcctgcaaggcgtctagaggcaccttcaacacctatgttttcacctgggtgcgacaggcccctggacaagggcttgagtggatgggagggatcatccctttctttggtacagcagactacgcacagaagttccagggcagagtcacgattaccgcggacgactccacgagcacagcctacatggagctgagcagcctgagatctgaggacacggccgtgtattactgttcgaggctcagccagtgggacctactacccatgtggggccagggaaccctggtcaccgtctcctcag

SEQ ID NO: 622 - protein, 118 aa, Homo sapiens
EVQLVQSGAEVKKPGSSVKVSCKASRGTFNTYVFTWVRQAPGQGLEWMGGIIPFFGTADYAQKFQGRVTITADDSTSTAYMELSSLRSEDTAVYYCSRLSQWDLLPMWGQGTLVTVSS

SEQ ID NO: 623 - DNA, 331 bp, Homo sapiens
  source 1..331: mol_type = other DNA
gatattgtgatgactcagtctccaggcaccctgtctttgtctccaggggaaagagccaccctctcctgcagggccagtcagagttttaccagcagctacttagcctggtaccagcagaaacctggccaggctcccaggctcctcatctatggtgcatccagcagggccactggcatcccagacaggttcagtggcactgggtctgggacagacttcactctcaccatcagcagactggagcctgaagattttgcagtatattactgtcagcagtatggtacgtcacctcgcatgtacacttttggccaggggaccaaagtggatatcaaac

SEQ ID NO: 624 - protein, 110 aa, Homo sapiens
DIVMTQSPGTLSLSPGERATLSCRASQSFTSSYLAWYQQKPGQAPRLLIYGASSRATGIPDRFSGTGSGTDFTLTISRLEPEDFAVYYCQQYGTSPRMYTFGQGTKVDIK

SEQ ID NO: 625 - protein, 8 aa, Homo sapiens
RGTFNTYV

SEQ ID NO: 626 - protein, 8 aa, Homo sapiens
IIPFFGTA

SEQ ID NO: 627 - protein, 11 aa, Homo sapiens
SRLSQWDLLPM

SEQ ID NO: 628 - protein, 7 aa, Homo sapiens
QSFTSSY

SEQ ID NO: 629 - skipped

SEQ ID NO: 630 - protein, 11 aa, Homo sapiens
QQYGTSPRMYT

SEQ ID NO: 631 - DNA, 361 bp, Homo sapiens
  source 1..361: mol_type = other DNA
cagctgcagctggtggagtctggggctgaggtgaagaagcctggggcttcagtgaaggtctcctgcaaggtttccggatacaccctcactgaattatccatgcactgggtgcgacaggctcctggaaaagggcttgagtggatggggggttttgatcctgaagatggtgagacaatctacgcacagaagttccagggcagagtcaccatgaccgaggacacatctatagacacagtgtacatggagctgagcagcctgagatctgaggacacggccgtgtattactgtgcaatagatcgcaagcactggctggtaggtcttgactactggggccagggaaccctggtcaccgtctcctcag

SEQ ID NO: 632 - protein, 120 aa, Homo sapiens
QLQLVESGAEVKKPGASVKVSCKVSGYTLTELSMHWVRQAPGKGLEWMGGFDPEDGETIYAQKFQGRVTMTEDTSIDTVYMELSSLRSEDTAVYYCAIDRKHWLVGLDYWGQGTLVTVSS

SEQ ID NO: 633 - DNA, 322 bp, Homo sapiens
  source 1..322: mol_type = other DNA
gccatccggatgacccagtctccatcctcactgtctgcatctgtaggagacagagtcaccatcacttgtcgggcgagtcagggcattaggaattatttagcctggtttcagcagaaaccagggaaagcccctaagtccctgatctatgctgcatccagtttgcaaagtggggtcccatcaaagttcagcggcagtggatctgggacagatttcactctcaccatcagcagcctgcagcctgaagattttgcaacttattactgccaacagtataatagttaccccctcaccttcggccaagggacacgactggagattaaac

SEQ ID NO: 634 - protein, 107 aa, Homo sapiens
AIRMTQSPSSLSASVGDRVTITCRASQGIRNYLAWFQQKPGKAPKSLIYAASSLQSGVPSKFSGSGSGTDFTLTISSLQPEDFATYYCQQYNSYPLTFGQGTRLEIK

SEQ ID NO: 635 - protein, 8 aa, Homo sapiens
GYTLTELS

SEQ ID NO: 636 - protein, 8 aa, Homo sapiens
FDPEDGET

SEQ ID NO: 637 - protein, 13 aa, Homo sapiens
AIDRKHWLVGLDY

SEQ ID NO: 638 - protein, 6 aa, Homo sapiens
QGIRNY

SEQ ID NO: 639 - skipped

SEQ ID NO: 640 - protein, 9 aa, Homo sapiens
QQYNSYPLT

SEQ ID NO: 641 - DNA, 364 bp, Homo sapiens
  source 1..364: mol_type = other DNA
caggtgcagctggtgcagtccggagcagaggtgaaaaagcccggggagtctctgaggatctcctgtaagggttctggacacaactctcccagctactggattagctgggtgcgccagatgcccgggaaaggcctggagtggatggggagaattgatcctagtgactcttataccaactacagcccgtccttccaaggccatgtcaccatctcagctgacaagtccatcagtactgcctacctacagtggagcagcctgcaggcctcggacaccgccatttattactgtgcgagacacgtggttgcattgactcatttgtaccctgactactggggccagggaaccctggtcaccgtctcctcag

SEQ ID NO: 642 - protein, 121 aa, Homo sapiens
QVQLVQSGAEVKKPGESLRISCKGSGHNSPSYWISWVRQMPGKGLEWMGRIDPSDSYTNYSPSFQGHVTISADKSISTAYLQWSSLQASDTAIYYCARHVVALTHLYPDYWGQGTLVTVSS

SEQ ID NO: 643 - DNA, 325 bp, Homo sapiens
  source 1..325: mol_type = other DNA
gacatccagatgacccagtctccagccaccctgtctgtgtctccaggggaaagagccaccctctcctgcagggccagtcaaagtgttagcagcaccttagcctggtaccagcagaaacctggccaggctcccaggctcctcatctatggtgcatccaccagggccactggtatcccagccaggttcagtggcagtgggtctgggacagagttcactctcaccatcagcagcctgcagtctgaagattttgcagtttattactgtcagcaatataataactggtccacgtggacgttcggccaagggaccaaagtggatatcaaac

SEQ ID NO: 644 - protein, 108 aa, Homo sapiens
DIQMTQSPATLSVSPGERATLSCRASQSVSSTLAWYQQKPGQAPRLLIYGASTRATGIPARFSGSGSGTEFTLTISSLQSEDFAVYYCQQYNNWSTWTFGQGTKVDIK

SEQ ID NO: 645 - protein, 8 aa, Homo sapiens
GHNSPSYW

SEQ ID NO: 646 - protein, 8 aa, Homo sapiens
IDPSDSYT

SEQ ID NO: 647 - protein, 14 aa, Homo sapiens
ARHVVALTHLYPDY

SEQ ID NO: 648 - protein, 6 aa, Homo sapiens
QSVSST

SEQ ID NO: 649 - skipped

SEQ ID NO: 650 - protein, 10 aa, Homo sapiens
QQYNNWSTWT

SEQ ID NO: 651 - DNA, 379 bp, Homo sapiens
  source 1..379: mol_type = other DNA
caggtgcagctgcaggagtcgggcccaggactggtgaagccttcggagaccctgtccctcacctgcactgtctttggtggctccatcaccagtagtaatcactactgggtctggatccgccagcccccagggaaggggctggagtggattgggagtatgtattatagtgggagcaccgcctacaacccgtccctcacgaatcgagtcaccatatccgtagacacgtccaagaaccagttctccctgaagctgagctccgtgaccgccgcagacacggctgtgtattactgtgcgagacaaatcgggcccaagaggccctcgcaagtggctgactggttcgacccctggggccagggaaccctggtcaccgtctcctcag

SEQ ID NO: 652 - protein, 126 aa, Homo sapiens
QVQLQESGPGLVKPSETLSLTCTVFGGSITSSNHYWVWIRQPPGKGLEWIGSMYYSGSTAYNPSLTNRVTISVDTSKNQFSLKLSSVTAADTAVYYCARQIGPKRPSQVADWFDPWGQGTLVTVSS

SEQ ID NO: 653 - DNA, 322 bp, Homo sapiens
  source 1..322: mol_type = other DNA
gacatccagttgacccagtctccatccttcctgtctgcatctgtaggagacagagtcaccatcacttgccgggccagtcagggcattagcagttatttagcctggtatcagcaaaaacctgggaaagcccctaagctcctgatctatgctgcatccactttgcaaagtggggtcccatcaaggttcagcggcagtggatctgggacagaattcactctcacaatcagcagcctgcagcctgaagattttgcaacttattactgtcaacagcttaatagttacccgctcactttcggcggagggaccaaggtggaaatcaaac

SEQ ID NO: 654 - protein, 107 aa, Homo sapiens
DIQLTQSPSFLSASVGDRVTITCRASQGISSYLAWYQQKPGKAPKLLIYAASTLQSGVPSRFSGSGSGTEFTLTISSLQPEDFATYYCQQLNSYPLTFGGGTKVEIK

SEQ ID NO: 655 - protein, 10 aa, Homo sapiens
GGSITSSNHY

SEQ ID NO: 656 - protein, 7 aa, Homo sapiens
MYYSGST

SEQ ID NO: 657 - protein, 18 aa, Homo sapiens
ARQIGPKRPSQVADWFDP

SEQ ID NO: 658 - protein, 6 aa, Homo sapiens
QGISSY

SEQ ID NO: 659 - skipped

SEQ ID NO: 660 - protein, 9 aa, Homo sapiens
QQLNSYPLT

SEQ ID NO: 661 - DNA, 382 bp, Homo sapiens
  source 1..382: mol_type = other DNA
caggtgcagctgcaggagtcgggcccaggactggtgaagccttcggagaccctgtccctcacttgcactgtctctggtgactccatcagcagtagtcgttactactggggctggatccgccagcccccagggaaggggctggagtggattgggactttctattatagtgggatcacgtactacaacccgtccctcaagagtcgagtcaccatattcgtagacacgtccaagaaccagttctccctgaagctgagctctgtgaccgccgcagacacggctgtttattactgtgcgagaccccgaccccccgattactatgataatagtggtgcgctcctttttgatatctggggccaagggacaatggtcaccgtctcttcag

SEQ ID NO: 662 - protein, 127 aa, Homo sapiens
QVQLQESGPGLVKPSETLSLTCTVSGDSISSSRYYWGWIRQPPGKGLEWIGTFYYSGITYYNPSLKSRVTIFVDTSKNQFSLKLSSVTAADTAVYYCARPRPPDYYDNSGALLFDIWGQGTMVTVSS

SEQ ID NO: 663 - DNA, 325 bp, Homo sapiens
  source 1..325: mol_type = other DNA
gccatccggatgacccagtctccttccaccctgtctgcatctgtaggagacagagtcaccatcgcttgccgggccagtcagagtattagtgcctggttggcctggtatcagcagaaaccagggaaagcccctaagctcctgatctataaggcatctagtttagaaagtggggtcccatcaaggttcagcggcagtggatctgggacagaattcactctcaccatcaacagcctgcagcctgatgattttgccacttattactgccaacagtatattagttcttctccgtggacgttcggccaagggaccaaggtggaaatcaaac

SEQ ID NO: 664 - protein, 108 aa, Homo sapiens
AIRMTQSPSTLSASVGDRVTIACRASQSISAWLAWYQQKPGKAPKLLIYKASSLESGVPSRFSGSGSGTEFTLTINSLQPDDFATYYCQQYISSSPWTFGQGTKVEIK

SEQ ID NO: 665 - protein, 10 aa, Homo sapiens
GDSISSSRYY

SEQ ID NO: 666 - protein, 7 aa, Homo sapiens
FYYSGIT

SEQ ID NO: 667 - protein, 19 aa, Homo sapiens
ARPRPPDYYDNSGALLFDI

SEQ ID NO: 668 - protein, 6 aa, Homo sapiens
QSISAW

SEQ ID NO: 669 - skipped

SEQ ID NO: 670 - protein, 10 aa, Homo sapiens
QQYISSSPWT

SEQ ID NO: 671 - DNA, 370 bp, Homo sapiens
  source 1..370: mol_type = other DNA
cagctgcagctgcaggagtcgggcccaggactggtgaggccttcacagaccctgtccctctcctgcactgtctctggtggctccatcagcagtgccactcactactggagctggatccgccagcacccagggagaggcctggagtggattgggtacatctattacactgggggcaccttttacaatccgtccctcaagagtcgacttaccatatcagtggacacgtctaagaaccagttctccctgaagctgagcgctgtgactgccgcggacacggccgtgtattactgtgcgagagttatagcagctcgtccgggatctacctactttgacttctggggccggggaaccctggtcaccgtctcctcag

SEQ ID NO: 672 - protein, 123 aa, Homo sapiens
QLQLQESGPGLVRPSQTLSLSCTVSGGSISSATHYWSWIRQHPGRGLEWIGYIYYTGGTFYNPSLKSRLTISVDTSKNQFSLKLSAVTAADTAVYYCARVIAARPGSTYFDFWGRGTLVTVSS

SEQ ID NO: 673 - DNA, 337 bp, Homo sapiens
  source 1..337: mol_type = other DNA
caatctgccctgactcagcctgcctccgtgtctgggtctcctggacagtcgatcaccatctcctgcactggaaccagcagtgacgttagtggctataactatgtctcctggtaccaacaacacccagacaaagcccccaaactcttgatttatgatgtcactaatcggcccacaggggtttctaatcgcttctctgcctccaagtctggcaacacggcctccctgaccatctctgggctccaggctgaggacgaggctgattattactgcagctcagatacaaatagtattcctcggtatgtggtgttcggcggagggaccaagctgaccgtcctag

SEQ ID NO: 674 - protein, 112 aa, Homo sapiens
QSALTQPASVSGSPGQSITISCTGTSSDVSGYNYVSWYQQHPDKAPKLLIYDVTNRPTGVSNRFSASKSGNTASLTISGLQAEDEADYYCSSDTNSIPRYVVFGGGTKLTVL

SEQ ID NO: 675 - protein, 10 aa, Homo sapiens
GGSISSATHY

SEQ ID NO: 676 - protein, 7 aa, Homo sapiens
IYYTGGT

SEQ ID NO: 677 - protein, 15 aa, Homo sapiens
ARVIAARPGSTYFDF

SEQ ID NO: 678 - protein, 9 aa, Homo sapiens
SSDVSGYNY

SEQ ID NO: 679 - skipped

SEQ ID NO: 680 - protein, 9 aa, Homo sapiens
SSDTNSIPR

SEQ ID NO: 681 - DNA, 394 bp, Homo sapiens
  source 1..394: mol_type = other DNA
gaggtgcagctggtggagtctggggctgaggtgaagaagcctgggtcctcggtgaaggtctcctgcaaggcttctggaggcaccttcagcagctatgctatcaactgggtgcgacaggcccctggacaagggcttgagtggatgggagggatcatccctatctttcgtacgccgcactacgcacagaaattccagggcagagtcacgattaccgcggacgaatctacgggcacagcctacatggagctgagcagcctgcgatctgaagacacggccgtgtattactgtgcgagcccctcttgtggtggtgactgcccccagtacttaaaatcatccaaactagactggtacttcgatctctggggccgtggcaccctggtcaccgtctcctcag

SEQ ID NO: 682 - protein, 131 aa, Homo sapiens
EVQLVESGAEVKKPGSSVKVSCKASGGTFSSYAINWVRQAPGQGLEWMGGIIPIFRTPHYAQKFQGRVTITADESTGTAYMELSSLRSEDTAVYYCASPSCGGDCPQYLKSSKLDWYFDLWGRGTLVTVSS

SEQ ID NO: 683 - DNA, 325 bp, Homo sapiens
  source 1..325: mol_type = other DNA
gtcatctggatgacccagtctccaggcaccctgtctttgtctccaggggaaagagccaccctctcctgcagggccagtcagagtgttagcagcacctacttagcctggtaccagcagaaacctggccaggctcccaggctcctcatctatggtgcatccagcagggccactggcatcccagacaggttcagtggcagtgggtctgggacagacttcactctcaccatcagcagactggaacctgaagattttgcagtgtattactgtcagcactatggtagctcacctctcaccttcggccaagggacacgactggagattaaac

SEQ ID NO: 684 - protein, 108 aa, Homo sapiens
VIWMTQSPGTLSLSPGERATLSCRASQSVSSTYLAWYQQKPGQAPRLLIYGASSRATGIPDRFSGSGSGTDFTLTISRLEPEDFAVYYCQHYGSSPLTFGQGTRLEIK

SEQ ID NO: 685 - protein, 8 aa, Homo sapiens
GGTFSSYA

SEQ ID NO: 686 - protein, 8 aa, Homo sapiens
IIPIFRTP

SEQ ID NO: 687 - protein, 24 aa, Homo sapiens
ASPSCGGDCPQYLKSSKLDWYFDL

SEQ ID NO: 688 - protein, 7 aa, Homo sapiens
QSVSSTY

SEQ ID NO: 689 - skipped

SEQ ID NO: 690 - protein, 9 aa, Homo sapiens
QHYGSSPLT

SEQ ID NO: 691 - DNA, 355 bp, Homo sapiens
  source 1..355: mol_type = other DNA
gaggtgcagctggtggagtctggaggaggcttgatccagcctggggggtccctgagactctcctgtgcagcctctgagatcatcgtcagtaggaactacatgagctgggtccgccaggctccagggaaggggctggagtgggtctcagttatttatagcggtggtagcacgttctacgcagactccgtgaagggccgattcaccatctccagagacaattccaagaacacgctgtatcttcaaatgaacagcctgagagccgaggacacggccgtgtattactgtgcgagagacctcgacgtagtgggaggtactgactactggggccagggaaccctggtcaccgtctcctcag

SEQ ID NO: 692 - protein, 118 aa, Homo sapiens
EVQLVESGGGLIQPGGSLRLSCAASEIIVSRNYMSWVRQAPGKGLEWVSVIYSGGSTFYADSVKGRFTISRDNSKNTLYLQMNSLRAEDTAVYYCARDLDVVGGTDYWGQGTLVTVSS

SEQ ID NO: 693 - DNA, 328 bp, Homo sapiens
  source 1..328: mol_type = other DNA
gaaattgtgttgacacagtctccaggcaccctgtctttgtctccaggggaaagagccaccctctcctgcagggccagtcagagtgttagcagcagctacttagcctggtaccagcagaaacctggccaggctcccaggctcctcatctatggtgcatccagcagggccactggcatcccagacaggttcagtggcagtgggtctgggacagacttcactctcaccatcagcagactggagcctgaagattttgcagtgtattactgtcagcagtatggtagctcaccagggtacacttttggccaggggaccaaagtggatatcaaac

SEQ ID NO: 694 - protein, 109 aa, Homo sapiens
EIVLTQSPGTLSLSPGERATLSCRASQSVSSSYLAWYQQKPGQAPRLLIYGASSRATGIPDRFSGSGSGTDFTLTISRLEPEDFAVYYCQQYGSSPGYTFGQGTKVDIK

SEQ ID NO: 695 - protein, 8 aa, Homo sapiens
EIIVSRNY

SEQ ID NO: 696 - protein, 7 aa, Homo sapiens
IYSGGST

SEQ ID NO: 697 - protein, 12 aa, Homo sapiens
ARDLDVVGGTDY

SEQ ID NO: 698 - protein, 7 aa, Homo sapiens
QSVSSSY

SEQ ID NO: 699 - skipped

SEQ ID NO: 700 - protein, 10 aa, Homo sapiens
QQYGSSPGYT

SEQ ID NO: 701 - DNA, 373 bp, Homo sapiens
  source 1..373: mol_type = other DNA
gaggtgcagctgttggagtcgggcccaggactggtgaagccttcggagaccctgtccctcacctgcaccgtctctggtggctccatcagcagatactcctggtcctggatccggcagcccgccgggaggggactggagtggatcgggcgtatgtatagcagtgggggcaccaactataacccctccctcgagagtcgagtcaccatgtcacttgacacgtccaagaagcagttctccctgaagctgagctctgtgaccgccgcggacacggccgtgtattactgtgcggcggcttcaattgatcaagtatgggggacttatcgtgatgcttttgatatctggggtcaagggacaatggtcaccgtctcttcag

SEQ ID NO: 702 - protein, 124 aa, Homo sapiens
EVQLLESGPGLVKPSETLSLTCTVSGGSISRYSWSWIRQPAGRGLEWIGRMYSSGGTNYNPSLESRVTMSLDTSKKQFSLKLSSVTAADTAVYYCAAASIDQVWGTYRDAFDIWGQGTMVTVSS

SEQ ID NO: 703 - DNA, 322 bp, Homo sapiens
  source 1..322: mol_type = other DNA
gccatccggatgacccagtctccatcctccctggctgcatctgtaggagacagagtcaccatctcttgccgggcaggtcagagcattagcagctttttacattggtatcagcagaaagtagggaaagcccctaagctcctgatctatgatgcgtccagtttgcaaagtggggtcccatcaaggttcagtggcagtggatctgggacagatttcactctcaccatcagcagtctgcaacctgaagattttgcagcttactactgtcaacagagttacgaaaacccgcttactttcggcggagggaccaaagtggatatcaaac

SEQ ID NO: 704 - protein, 107 aa, Homo sapiens
AIRMTQSPSSLAASVGDRVTISCRAGQSISSFLHWYQQKVGKAPKLLIYDASSLQSGVPSRFSGSGSGTDFTLTISSLQPEDFAAYYCQQSYENPLTFGGGTKVDIK

SEQ ID NO: 705 - protein, 8 aa, Homo sapiens
GGSISRYS

SEQ ID NO: 706 - protein, 7 aa, Homo sapiens
MYSSGGT

SEQ ID NO: 707 - protein, 18 aa, Homo sapiens
AAASIDQVWGTYRDAFDI

SEQ ID NO: 708 - protein, 6 aa, Homo sapiens
QSISSF

SEQ ID NO: 709 - skipped

SEQ ID NO: 710 - protein, 9 aa, Homo sapiens
QQSYENPLT

SEQ ID NO: 711 - DNA, 373 bp, Homo sapiens
  source 1..373: mol_type = other DNA
gaagtgcagctggtggagtctggggctgaggtgaagaggcctggggcctcagtgaaggtttcctgcaaggcatctggatacaccttcaccaactactttatgcactgggtgcgacaggcccctggacaagggcttgagtggatgggagttatcaaccctagtgatggtggcgcaagctacccacagaagttccagggcagagtcaccatgaccagggacacgtccacgagcacagtctacatggatctgagcagcctgagatctgaggacacggccgtctattcctgtgcgaggggggcttttgatgttagcggcagctggtacgtcccctttgactactggggccagggaactctggtcaccgtctcctcag

SEQ ID NO: 712 - protein, 124 aa, Homo sapiens
EVQLVESGAEVKRPGASVKVSCKASGYTFTNYFMHWVRQAPGQGLEWMGVINPSDGGASYPQKFQGRVTMTRDTSTSTVYMDLSSLRSEDTAVYSCARGAFDVSGSWYVPFDYWGQGTLVTVSS

SEQ ID NO: 713 - DNA, 340 bp, Homo sapiens
  source 1..340: mol_type = other DNA
cagtctgtcgtgacgcagccgccctcagtgtctggggccccagggcagagggtcaccatctcctgcactgggagcagctccaacatcggggcaggttatgatgtacactggtaccagcagcttccaggagcagcccccaaactcctcatctatggtaacaccaatcggccctcaggggtccctgaccgattctctggctccaagtctggcacctccgcctccctggccatcactgggctccaggctgaggatgaggctgattattactgccagtcctatgacatcaccctgagtggttcggggtatgtcttcggaactgggaccaaggtcaccgtcctag

SEQ ID NO: 714 - protein, 113 aa, Homo sapiens
QSVVTQPPSVSGAPGQRVTISCTGSSSNIGAGYDVHWYQQLPGAAPKLLIYGNTNRPSGVPDRFSGSKSGTSASLAITGLQAEDEADYYCQSYDITLSGSGYVFGTGTKVTVL

SEQ ID NO: 715 - protein, 8 aa, Homo sapiens
GYTFTNYF

SEQ ID NO: 716 - protein, 8 aa, Homo sapiens
INPSDGGA

SEQ ID NO: 717 - protein, 17 aa, Homo sapiens
ARGAFDVSGSWYVPFDY

SEQ ID NO: 718 - protein, 9 aa, Homo sapiens
SSNIGAGYD

SEQ ID NO: 719 - skipped

SEQ ID NO: 720 - protein, 13 aa, Homo sapiens
QSYDITLSGSGYV

SEQ ID NO: 721 - DNA, 367 bp, Homo sapiens
  source 1..367: mol_type = other DNA
caggtgcagctggtggagtctgggggaggcgtggtccagcctgggaggtccctgagactctcctgtgcagcctctggattcaccttcaggacctatgctgtgcactgggtccgccaggctccaggcaaggggccagagtgggtggcagttatatcatatgatggaagtaataaatactacgcagactccgttaagggccgattcaccctctccagagacacttccaagaacacgctgtatctgcaaatgaacagcctgagagctgaggacacggctgtgtattactgtgcgagcagaggggacacggtgactacaggtgacgcttttgatatctggggccaagggacaatggtcaccgtctcttcag

SEQ ID NO: 722 - protein, 122 aa, Homo sapiens
QVQLVESGGGVVQPGRSLRLSCAASGFTFRTYAVHWVRQAPGKGPEWVAVISYDGSNKYYADSVKGRFTLSRDTSKNTLYLQMNSLRAEDTAVYYCASRGDTVTTGDAFDIWGQGTMVTVSS

SEQ ID NO: 723 - DNA, 334 bp, Homo sapiens
  source 1..334: mol_type = other DNA
tcctatgagctgacacagccaccctcggtgtcagtgtccccaggacagacggccaggatcacctgctctggagatgcattgccaaagcaatatacttattggtaccagcagaagccaggccagccccctgtgctggtgatatataaagacagtgagaggccctcagggatccctgagcgattctctggctccagctcagggacaacagtcacgttgaccatcagtggagtccaggcagaagatgaggctgactattactgtcaatcaacagacagcagtgctacttatccgggaaatgtggttttcggcggagggaccaagttgaccgtcctag

SEQ ID NO: 724 - protein, 111 aa, Homo sapiens
SYELTQPPSVSVSPGQTARITCSGDALPKQYTYWYQQKPGQPPVLVIYKDSERPSGIPERFSGSSSGTTVTLTISGVQAEDEADYYCQSTDSSATYPGNVVFGGGTKLTVL

SEQ ID NO: 725 - protein, 8 aa, Homo sapiens
GFTFRTYA

SEQ ID NO: 726 - protein, 8 aa, Homo sapiens
ISYDGSNK

SEQ ID NO: 727 - protein, 15 aa, Homo sapiens
ASRGDTVTTGDAFDI

SEQ ID NO: 728 - protein, 6 aa, Homo sapiens
ALPKQY

SEQ ID NO: 729 - skipped

SEQ ID NO: 730 - protein, 14 aa, Homo sapiens
QSTDSSATYPGNVV

SEQ ID NO: 731 - DNA, 370 bp, Homo sapiens
  source 1..370: mol_type = other DNA
gaggtgcagctggtggagtctgggcctgaggtgaagaagcctgggacctcagtgaaggtctcctgcaaggcgtctggattcagttttagtatgtctgctatgcagtgggtgcgacgggctcgtggacaacgccttgagtggataggatggatcgtccctggcagtggtaacgcaaactacgcgcagaagtttcaggaaagagtcaccattactagggacgagtccacaaacacaggttatatggagttgagcagcctgagatccgaggacacggccgtgtattattgtgcggcccctcattgtaataagaccaactgctatgatgcttttgatatctggggccaagggacaatggtcaccgtctcttcag

SEQ ID NO: 732 - protein, 123 aa, Homo sapiens
EVQLVESGPEVKKPGTSVKVSCKASGFSFSMSAMQWVRRARGQRLEWIGWIVPGSGNANYAQKFQERVTITRDESTNTGYMELSSLRSEDTAVYYCAAPHCNKTNCYDAFDIWGQGTMVTVSS

SEQ ID NO: 733 - DNA, 325 bp, Homo sapiens
  source 1..325: mol_type = other DNA
gccatccggatgacccagtctccaggcaccctgtctttgtctccaggggaaagagccaccctctcctgcagggccagtcagagcgttaggagcagttacttagcctggtaccagcagaaacctggccaggctcccaggctcctcatctatggtgcatccaccagggccactggcatcccagacaggttcagtggcagtgggtctgggacagacttcattctcaccatcaacagactggagcctgaagatcttgcagtctattactgtcagcagtttggtagctcaccatggacgttcggccaagggaccaaagtggatatcaaac

SEQ ID NO: 734 - protein, 108 aa, Homo sapiens
AIRMTQSPGTLSLSPGERATLSCRASQSVRSSYLAWYQQKPGQAPRLLIYGASTRATGIPDRFSGSGSGTDFILTINRLEPEDLAVYYCQQFGSSPWTFGQGTKVDIK

SEQ ID NO: 735 - protein, 8 aa, Homo sapiens
GFSFSMSA

SEQ ID NO: 736 - protein, 8 aa, Homo sapiens
IVPGSGNA

SEQ ID NO: 737 - protein, 16 aa, Homo sapiens
AAPHCNKTNCYDAFDI

SEQ ID NO: 738 - protein, 7 aa, Homo sapiens
QSVRSSY

SEQ ID NO: 739 - skipped

SEQ ID NO: 740 - protein, 9 aa, Homo sapiens
QQFGSSPWT

SEQ ID NO: 741 - DNA, 355 bp, Homo sapiens
  source 1..355: mol_type = other DNA
gaggtgcagctggtggagtctgggggaggtgtggtccagcctggggggtccctgagactctcctgtgcagcctctggaatcatagtcagtgccaactacatgacctgggtccgccaggctccagggaaggggctggaatgggtctcagttatttatcccggtggtagcacattctacgcggactccgtgaagggccgattcaccatctccagagacaactccaagaacacactgtatcttcaaatgaacagcctgagagttgaggactcggctgtgtattactgtgcgagagatttggagctggctggtttcaatgacttctggggtcagggaaccctggtcaccgtctcctcag

SEQ ID NO: 742 - protein, 118 aa, Homo sapiens
EVQLVESGGGVVQPGGSLRLSCAASGIIVSANYMTWVRQAPGKGLEWVSVIYPGGSTFYADSVKGRFTISRDNSKNTLYLQMNSLRVEDSAVYYCARDLELAGFNDFWGQGTLVTVSS

SEQ ID NO: 743 - DNA, 328 bp, Homo sapiens
  source 1..328: mol_type = other DNA
gatgttgtgatgactcagtctccaggcaccctggctttgtctccaggggaaagagccaccctctcctgcaggaccagccagagtgttagcagcaactacttagcctggtaccagcagaaacctggccaggctcccaggctcctcatctatggtgcatccagcagggccactggcatcccagacaggttcagtggcagtgggtctgggacagacttcactctcaccatcagcagactggagcctgaagattttgcagtgtattactgtcagcagtttggtagttcacctcggtacacttttggccaggggaccaaggtggagatcaaac

SEQ ID NO: 744 - protein, 109 aa, Homo sapiens
DVVMTQSPGTLALSPGERATLSCRTSQSVSSNYLAWYQQKPGQAPRLLIYGASSRATGIPDRFSGSGSGTDFTLTISRLEPEDFAVYYCQQFGSSPRYTFGQGTKVEIK

SEQ ID NO: 745 - protein, 8 aa, Homo sapiens
GIIVSANY

SEQ ID NO: 746 - protein, 7 aa, Homo sapiens
IYPGGST

SEQ ID NO: 747 - protein, 12 aa, Homo sapiens
ARDLELAGFNDF

SEQ ID NO: 748 - protein, 7 aa, Homo sapiens
QSVSSNY

SEQ ID NO: 749 - skipped

SEQ ID NO: 750 - protein, 10 aa, Homo sapiens
QQFGSSPRYT

SEQ ID NO: 751 - DNA, 355 bp, Homo sapiens
  source 1..355: mol_type = other DNA
caggtgcagctggtggagtctgggggaggtgtggtccagcctggggggtccctgagactctcctgtgcagcctctggagtcaccgtcagtagcaactacatgagctgggtccgccaggctccagggaaggggctggagtgggtctcagttctttatgccggtggtagcacattctacgcagactccgtgaagggccgattcaccatctccagagacaattccaagaacacgctgtatcttcaaatgaacagcctgagagctgaggacacggctgcgtattactgtgcgagagatttggcagtggctggtttccttgactcctggggccagggaaccctggtcaccgtctcctcag

SEQ ID NO: 752 - protein, 118 aa, Homo sapiens
QVQLVESGGGVVQPGGSLRLSCAASGVTVSSNYMSWVRQAPGKGLEWVSVLYAGGSTFYADSVKGRFTISRDNSKNTLYLQMNSLRAEDTAAYYCARDLAVAGFLDSWGQGTLVTVSS

SEQ ID NO: 753 - DNA, 328 bp, Homo sapiens
  source 1..328: mol_type = other DNA
gatattgtgatgacccagtctccgggcaccctgtctttgtctccaggggaaagagccaccctctcctgcagggccagtcagggtgttagcagcatctacttagcctggtaccagcagaaacctggccaggctcccaggctcgtcctctatggcgcatccagtagggccactggcatcccagacaggttcagtggcagtgggtctgggacagacttcactctcaccatcagcagactggagcctgaagattttgcagtgtattactgtcagcagtatggtagctcacctcggtacacttttggccaggggaccaaggtggagatcaaac

SEQ ID NO: 754 - protein, 109 aa, Homo sapiens
DIVMTQSPGTLSLSPGERATLSCRASQGVSSIYLAWYQQKPGQAPRLVLYGASSRATGIPDRFSGSGSGTDFTLTISRLEPEDFAVYYCQQYGSSPRYTFGQGTKVEIK

SEQ ID NO: 755 - protein, 8 aa, Homo sapiens
GVTVSSNY

SEQ ID NO: 756 - protein, 7 aa, Homo sapiens
LYAGGST

SEQ ID NO: 757 - protein, 12 aa, Homo sapiens
ARDLAVAGFLDS

SEQ ID NO: 758 - protein, 7 aa, Homo sapiens
QGVSSIY

SEQ ID NO: 759 - skipped

SEQ ID NO: 760 - protein, 10 aa, Homo sapiens
QQYGSSPRYT

SEQ ID NO: 761 - DNA, 351 bp, Homo sapiens
  source 1..351: mol_type = other DNA
caggtgcagctggtggagtctggaggaggcttgatccagccgggggggtccctgagactctcctgtgcagcctctgggatcaccgtcagtagcaactacatgacctgggtccgccaggctccagggaaggggctggagtgggtctcacttctttatgccggtggtagcgcattctatgctgactccgtgaagggccgattcaccatctccagagacaattccaagaacacgctgtatcttctaatgaacagcctgagagtcggcgacacggccgtttattactgtgcgagagatctccaggtctacggtatggacgtctggggccaagggaccacggtcaccgtctcctca

SEQ ID NO: 762 - protein, 117 aa, Homo sapiens
QVQLVESGGGLIQPGGSLRLSCAASGITVSSNYMTWVRQAPGKGLEWVSLLYAGGSAFYADSVKGRFTISRDNSKNTLYLLMNSLRVGDTAVYYCARDLQVYGMDVWGQGTTVTVSS

SEQ ID NO: 763 - DNA, 322 bp, Homo sapiens
  source 1..322: mol_type = other DNA
tcctatgagctgactcagccaccctcggtgtcagtggccccaggacagacggccaggattacctgtgggggaaacaacgatggagctaaaagtgtgcactggtaccagcagaagccaggccaggcccctgtgctggtcgtctatgatgatagcgaccggccctcagggatccctgaacgattctctggctccaactctgggaacacggccaccctgaccatcaccaggatcgaagccggggatgaggccgactattactgtcaggtctgggatagtagtcgtgatcatgtcttcggaactgggaccaaggtcaccgtcctgg

SEQ ID NO: 764 - protein, 107 aa, Homo sapiens
SYELTQPPSVSVAPGQTARITCGGNNDGAKSVHWYQQKPGQAPVLVVYDDSDRPSGIPERFSGSNSGNTATLTITRIEAGDEADYYCQVWDSSRDHVFGTGTKVTVL

SEQ ID NO: 765 - protein, 8 aa, Homo sapiens
GITVSSNY

SEQ ID NO: 766 - protein, 7 aa, Homo sapiens
LYAGGSA

SEQ ID NO: 767 - protein, 11 aa, Homo sapiens
ARDLQVYGMDV

SEQ ID NO: 768 - protein, 6 aa, Homo sapiens
NDGAKS

SEQ ID NO: 769 - skipped

SEQ ID NO: 770 - protein, 10 aa, Homo sapiens
QVWDSSRDHV

SEQ ID NO: 771 - DNA, 351 bp, Homo sapiens
  source 1..351: mol_type = other DNA
gaggtgcagctggtggagtctgggggaggcttggtccagcctggggggtccctgaggctctcctgtgaagcctctgaaataaccgtcagtagcaactacatgaattgggtccgccaggctccagggaaggggctggagtgggtctcagttctttttgccggtggtactacatactacgcagactccgtgaagggccgattcaccatctccagagacaattccaagaacacactgtatcttcaaatgaacaccctgagaattgaggacacggctatttattactgtgcgagagatctcgtcgcatacggtgtggacgtctggggccaagggaccacggtcaccgtctcctca

SEQ ID NO: 772 - protein, 117 aa, Homo sapiens
EVQLVESGGGLVQPGGSLRLSCEASEITVSSNYMNWVRQAPGKGLEWVSVLFAGGTTYYADSVKGRFTISRDNSKNTLYLQMNTLRIEDTAIYYCARDLVAYGVDVWGQGTTVTVSS

SEQ ID NO: 773 - DNA, 322 bp, Homo sapiens
  source 1..322: mol_type = other DNA
gccatccagatgacccagtctccatccttcctgtctgcatctgtaggagacagagtcaccatcacttgccgggccagtcagggcattagcggtgatttagcctggtatcagcaaaaaccagggaaagcccctaagctcctgatctatgctgcatccactttgcaaagtggggtcccatcaaggttcagcggcagtggatctgggacagaattcactctcacaatcagcagcctgcagcctgaagattttgcaacttattactgtcaacaccttaatagttaccctctcacgttcggcggagggaccaaggtggaaatcaaac

SEQ ID NO: 774 - protein, 107 aa, Homo sapiens
AIQMTQSPSFLSASVGDRVTITCRASQGISGDLAWYQQKPGKAPKLLIYAASTLQSGVPSRFSGSGSGTEFTLTISSLQPEDFATYYCQHLNSYPLTFGGGTKVEIK

SEQ ID NO: 775 - protein, 8 aa, Homo sapiens
EITVSSNY

SEQ ID NO: 776 - protein, 7 aa, Homo sapiens
LFAGGTT

SEQ ID NO: 777 - protein, 11 aa, Homo sapiens
ARDLVAYGVDV

SEQ ID NO: 778 - protein, 6 aa, Homo sapiens
QGISGD

SEQ ID NO: 779 - skipped

SEQ ID NO: 780 - protein, 9 aa, Homo sapiens
QHLNSYPLT

SEQ ID NO: 781 - DNA, 352 bp, Homo sapiens
  source 1..352: mol_type = other DNA
caggtacagctgcaggagtcgggcccaggactggtgaagtcttcacagaccctgtccctcacgtgcactgtctctggtgactccatcagccgtggtggttactactggagctggatccgccagcacccagggaagggcctggagtggattgggtccatctattacagtgggagcacctactacaacccgtccctcaagagtcgatttaccatatcagtagacacgtctaagaaccagttctccctgaagctgagctctgtgactgccgcggacacggccgtgtatcactgtgcgagagaaattggtttccttgactactggggccagggaaccctggtcaccgtctcctcag

SEQ ID NO: 782 - protein, 117 aa, Homo sapiens
QVQLQESGPGLVKSSQTLSLTCTVSGDSISRGGYYWSWIRQHPGKGLEWIGSIYYSGSTYYNPSLKSRFTISVDTSKNQFSLKLSSVTAADTAVYHCAREIGFLDYWGQGTLVTVSS

SEQ ID NO: 783 - DNA, 325 bp, Homo sapiens
  source 1..325: mol_type = other DNA
gccatccagatgacccagtctccatcctccctgtctgcatctgtaggagacagagtcaccatcacttgccgggcgagtcaggccattagcaattctttagcctggtatcagcagaaaccagggaaagcccctaagctcctactctatgctgcatccacattggaaagtggggtcccatccaggttcagtggcagtggatctgggacggatttcactctcaccatcagcagcctgcagcctgaagattttgcaacttatttctgtcagcagtactatagtacccctccgaggacgttcggccaagggaccaaagtggatatcaaac

SEQ ID NO: 784 - protein, 108 aa, Homo sapiens
AIQMTQSPSSLSASVGDRVTITCRASQAISNSLAWYQQKPGKAPKLLLYAASTLESGVPSRFSGSGSGTDFTLTISSLQPEDFATYFCQQYYSTPPRTFGQGTKVDIK

SEQ ID NO: 785 - protein, 10 aa, Homo sapiens
GDSISRGGYY

SEQ ID NO: 786 - protein, 7 aa, Homo sapiens
IYYSGST

SEQ ID NO: 787 - protein, 9 aa, Homo sapiens
AREIGFLDY

SEQ ID NO: 788 - protein, 6 aa, Homo sapiens
QAISNS

SEQ ID NO: 789 - skipped

SEQ ID NO: 790 - protein, 10 aa, Homo sapiens
QQYYSTPPRT

SEQ ID NO: 791 - DNA, 382 bp, Homo sapiens
  source 1..382: mol_type = other DNA
caggtgcagctggtggagtctggggctgaggtgaagaagcctgggtcctcggtgaaggtctcctgcaaggcttctggaggcaccttcagcagccatggtgtcatctgggtgcgacaggcccctggacaagggcttgagtggatgggagggatcatccccatctttcccacagcaaactacgcacagaaattccagggcagagtcacaattaccgcggacaaaccctccaacacagcctacatggagctgagcagcctgagatctgaggacacggccgtatattactgtgcgagggcaaggggagaacatgattccgtttggggaagttttcattactattttgactactggggccagggaaccctggtcaccgtctcctcag

SEQ ID NO: 792 - protein, 127 aa, Homo sapiens
QVQLVESGAEVKKPGSSVKVSCKASGGTFSSHGVIWVRQAPGQGLEWMGGIIPIFPTANYAQKFQGRVTITADKPSNTAYMELSSLRSEDTAVYYCARARGEHDSVWGSFHYYFDYWGQGTLVTVSS

SEQ ID NO: 793 - DNA, 325 bp, Homo sapiens
  source 1..325: mol_type = other DNA
cgtcattggatgacccagtctccagccaccctgtctgtgtctccaggggaaagagccaccctctcctgcagggccagtcaaagtattggcagcaacttagcctggtaccagcagaaacctggtcaggctcccaggctcctcatctatggtgcagccaccagggccactggtatcccagccaggttcagtggcagtgggtctgggacagagttcactctcaccatcagcagcctgcagtctgaagattttgcagtttactactgtcagcagtataatgactggcctccgaggacgttcggccaagggaccaaggtggaaatcaaac

SEQ ID NO: 794 - protein, 108 aa, Homo sapiens
RHWMTQSPATLSVSPGERATLSCRASQSIGSNLAWYQQKPGQAPRLLIYGAATRATGIPARFSGSGSGTEFTLTISSLQSEDFAVYYCQQYNDWPPRTFGQGTKVEIK

SEQ ID NO: 795 - protein, 8 aa, Homo sapiens
GGTFSSHG

SEQ ID NO: 796 - protein, 8 aa, Homo sapiens
IIPIFPTA

SEQ ID NO: 797 - protein, 20 aa, Homo sapiens
ARARGEHDSVWGSFHYYFDY

SEQ ID NO: 798 - protein, 6 aa, Homo sapiens
QSIGSN

SEQ ID NO: 799 - skipped

SEQ ID NO: 800 - protein, 10 aa, Homo sapiens
QQYNDWPPRT

SEQ ID NO: 801 - DNA, 369 bp, Homo sapiens
  source 1..369: mol_type = other DNA
caggtgcagctggtggagtctgggggaggcttggtacagcctggcaggtccctgagactctcctgtgcagcctctggattcacgtttgatgattatgccatgcactgggtccggcaagttccagggaagggcctggagtgggtctcaggaattagttggaacagtggtagcatagtctatgcggactttgtgaagggccgattcaccatcgccagagacaacgccaagaactccctgtttctgcaaatgaacagtctgagagctgaggacacggccttgtattactgtgcaaaaagtacggctctacgtcatcagtactactacggtatggacgtctggggccaagggaccacggtcaccgtctcctca

SEQ ID NO: 802 - protein, 123 aa, Homo sapiens
QVQLVESGGGLVQPGRSLRLSCAASGFTFDDYAMHWVRQVPGKGLEWVSGISWNSGSIVYADFVKGRFTIARDNAKNSLFLQMNSLRAEDTALYYCAKSTALRHQYYYGMDVWGQGTTVTVSS

SEQ ID NO: 803 - DNA, 322 bp, Homo sapiens
  source 1..322: mol_type = other DNA
gccatccagatgacccagtctccatcctccctgtctgcatctgtaggagacagagtcaccatcacttgccggacaagtcagaccattagcagctatttaaattggtatcagcagaaaccagggaaagcccctaagctcctgatatatgacgcatccagtttgcaaagtggggtcccatcaaggttcagtggcagtggatatgggacagatttcactctcaccatcagcagtctgcaacctgaagattttgcaacttacttctgtcaacagagttacaataccccgtacgcttttggccaggggaccaaggtggagatcaaac

SEQ ID NO: 804 - protein, 107 aa, Homo sapiens
AIQMTQSPSSLSASVGDRVTITCRTSQTISSYLNWYQQKPGKAPKLLIYDASSLQSGVPSRFSGSGYGTDFTLTISSLQPEDFATYFCQQSYNTPYAFGQGTKVEIK

SEQ ID NO: 805 - protein, 8 aa, Homo sapiens
GFTFDDYA

SEQ ID NO: 806 - protein, 8 aa, Homo sapiens
ISWNSGSI

SEQ ID NO: 807 - protein, 16 aa, Homo sapiens
AKSTALRHQYYYGMDV

SEQ ID NO: 808 - protein, 6 aa, Homo sapiens
QTISSY

SEQ ID NO: 809 - skipped

SEQ ID NO: 810 - protein, 9 aa, Homo sapiens
QQSYNTPYA

SEQ ID NO: 811 - DNA, 358 bp, Homo sapiens
  source 1..358: mol_type = other DNA
caggttcagctggtgcagtctggcactgaggtgaagaagcctggggcctcagtgaaggtctcctgcaaggcttctgattacacctttaccaggtttggtatcatctgggtgcgacaggcccctggacaagggcttgagtggatgggacagatcaacccttacaatggtaacacagactatgcacagaagttccagggcagagtcaccttgaccacagacacatccacgaacacagcctacatggaactgaggagcctgagatctgacgacacggccgtgtattattgtgcgaggtccgctgggagccctaccggccttgactactggggccagggaaccctggtcaccgtctcctcag

SEQ ID NO: 812 - protein, 119 aa, Homo sapiens
QVQLVQSGTEVKKPGASVKVSCKASDYTFTRFGIIWVRQAPGQGLEWMGQINPYNGNTDYAQKFQGRVTLTTDTSTNTAYMELRSLRSDDTAVYYCARSAGSPTGLDYWGQGTLVTVSS

SEQ ID NO: 813 - DNA, 331 bp, Homo sapiens
  source 1..331: mol_type = other DNA
cagtctgtcgtgacgcagccaccctcggtgtctgaagcccccaggcagagggtcaccatctcctgttctggaagcaactccaacatcggaaataatgctgtaaactggtaccagcagctcccaggaaaggctcccaaactcctcgtctattatgatgatctgctgccctcaggggtctctgaccgattctctggctccaagtctggcacctcagcctccctggccatcagtgggctccagtctgaggataaggctgattattactgtgcagcatgggatgacagcctgaatgccttggtgttcggcggagggaccaagctgaccgtcctag

SEQ ID NO: 814 - protein, 110 aa, Homo sapiens
QSVVTQPPSVSEAPRQRVTISCSGSNSNIGNNAVNWYQQLPGKAPKLLVYYDDLLPSGVSDRFSGSKSGTSASLAISGLQSEDKADYYCAAWDDSLNALVFGGGTKLTVL

SEQ ID NO: 815 - protein, 8 aa, Homo sapiens
DYTFTRFG

SEQ ID NO: 816 - protein, 8 aa, Homo sapiens
INPYNGNT

SEQ ID NO: 817 - protein, 12 aa, Homo sapiens
ARSAGSPTGLDY

SEQ ID NO: 818 - protein, 8 aa, Homo sapiens
NSNIGNNA

SEQ ID NO: 819 - skipped

SEQ ID NO: 820 - protein, 11 aa, Homo sapiens
AAWDDSLNALV

SEQ ID NO: 821 - DNA, 354 bp, Homo sapiens
  source 1..354: mol_type = other DNA
gaagtgcagctgttggagtctgggggaggcttggtccagcctggggggtccctgagactctcctgtgtagcctctggactcaccgtcagtagcaactacatgagctgggtccgccaggctccagggaaggggctggagtgggtctcaattatttatcccggtggtaccacatactacgcagactccgtgaagggcagattcaccacctccagagacaaatccaagaacacgctgtatcttcaaatgaacagcctgagagccgaggacacggctgtgtattactgtgcgagagatctggcagtggctgggggtatggacgtctggggccaagggaccacggtcaccgtctcctca

SEQ ID NO: 822 - protein, 118 aa, Homo sapiens
EVQLLESGGGLVQPGGSLRLSCVASGLTVSSNYMSWVRQAPGKGLEWVSIIYPGGTTYYADSVKGRFTTSRDKSKNTLYLQMNSLRAEDTAVYYCARDLAVAGGMDVWGQGTTVTVSS

SEQ ID NO: 823 - DNA, 322 bp, Homo sapiens
  source 1..322: mol_type = other DNA
gaaatagtgatgacgcagtctccatcctccctgtctgcatctgtaggagacagagttaccatcacttgccgggcaagtcagggcattggaaatgatttagggtggtatcagcagaaaccagggaaagcccctaaagtcctgatttatgctgcatccaatttacaaagtggggtcccatcaaggttcagcggcagtggatctggcacagatttcactctcaccatcagcagcctgcagcctgaagattttgcaacttattactgtctacaagattccaattatccctacacttttggccaggggaccaaggtggagatcaaac

SEQ ID NO: 824 - protein, 107 aa, Homo sapiens
EIVMTQSPSSLSASVGDRVTITCRASQGIGNDLGWYQQKPGKAPKVLIYAASNLQSGVPSRFSGSGSGTDFTLTISSLQPEDFATYYCLQDSNYPYTFGQGTKVEIK

SEQ ID NO: 825 - protein, 8 aa, Homo sapiens
GLTVSSNY

SEQ ID NO: 826 - protein, 7 aa, Homo sapiens
IYPGGTT

SEQ ID NO: 827 - protein, 12 aa, Homo sapiens
ARDLAVAGGMDV

SEQ ID NO: 828 - protein, 6 aa, Homo sapiens
QGIGND

SEQ ID NO: 829 - skipped

SEQ ID NO: 830 - protein, 9 aa, Homo sapiens
LQDSNYPYT

SEQ ID NO: 831 - DNA, 355 bp, Homo sapiens
  source 1..355: mol_type = other DNA
gaagtgcagctggtggagtctgggggaggcttggtccagcctggggggtccctgagactctcctgtgcagcctctggagtcatcgtcagtagcaactacatgagctgggtccgccaggctccagggaaggggctgcaatgggtctcagttatttatagcggtggtagcactttctacgcagactccgtgaagggcagattcaccatctccagagacaattccaagaacacgttgtatcttcaaatgaacagcctgagagccgaggacacggctgtgtattactgtgcgagagatttgttagaggcaggcggaactgactactggggccagggaaccctggtcaccgtctcctcag

SEQ ID NO: 832 - protein, 118 aa, Homo sapiens
EVQLVESGGGLVQPGGSLRLSCAASGVIVSSNYMSWVRQAPGKGLQWVSVIYSGGSTFYADSVKGRFTISRDNSKNTLYLQMNSLRAEDTAVYYCARDLLEAGGTDYWGQGTLVTVSS

SEQ ID NO: 833 - DNA, 325 bp, Homo sapiens
  source 1..325: mol_type = other DNA
gatgttgtgatgactcagtctccaggcaccctgtctttgtctccaggggaaagagccaccctctcctgcagggccagtcagtttattggcagctcctacttagcctggtaccagcagaaacctggccaggctcccaggctcctcatctatggtgcatccaacagggccactggcgtcccagacaggttcagtggcagtgggtctgggacagacttcactctcaccatcagcagactggagcctgaagattttgcagtgtattactgtcagcagtatgggagtgcacctgggacgttcggccaagggaccaaggtggaaatcaaac

SEQ ID NO: 834 - protein, 108 aa, Homo sapiens
DVVMTQSPGTLSLSPGERATLSCRASQFIGSSYLAWYQQKPGQAPRLLIYGASNRATGVPDRFSGSGSGTDFTLTISRLEPEDFAVYYCQQYGSAPGTFGQGTKVEIK

SEQ ID NO: 835 - protein, 8 aa, Homo sapiens
GVIVSSNY

SEQ ID NO: 836 - protein, 7 aa, Homo sapiens
IYSGGST

SEQ ID NO: 837 - protein, 12 aa, Homo sapiens
ARDLLEAGGTDY

SEQ ID NO: 838 - protein, 7 aa, Homo sapiens
QFIGSSY

SEQ ID NO: 839 - skipped

SEQ ID NO: 840 - protein, 9 aa, Homo sapiens
QQYGSAPGT

SEQ ID NO: 841 - DNA, 351 bp, Homo sapiens
  source 1..351: mol_type = other DNA
caggtgcagctggtggagtctggaggaggcttggtccagcctggggggtccctgagactctcctgtgcagcctctggtttaatcgtcagtaggaactacatgagctgggtccgccaggctccagggaaggggctggagtgggtctcacttatttatgccggtggtagcacattctactcagactccgtgaagggccgattcaccatctccagacacagttccgagaacacgctgtttcttcaaatgaacagcctgagagctgaggacacggctgtgtattattgtgcgagagatctagtccactacggcatggacgtctggggccaagggaccacggtcaccgtctcctca

SEQ ID NO: 842 - protein, 117 aa, Homo sapiens
QVQLVESGGGLVQPGGSLRLSCAASGLIVSRNYMSWVRQAPGKGLEWVSLIYAGGSTFYSDSVKGRFTISRHSSENTLFLQMNSLRAEDTAVYYCARDLVHYGMDVWGQGTTVTVSS

SEQ ID NO: 843 - DNA, 331 bp, Homo sapiens
  source 1..331: mol_type = other DNA
aattttatgctgactcagcctgcctccgtgtctgggtctcctggacagtcgatcaccatctcctgcactggaaccagcagtgacgttggtggttataactatgtctcctggtaccaacagcacccaggcaaagcccccaaactcatgatttatgatgtcagtaatcggccctcaggggtttctaatcgcttctctggctccaactctggcaacacggcctccctcaccatctctgggctccaggctgaggacgaggctgattattactgcagctcatatacaagcggcagcacttgggtgttcggcggagggaccaagctgaccgtcctag

SEQ ID NO: 844 - protein, 110 aa, Homo sapiens
NFMLTQPASVSGSPGQSITISCTGTSSDVGGYNYVSWYQQHPGKAPKLMIYDVSNRPSGVSNRFSGSNSGNTASLTISGLQAEDEADYYCSSYTSGSTWVFGGGTKLTVL

SEQ ID NO: 845 - protein, 8 aa, Homo sapiens
GLIVSRNY

SEQ ID NO: 846 - protein, 7 aa, Homo sapiens
IYAGGST

SEQ ID NO: 847 - protein, 11 aa, Homo sapiens
ARDLVHYGMDV

SEQ ID NO: 848 - protein, 9 aa, Homo sapiens
SSDVGGYNY

SEQ ID NO: 849 - skipped

SEQ ID NO: 850 - protein, 10 aa, Homo sapiens
SSYTSGSTWV

SEQ ID NO: 851 - DNA, 390 bp, Homo sapiens
  source 1..390: mol_type = other DNA
gaagtgcagctggtggagtctggggctgaggtgaagaagcctgggtcctcagtgaaggtctcctgcaaggcttctggaggcaccttcagcaggtatgctatcagctgggtgcgacaggcccctggacaaggacttgagtggatgggagggatcatccctatctttgatgcaacaaactacgcacagaagttccatgacagagtcaccattaccgcggacaaatccgcgagcacagcctacatggaactgagcagcctgagatctgacgacacggccgtgtattactgtgcgagagaacggacatattgtagtggtggtacttgctacggaggatacttctactacggtatggacgtctggggccaaggaaccacggtcaccgtctcctca

SEQ ID NO: 852 - protein, 130 aa, Homo sapiens
EVQLVESGAEVKKPGSSVKVSCKASGGTFSRYAISWVRQAPGQGLEWMGGIIPIFDATNYAQKFHDRVTITADKSASTAYMELSSLRSDDTAVYYCARERTYCSGGTCYGGYFYYGMDVWGQGTTVTVSS

SEQ ID NO: 853 - DNA, 331 bp, Homo sapiens
  source 1..331: mol_type = other DNA
cagtctgtgctgactcagccaccctcagcgtctgggacccccgggcagagggtcaccatctcttgttctggaagcagctccaacatcggaggcgatattgtaaactggtacctccagctcccagggacggcccccaaactcctcatttatagtaataatcagcggccctcaggcgtccctgaccgattctctggctccaggtctggcacctcagcctccctggccatcagtgggctccagtctgaggatgagggttattattactgtgcagcatgggatgacagcctgaatggtcaagtgttcggcggagggaccaagctgaccgtcctag

SEQ ID NO: 854 - protein, 110 aa, Homo sapiens
QSVLTQPPSASGTPGQRVTISCSGSSSNIGGDIVNWYLQLPGTAPKLLIYSNNQRPSGVPDRFSGSRSGTSASLAISGLQSEDEGYYYCAAWDDSLNGQVFGGGTKLTVL

SEQ ID NO: 855 - protein, 8 aa, Homo sapiens
GGTFSRYA

SEQ ID NO: 856 - protein, 8 aa, Homo sapiens
IIPIFDAT

SEQ ID NO: 857 - protein, 23 aa, Homo sapiens
ARERTYCSGGTCYGGYFYYGMDV

SEQ ID NO: 858 - protein, 8 aa, Homo sapiens
SSNIGGDI

SEQ ID NO: 859 - skipped

SEQ ID NO: 860 - protein, 11 aa, Homo sapiens
AAWDDSLNGQV

SEQ ID NO: 861 - DNA, 384 bp, Homo sapiens
  source 1..384: mol_type = other DNA
gaggtgcagctggtgcagtctggggctgaggtgaagaagcctgggtcctcggtgaaggtctcctgcaaggcttctggaggcaccttcagtagctatggtatcagctgggtgcgacaggcccctggactagggcttgagtggatggggggggtcatccctatcctaagtgcaaaacactacgcgcagcggttccagggcagagtcacgatcaccgcggacaagtccacgggcacagcctacatggagctgagcagcctgagatctgaggacacggccgtatactactgtgcgagagatatccttcatcatgacgacctttgggggaggttctactacgacggtatggacgtctggggccaagggaccacggtcaccgtctcctca

SEQ ID NO: 862 - protein, 128 aa, Homo sapiens
EVQLVQSGAEVKKPGSSVKVSCKASGGTFSSYGISWVRQAPGLGLEWMGGVIPILSAKHYAQRFQGRVTITADKSTGTAYMELSSLRSEDTAVYYCARDILHHDDLWGRFYYDGMDVWGQGTTVTVSS

SEQ ID NO: 863 - DNA, 331 bp, Homo sapiens
  source 1..331: mol_type = other DNA
cagtctgtcgtgacgcagccaccctcagcgtctgggacccccgggcagagggtcaccatctcttgttctggaagcagctccgacatcggaagtaatactgtaaactggtaccagcagctcccaggaacggcccccaaactcctcatctatactaataatcagcggccctcaggggtccctgaccgattctctggctccaagtctggcacctcagcctccctggccatcactgggctccagtctgaggatgaggctgattatttctgtgcagcatgggatgaaagcctgaatggtcgagtgttcggcggagggaccaagctgaccgtcctag

SEQ ID NO: 864 - protein, 110 aa, Homo sapiens
QSVVTQPPSASGTPGQRVTISCSGSSSDIGSNTVNWYQQLPGTAPKLLIYTNNQRPSGVPDRFSGSKSGTSASLAITGLQSEDEADYFCAAWDESLNGRVFGGGTKLTVL

SEQ ID NO: 865 - protein, 8 aa, Homo sapiens
GGTFSSYG

SEQ ID NO: 866 - protein, 8 aa, Homo sapiens
VIPILSAK

SEQ ID NO: 867 - protein, 21 aa, Homo sapiens
ARDILHHDDLWGRFYYDGMDV

SEQ ID NO: 868 - protein, 8 aa, Homo sapiens
SSDIGSNT

SEQ ID NO: 869 - skipped

SEQ ID NO: 870 - protein, 11 aa, Homo sapiens
AAWDESLNGRV

SEQ ID NO: 871 - DNA, 349 bp, Homo sapiens
  source 1..349: mol_type = other DNA
gaagtgcaactggtggagtctgggggaggcgtggtccagcctgggaggtccctgagactctcctgtgcagcgtctggattcaccttcagtaactatggcatgcactgggtccgccaggctccaggcaagggactggagtgggtggcagtttattggtatgatggaggtaataaattctatgcagactccgtgaagggccgattcaccatctccagagacaattccaagaatacgttgtatctgcaaatgaacagcctgagagtcgaggacacggctgtttattactgtgcgagagatacggctcctccggactactggggccagggaaccctggtcaccgtctcctcag

SEQ ID NO: 872 - protein, 116 aa, Homo sapiens
EVQLVESGGGVVQPGRSLRLSCAASGFTFSNYGMHWVRQAPGKGLEWVAVYWYDGGNKFYADSVKGRFTISRDNSKNTLYLQMNSLRVEDTAVYYCARDTAPPDYWGQGTLVTVSS

SEQ ID NO: 873 - DNA, 328 bp, Homo sapiens
  source 1..328: mol_type = other DNA
gccatccggatgacccagtctccaggcaccctgtctttgtctccaggggaaagagccaccctctcctgcagggccagtcagagtattagtagcagcttcttagcctggtaccagcagaaacctggccaggctcccaggctcctcatctatggtgcatccagcagggccactggcatcccagacaggttcagtggcagtgggtctgggacagacttcactctcaccatcagcagactggagcctgaagattttgcagtgtattactgtcagcagtatggtacctcaccaaggctcactttcggcggagggaccaaagtggatatcaaac

SEQ ID NO: 874 - protein, 109 aa, Homo sapiens
AIRMTQSPGTLSLSPGERATLSCRASQSISSSFLAWYQQKPGQAPRLLIYGASSRATGIPDRFSGSGSGTDFTLTISRLEPEDFAVYYCQQYGTSPRLTFGGGTKVDIK

SEQ ID NO: 875 - protein, 8 aa, Homo sapiens
GFTFSNYG

SEQ ID NO: 876 - protein, 8 aa, Homo sapiens
YWYDGGNK

SEQ ID NO: 877 - protein, 9 aa, Homo sapiens
ARDTAPPDY

SEQ ID NO: 878 - protein, 7 aa, Homo sapiens
QSISSSF

SEQ ID NO: 879 - skipped

SEQ ID NO: 880 - protein, 10 aa, Homo sapiens
QQYGTSPRLT

SEQ ID NO: 881 - DNA, 349 bp, Homo sapiens
  source 1..349: mol_type = other DNA
gaggtgcagctgttggagtctgggggaggcgtggtccagcctggaaggtccctgagactctcctgtgcagcgtctggattcaaattcagtgactatggcatgcactgggtccgccaggctccaggcaaggggctggagtgggtggcagtttattggtatgatggaggtactaaattctatgcagactccgtgaagggccgattcaccatctccagagacaattccaagaatacgttgtatctgcaaatgagcagcctgagagtcgaggacacggctgtttattactgtgcgagagatacggctcctccggactactggggccagggaaccctggtcaccgtctcctcag

SEQ ID NO: 882 - protein, 116 aa, Homo sapiens
EVQLLESGGGVVQPGRSLRLSCAASGFKFSDYGMHWVRQAPGKGLEWVAVYWYDGGTKFYADSVKGRFTISRDNSKNTLYLQMSSLRVEDTAVYYCARDTAPPDYWGQGTLVTVSS

SEQ ID NO: 883 - DNA, 328 bp, Homo sapiens
  source 1..328: mol_type = other DNA
gaaattgtgttgacgcagtctccaggcaccctgtctttgtctccaggggaaagagccaccctctcctgcagggccagtcagagtattagtagcaacttcttagcctggtaccagcagaaacctggccaggctcccaggctcctcatctatggtgcatccagcagggccactggcatcccagacaggttcagtggcagtgggtctgggacagacttcactctcaccatcagcagactggagcctgaagattttgcagtgtattactgtcagcagtatggtacctcaccaaggctcactttcggcggagggaccaaagtggatatcaaac

SEQ ID NO: 884 - protein, 109 aa, Homo sapiens
EIVLTQSPGTLSLSPGERATLSCRASQSISSNFLAWYQQKPGQAPRLLIYGASSRATGIPDRFSGSGSGTDFTLTISRLEPEDFAVYYCQQYGTSPRLTFGGGTKVDIK

SEQ ID NO: 885 - protein, 8 aa, Homo sapiens
GFKFSDYG

SEQ ID NO: 886 - protein, 8 aa, Homo sapiens
YWYDGGTK

SEQ ID NO: 887 - protein, 9 aa, Homo sapiens
ARDTAPPDY

SEQ ID NO: 888 - protein, 7 aa, Homo sapiens
QSISSNF

SEQ ID NO: 889 - skipped

SEQ ID NO: 890 - protein, 10 aa, Homo sapiens
QQYGTSPRLT

SEQ ID NO: 891 - DNA, 369 bp, Homo sapiens
  source 1..369: mol_type = other DNA
caggttcagctggtgcagtctggggctgaggtgaagaagcctgggtcctcggtgaaggtctcctgcaaggcttctggaggcaccttcagcagttatggtatcaggtgggtgcgacaggcccctggacaagggcttgagtggatgggagggatcatccccgtgtttggtgcaacaaactacgcacagaagttccaggacagagtcacaattaccgcggacaaatccacggccacagcctacatggaattgagtagcctgaaatctgacgacacggccgtgtatttttgtgcgagagatgcccttagtgccagtggctggacgggcccctttgactcgtggggccagggaaccctggtcaccgtctcctca

SEQ ID NO: 892 - protein, 123 aa, Homo sapiens
QVQLVQSGAEVKKPGSSVKVSCKASGGTFSSYGIRWVRQAPGQGLEWMGGIIPVFGATNYAQKFQDRVTITADKSTATAYMELSSLKSDDTAVYFCARDALSASGWTGPFDSWGQGTLVTVSS

SEQ ID NO: 893 - DNA, 337 bp, Homo sapiens
  source 1..337: mol_type = other DNA
cagtctgtgttgacgcagccgccctcagtgtctggggccccggggcagagggtcaccatctcctgcactgggagcagctccaacatcggggcagattatgatgtacactggtaccagcaacttccaggagcagcccccaaactcctcatctatggtaacaacaaccggccctcaggggtccctgaccgattctccggctccaagtctggcacctcagcctccctggccatcactgggctccaggctgaggatgaggctgattattactgccagtcctatgacagcagccagaatgctttctatgtcttcggaactgggaccaaggtcaccgtcctag

SEQ ID NO: 894 - protein, 112 aa, Homo sapiens
QSVLTQPPSVSGAPGQRVTISCTGSSSNIGADYDVHWYQQLPGAAPKLLIYGNNNRPSGVPDRFSGSKSGTSASLAITGLQAEDEADYYCQSYDSSQNAFYVFGTGTKVTVL

SEQ ID NO: 895 - protein, 8 aa, Homo sapiens
GGTFSSYG

SEQ ID NO: 896 - protein, 8 aa, Homo sapiens
IIPVFGAT

SEQ ID NO: 897 - protein, 16 aa, Homo sapiens
ARDALSASGWTGPFDS

SEQ ID NO: 898 - protein, 9 aa, Homo sapiens
SSNIGADYD

SEQ ID NO: 899 - skipped

SEQ ID NO: 900 - protein, 12 aa, Homo sapiens
QSYDSSQNAFYV

SEQ ID NO: 901 - DNA, 390 bp, Homo sapiens
  source 1..390: mol_type = other DNA
caggtgcagctggtggagtctgggggaggcttggtacagcctggcaggtccctgagactctcctgtgcagcctctggattcacctttgatgattatgccatgcactgggtccggcaagctccagggaagggcctggagtgggtctcaggaagtacttggaatagtggtaccatagactatgcggactctgtgaagggccgattcaccatctccagagacaacgccaagaactccctgtatctgcaaatgaacagtctgagagctgaggacacggccttgtattactgtgcaaaagataggtttcgtaaaggttgtagtagtaccggctgctataaggagaactacggtatggacgtctggggccaagggaccacggtcaccgtctcctca

SEQ ID NO: 902 - protein, 130 aa, Homo sapiens
QVQLVESGGGLVQPGRSLRLSCAASGFTFDDYAMHWVRQAPGKGLEWVSGSTWNSGTIDYADSVKGRFTISRDNAKNSLYLQMNSLRAEDTALYYCAKDRFRKGCSSTGCYKENYGMDVWGQGTTVTVSS

SEQ ID NO: 903 - DNA, 325 bp, Homo sapiens
  source 1..325: mol_type = other DNA
cagtctgtggtgactcagccaccctcggtgtcagtggccccaggacagacggccaggattacctgtggaggaaccaacattggaagtaaaagtgtccactggtaccagcagaagccaggccaggcccctgtgctggtcgtctatgatgatagcgaccggccctcagggatccctgagcgattctctggctccaactctgggaacacggccaccctgaccatcacctgggtcgaagccggggatgaggccgactattactgtcaggtgtgggatagtagtagtgataatgtgctattcggcggagggaccaagctgaccgtcctag

SEQ ID NO: 904 - protein, 108 aa, Homo sapiens
QSVVTQPPSVSVAPGQTARITCGGTNIGSKSVHWYQQKPGQAPVLVVYDDSDRPSGIPERFSGSNSGNTATLTITWVEAGDEADYYCQVWDSSSDNVLFGGGTKLTVL

SEQ ID NO: 905 - protein, 8 aa, Homo sapiens
GFTFDDYA

SEQ ID NO: 906 - protein, 8 aa, Homo sapiens
STWNSGTI

SEQ ID NO: 907 - protein, 23 aa, Homo sapiens
AKDRFRKGCSSTGCYKENYGMDV

SEQ ID NO: 908 - protein, 6 aa, Homo sapiens
NIGSKS

SEQ ID NO: 909 - skipped

SEQ ID NO: 910 - protein, 11 aa, Homo sapiens
QVWDSSSDNVL

SEQ ID NO: 911 - DNA, 355 bp, Homo sapiens
  source 1..355: mol_type = other DNA
gaggtgcagctggtggagtctgggggaggtgtggtccagcctggggggtccctgagactctcctgtgcagcctctggaatcatagtcagtgccaactacatgacctgggtccgccaggctccagggaagggactggaatgggtctcagttatttaccccggtggtagcacattctacgcggactccgtgaagggccgattcaccatctccagagacaactccaagaacacgttgtatcttcaaatgaacagcctgagagttgaggactcggctgtgtattactgtgcgagagatttggagctggctggtttcaatgactactggggccagggaaccctggtcaccgtctcctcag

SEQ ID NO: 912 - protein, 118 aa, Homo sapiens
EVQLVESGGGVVQPGGSLRLSCAASGIIVSANYMTWVRQAPGKGLEWVSVIYPGGSTFYADSVKGRFTISRDNSKNTLYLQMNSLRVEDSAVYYCARDLELAGFNDYWGQGTLVTVSS

SEQ ID NO: 913 - DNA, 328 bp, Homo sapiens
  source 1..328: mol_type = other DNA
gatattgtgatgactcagtctccaggcaccctgtctttgtctccaggggaaagagccaccctctcctgcaggaccagtcagagtgttagcagcaactacttagcctggtaccagcagaaacctggccaggctcccaggctcctcatctatggtgcatccagcagggccactggcatcccagacaggttcagtggcagtgggtctgggacagacttcactctcaccatcagcagactggagcctgaagattttgcagtgtattactgtcagcagtttggtagttcacctcggtacacttttggccaggggaccaaggtggagatcaaac

SEQ ID NO: 914 - protein, 109 aa, Homo sapiens
DIVMTQSPGTLSLSPGERATLSCRTSQSVSSNYLAWYQQKPGQAPRLLIYGASSRATGIPDRFSGSGSGTDFTLTISRLEPEDFAVYYCQQFGSSPRYTFGQGTKVEIK

SEQ ID NO: 915 - protein, 8 aa, Homo sapiens
GIIVSANY

SEQ ID NO: 916 - protein, 7 aa, Homo sapiens
IYPGGST

SEQ ID NO: 917 - protein, 12 aa, Homo sapiens
ARDLELAGFNDY

SEQ ID NO: 918 - protein, 7 aa, Homo sapiens
QSVSSNY

SEQ ID NO: 919 - skipped

SEQ ID NO: 920 - protein, 10 aa, Homo sapiens
QQFGSSPRYT

SEQ ID NO: 921 - DNA, 355 bp, Homo sapiens
  source 1..355: mol_type = other DNA
caggtgcagctggtggagtctggggctgaggtgaagaagcctgggtcctcggtgaaggtctcctgcaaggcttctggaggaaacttcaacatgtatactatcagttgggtgcgacaggcccctggacgaggacttgagtggatgggaaggttcatccctatcgctaataaagcaaactacgcacagaactttccgggcagagtcaccattaccgcggacaaatccactagcacagtctacatggagctgagaagcctgacatctgacgacacggccgtgtattactgtgcgagaagtgggagctacgatgcttttgatgtgtggggccaagggacaatggtcaccgtctcttcag

SEQ ID NO: 922 - protein, 118 aa, Homo sapiens
QVQLVESGAEVKKPGSSVKVSCKASGGNFNMYTISWVRQAPGRGLEWMGRFIPIANKANYAQNFPGRVTITADKSTSTVYMELRSLTSDDTAVYYCARSGSYDAFDVWGQGTMVTVSS

SEQ ID NO: 923 - DNA, 325 bp, Homo sapiens
  source 1..325: mol_type = other DNA
gccatccggatgacccagtctccttccaccctgtctgcatctgtaggagacagagtcaccatcacttgccgggccagtcagactattaatagttggttggcctggtatcagcagaaacccgggaaagcccctaagctcctgatctatgatgcctccaatttggaaagtggggtcccatcaaggttcagcggcagtggatctgggacagaattcactctcaccatcagcagcctgcagcctgatgattttgcaacttattactgccaacagtatgaaagttattctccgatcaccttcggccaagggacacgactggagattaaac

SEQ ID NO: 924 - protein, 108 aa, Homo sapiens
AIRMTQSPSTLSASVGDRVTITCRASQTINSWLAWYQQKPGKAPKLLIYDASNLESGVPSRFSGSGSGTEFTLTISSLQPDDFATYYCQQYESYSPITFGQGTRLEIK

SEQ ID NO: 925 - protein, 8 aa, Homo sapiens
GGNFNMYT

SEQ ID NO: 926 - protein, 8 aa, Homo sapiens
FIPIANKA

SEQ ID NO: 927 - protein, 11 aa, Homo sapiens
ARSGSYDAFDV

SEQ ID NO: 928 - protein, 6 aa, Homo sapiens
QTINSW

SEQ ID NO: 929 - skipped

SEQ ID NO: 930 - protein, 10 aa, Homo sapiens
QQYESYSPIT

SEQ ID NO: 931 - DNA, 369 bp, Homo sapiens
  source 1..369: mol_type = other DNA
caggtgcagctggtggagtctgggggagtcgtggtacagcctggggggtccctgagactctcctgtgcagcctctggattcagctttgatgattatagcatgcactgggtccgtcaagctccggggaagggtctggagtgggtctctgtcatttactgggatggtgttagcaaatactatgcagactctgtgaagggccgattcaccatctccagagacaacagcaaaaactccctgtatttgcaaatgaacagtctgagaactgaggacaccgccgtatattactgtgcaaaagatagtgaggattgtagtagtaccagctgctacatggacgtctggggcaaagggaccacggtcaccgtctcctca

SEQ ID NO: 932 - protein, 123 aa, Homo sapiens
QVQLVESGGVVVQPGGSLRLSCAASGFSFDDYSMHWVRQAPGKGLEWVSVIYWDGVSKYYADSVKGRFTISRDNSKNSLYLQMNSLRTEDTAVYYCAKDSEDCSSTSCYMDVWGKGTTVTVSS

SEQ ID NO: 933 - DNA, 340 bp, Homo sapiens
  source 1..340: mol_type = other DNA
gaaattgtgttgacacagtctccagactccctggctgtgtctctgggcgagagggccaccatcaactgcaagtccagccagaatgttttatacagctccaacaataagaattacttagcttggtaccagcagaaaccaggacagcctcctcaactactcatttactgggcatctacccgggaatccggggtccctgaccgattcagtggcagcgggtctgggacagatttcactctcaccatcagcagcctgcaggctgaagatgtggcagtttattactgtcaccaatattatagtactccattcactttcggccctgggaccaaagtggatatcaaac

SEQ ID NO: 934 - protein, 113 aa, Homo sapiens
EIVLTQSPDSLAVSLGERATINCKSSQNVLYSSNNKNYLAWYQQKPGQPPQLLIYWASTRESGVPDRFSGSGSGTDFTLTISSLQAEDVAVYYCHQYYSTPFTFGPGTKVDIK

SEQ ID NO: 935 - protein, 8 aa, Homo sapiens
GFSFDDYS

SEQ ID NO: 936 - protein, 8 aa, Homo sapiens
IYWDGVSK

SEQ ID NO: 937 - protein, 16 aa, Homo sapiens
AKDSEDCSSTSCYMDV

SEQ ID NO: 938 - protein, 12 aa, Homo sapiens
QNVLYSSNNKNY

SEQ ID NO: 939 - skipped

SEQ ID NO: 940 - protein, 9 aa, Homo sapiens
HQYYSTPFT

SEQ ID NO: 941 - DNA, 370 bp, Homo sapiens
  source 1..370: mol_type = other DNA
caggttcagctggtgcagtctggagctgaggtgaagaagcctggggcctcagtgaaggtctcctgcaaggctgctggttacagctttatgaactacggtatcaactgggtgcgacaggcccctggacaagggcttgagtggatgggatggatcaacacttacaatggtaacgcaaagtatgcacagaagttccagggccgagtcaccatgaccacagacacatccacgagcacagcctacatggagctgaggagcctgagatcgggcgacacggccgtgtattactgtgcgagggaccctttcaccggttatgatgacgtttgggggggggactactggggccagggaaccctggtcaccgtctcctcag

SEQ ID NO: 942 - protein, 123 aa, Homo sapiens
QVQLVQSGAEVKKPGASVKVSCKAAGYSFMNYGINWVRQAPGQGLEWMGWINTYNGNAKYAQKFQGRVTMTTDTSTSTAYMELRSLRSGDTAVYYCARDPFTGYDDVWGGDYWGQGTLVTVSS

SEQ ID NO: 943 - DNA, 340 bp, Homo sapiens
  source 1..340: mol_type = other DNA
gccatccagatgacccagtctccagactccctggctgtgtctctgggcgagagggccaccatcaactgcaagtccagccagagtgttttatacagctccaacaataagaattacttagcttggtaccagcagaaaccaggacagcctcctaagctggtcatttactgggcatctacccgggaatccggggtccctgaccgattcagtggcagcgggtctgggacagatttcactctcaccatcagcagcctgcaggctgaagatgtggcagtttattactgtcaccaatattatagtagtcctcgcacttttggccaggggaccaaggtggaaatcaaac

SEQ ID NO: 944 - protein, 113 aa, Homo sapiens
AIQMTQSPDSLAVSLGERATINCKSSQSVLYSSNNKNYLAWYQQKPGQPPKLVIYWASTRESGVPDRFSGSGSGTDFTLTISSLQAEDVAVYYCHQYYSSPRTFGQGTKVEIK

SEQ ID NO: 945 - protein, 8 aa, Homo sapiens
GYSFMNYG

SEQ ID NO: 946 - protein, 8 aa, Homo sapiens
INTYNGNA

SEQ ID NO: 947 - protein, 16 aa, Homo sapiens
ARDPFTGYDDVWGGDY

SEQ ID NO: 948 - protein, 12 aa, Homo sapiens
QSVLYSSNNKNY

SEQ ID NO: 949 - skipped

SEQ ID NO: 950 - protein, 9 aa, Homo sapiens
HQYYSSPRT

SEQ ID NO: 951 - DNA, 375 bp, Homo sapiens
  source 1..375: mol_type = other DNA
gaggtgcagctgttggagactgggggaggcttggttcagcccggcaggtccctgagactctcctgtgcagcctcgggattcccctttgatgattatgccatccactgggtccggctagctccagggaagggcctggagtgggtctcaagtattagttgggatagtggtagcataggctatgcggactctgtgaagggccggttcaccatctccagagacaacgccaagaactccctgtatctgcaaatgaacagtctgagagctgaggacacggccttgtattactgtgcaaagggggcctttcccgggtatagcagtggctggtactacggtttggacgtctggggccaaggggccacggtcaccgtctcctca

SEQ ID NO: 952 - protein, 125 aa, Homo sapiens
EVQLLETGGGLVQPGRSLRLSCAASGFPFDDYAIHWVRLAPGKGLEWVSSISWDSGSIGYADSVKGRFTISRDNAKNSLYLQMNSLRAEDTALYYCAKGAFPGYSSGWYYGLDVWGQGATVTVSS

SEQ ID NO: 953 - DNA, 328 bp, Homo sapiens
  source 1..328: mol_type = other DNA
cagtctgtcgtgacgcagcctccctccgcgtcggggtctcttggacagtcagtcaccatctcctgcactggaaccagcagtgacgttggtggttacaactatgtctcttggtaccaacaacacccaggcaaagcccccaaactcatgatttttgaggtcagtaagcggccctcaggggtccctgatcgcttctctggctccaagtctggcaacacggcctccctgaccgtctctgggctccaggctgaggatgaggctgattattactgcagctcatatgcaggcaacaaaggggtcttcggcggagggaccaaattgaccgtcctcg

SEQ ID NO: 954 - protein, 109 aa, Homo sapiens
QSVVTQPPSASGSLGQSVTISCTGTSSDVGGYNYVSWYQQHPGKAPKLMIFEVSKRPSGVPDRFSGSKSGNTASLTVSGLQAEDEADYYCSSYAGNKGVFGGGTKLTVL

SEQ ID NO: 955 - protein, 8 aa, Homo sapiens
GFPFDDYA

SEQ ID NO: 956 - protein, 8 aa, Homo sapiens
ISWDSGSI

SEQ ID NO: 957 - protein, 18 aa, Homo sapiens
AKGAFPGYSSGWYYGLDV

SEQ ID NO: 958 - protein, 9 aa, Homo sapiens
SSDVGGYNY

SEQ ID NO: 959 - skipped

SEQ ID NO: 960 - protein, 9 aa, Homo sapiens
SSYAGNKGV

SEQ ID NO: 961 - protein, 97 aa, Homo sapiens
MQLVQSGPEVKKPGTSVKVSCKASGFTFTSSAVQWVRQARGQRLEWIGWIVVGSGNTNYAQKFQERVTITRDMSTSTAYMELSSLRSEDTAVYYCAA

SEQ ID NO: 962 - DNA, 369 bp, Homo sapiens
  source 1..369: mol_type = other DNA
caaatgcagctggtgcagtctgggcctgaggtgaagaagcctgggacctcagtgaaggtctcctgcaaggcttctggattcacctttatgagctctgctgtgcagtgggtgcgacaggctcgtggacaacgccttgagtggataggatggatcgtcattggcagtggtaacacaaactacgcacagaagttccaggaaagagtcaccattaccagggacatgtccacaagcacagcctacatggagctgagcagcctgagatccgaggacacggccgtgtattactgtgcggccccatattgtagtagtatcagctgcaatgatggttttgatatctggggccaagggacaatggtcaccgtctcttca

SEQ ID NO: 963 - protein, 123 aa, Homo sapiens
QMQLVQSGPEVKKPGTSVKVSCKASGFTFMSSAVQWVRQARGQRLEWIGWIVIGSGNTNYAQKFQERVTITRDMSTSTAYMELSSLRSEDTAVYYCAAPYCSSISCNDGFDIWGQGTMVTVSS

SEQ ID NO: 964 - DNA, 327 bp, Homo sapiens
  source 1..327: mol_type = other DNA
gaaattgtgttgacgcagtctccaggcaccctgtctttgtctccaggggagagagccaccctctcctgcagggccagtcagagtgttagcagcagctacttagcctggtaccagcagaaacctggccaggctcccaggctcctcatctatggtgcatccagcagggccactggcatcccagacaggttcagtggcagtgggtctgggacagacttcactctcaccatcagcagactggagcctgaagattttgcagtgtattactgtcagcactatggtagctcacggggttggacgttcggccaagggaccaaggtggaaatcaaa

SEQ ID NO: 965 - protein, 109 aa, Homo sapiens
EIVLTQSPGTLSLSPGERATLSCRASQSVSSSYLAWYQQKPGQAPRLLIYGASSRATGIPDRFSGSGSGTDFTLTISRLEPEDFAVYYCQHYGSSRGWTFGQGTKVEIK

SEQ ID NO: 966 - protein, 1273 aa, Homo sapiens
MFVFLVLLPLVSSQCVNLTTRTQLPPAYTNSFTRGVYYPDKVFRSSVLHSTQDLFLPFFSNVTWFHAIHVSGTNGTKRFDNPVLPFNDGVYFASTEKSNIIRGWIFGTTLDSKTQSLLIVNNATNVVIKVCEFQFCNDPFLGVYYHKNNKSWMESEFRVYSSANNCTFEYVSQPFLMDLEGKQGNFKNLREFVFKNIDGYFKIYSKHTPINLVRDLPQGFSALEPLVDLPIGINITRFQTLLALHRSYLTPGDSSSGWTAGAAAYYVGYLQPRTFLLKYNENGTITDAVDCALDPLSETKCTLKSFTVEKGIYQTSNFRVQPTESIVRFPNITNLCPFGEVFNATRFASVYAWNRKRISNCVADYSVLYNSASFSTFKCYGVSPTKLNDLCFTNVYADSFVIRGDEVRQIAPGQTGKIADYNYKLPDDFTGCVIAWNSNNLDSKVGGNYNYLYRLFRKSNLKPFERDISTEIYQAGSTPCNGVEGFNCYFPLQSYGFQPTNGVGYQPYRVVVLSFELLHAPATVCGPKKSTNLVKNKCVNFNFNGLTGTGVLTESNKKFLPFQQFGRDIADTTDAVRDPQTLEILDITPCSFGGVSVITPGTNTSNQVAVLYQDVNCTEVPVAIHADQLTPTWRVYSTGSNVFQTRAGCLIGAEHVNNSYECDIPIGAGICASYQTQTNSPRRARSVASQSIIAYTMSLGAENSVAYSNNSIAIPTNFTISVTTEILPVSMTKTSVDCTMYICGDSTECSNLLLQYGSFCTQLNRALTGIAVEQDKNTQEVFAQVKQIYKTPPIKDFGGFNFSQILPDPSKPSKRSFIEDLLFNKVTLADAGFIKQYGDCLGDIAARDLICAQKFNGLTVLPPLLTDEMIAQYTSALLAGTITSGWTFGAGAALQIPFAMQMAYRFNGIGVTQNVLYENQKLIANQFNSAIGKIQDSLSSTASALGKLQDVVNQNAQALNTLVKQLSSNFGAISSVLNDILSRLDKVEAEVQIDRLITGRLQSLQTYVTQQLIRAAEIRASANLAATKMSECVLGQSKRVDFCGKGYHLMSFPQSAPHGVVFLHVTYVPAQEKNFTTAPAICHDGKAHFPREGVFVSNGTHWFVTQRNFYEPQIITTDNTFVSGNCDVVIGIVNNTVYDPLQPELDSFKEELDKYFKNHTSPDVDLGDISGINASVVNIQKEIDRLNEVAKNLNESLIDLQELGKYEQYIKWPWYIWLGFIAGLIAIVMVTIMLCCMTSCCSCLKGCCSCGSCCKFDEDDSEPVLKGVKLHYT

SEQ ID NO: 967 - protein, 96 aa, Homo sapiens
EIVLTQSPGTLSLSPGERATLSCRASQSVSSSYLAWYQQKPGQAPRLLIYGASSRATGIPDRFSGSGSGTDFTLTISRLEPEDFAVYYCQQYGSSP